European Patent Application EP 4 729 075 A1, published April 22, 2026. Title: 靶向乙型肝炎病毒基因的表观编辑工具. Applicant: 益杰立科（上海）生物科技有限公司. The sequence listing filed with the application follows.

SEQUENCE LISTING (1196 sequences)

SEQ ID NO: 1 - DNA, 3215 bp, synthetic construct
  misc_feature 1..3215: note = HBV-B gene
  source 1..3215: mol_type = other DNA
ctccaccactttccaccaaactcttcaagatcccagagtcagggccctgtactttcctgctggtggctccagttcaggaacagtgagccctgctcagaatactgtctctgccatatcgtcaatcttatcgaagactggggaccctgtaccgaacatggagaacatcgcatcaggactcctaggacccctgctcgtgttacaggcggggtttttcttgttgacaaaaatcctcacaataccacagagtctagactcgtggtggacttctctcaattttctagggggaacacccgtgtgtcttggccaaaattcgcagtcccaaatctccagtcactcaccaacctgttgtcctccaatttgtcctggttatcgctggatgtgtctgcggcgttttatcatcttcctctgcatcctgctgctatgcctcatcttcttgttggttcttctggactatcaaggtatgttgcccgtttgtcctctaattccaggatcatcaacaaccagcaccggaccatgcaaaacctgcacaactcctgctcaaggaacctctatgtttccctcatgttgctgtacaaaacctacggacggaaactgcacctgtattcccatcccatcatcttgggctttcgcaaaatacctatgggagtgggcctcagtccgtttctcttggctcagtttactagtgccatttgttcagtggttcgtagggctttcccccactgtctggctttcagttatatggatgatgtggttttgggggccaagtctgtacaacatcttgagtccctttatgccgctgttaccaattttcttttgtctttgggtatacatttaaaccctcacaaaacaaaaagatggggatattcccttaacttcatgggatatgtaattgggagttggggcacattgccacaggaacatattgtacaaaaaatcaaaatgtgttttaggaaacttcctgtaaacaggcctattgattggaaagtatgtcaacgaattgtgggtcttttggggtttgccgcccctttcacgcaatgtggatatcctgctttaatgcctttatatgcatgtatacaagcgaaacaggcttttactttctcgccaacttacaaggcctttctaagtaaacagtatctgaacctttaccccgttgctcggcaacggcctggtctgtgccaagtgtttgctgacgcaacccccactggttggggcttggccataggccatcagcgcatgcgtggaacctttgtgtctcctctaccgatccatactgcggaactcctagccgcttgttttgctcgcagcaggtctggggcaaacctcatcgggactgacaattctgtcgtgctctcccgcaagtatacatcatttccatggctgctaggctgtgctgccaactggatcctgcgcgggacgtcctttgtttacgtcccgtcggcgctgaatcccgcggacgacccctctcggggccgcttgggactctaccgcccgcttctccgcctattgtaccggccgaccacggggcgcacctctctttacgcggactccccgtctgtgccttctcatctgccggaccgtgtgcacttcgcttcacctctgcacgtcgcatggagaccaccgtgaacgcccacaggaacctgcccaaggtcttgcataagaggactcttggactttcagcaatgtcaacgaccgaccttgaggcatacttcaaagactgtgtgtttactgagtgggaggagttgggggaggaggttaggttaaaggtctttgtactaggaggctgtaggcataaattggtgtgttcaccagcaccatgcaactttttcacctctgcctaatcatctcatgttcatgtcctactgttcaagcctccaagctgtgccttgggtggctttggggcatggacattgacccgtataaagaatttggagcttctgtggagttactctcttttttgccttctgacttctttccttctattcgagatctcctcgacaccgcctctgctctgtatcgggaggccttagagtctccggaacattgttcacctcaccatacggcactcaggcaagctatcctgtgttggggtgagttgatgaatctagctacctgggtgggaagtaatttggaagatccagcatccagggaattagtagtcagctatgtcaacgttaacatgggcctaaaaatcagacaactcttgtggtttcacatttcctgtcttacttttgggagagaaactgtccttgaatatttggtgtcttttggagtgtggattcgcactcctcctgcatatagaccaccaaatgcccctatcttatcaactcttccggaaactactgttgttagacgacgaggcaggtcccctagaagaagaactccctcgcctcgcagacgaaggtctcaatcgccgcgtcgcagaagatatcaatctcgggaatctcaatgttagtattccttggacacataaggtgggaaactttacggggctttattcttctacggtaccttgctttaatcctaaatggcaaactccttcttttcctgacattcatttgcaggaggacattgttgatagatgtaagcaatttgtggggccccttacagtaaatgaaaacaggagactgaaattaattatgcctgctaggttttatcccaatgttactaaatatttgcccttagataaagggatcaaaccgtattatccagagtatgtagttaatcattacttccagacgcgacattatttacacactctttggaaggcggggatcttatataaaagagagtccacacgtagcgcctcattttgcgggtcaccatattcttgggaacaagatctacagcatgggaggttggtcttccaaacctcgaaaaggcatggggacaaatctttctgtccccaatcccctgggattcttccccgatcatcagttggaccctgcattcaaagccaactcagaaagtccagattgggacctcaacccgcacaaggacaactggccggacgccaacaaggtgggagtgggagcattcgggccagggttcacccctccccatgggggactgttggggtggagccctcaggctcagggcctactcacaactgtgccagcagctcctcctcctgcctccaccaatcggcagtcaggaaggcagcctactcccttatctccacctctaagggacactcatcctcaggccatgcagtggaa

SEQ ID NO: 2 - DNA, 3215 bp, synthetic construct
  misc_feature 1..3215: note = HBV-C gene
  source 1..3215: mol_type = other DNA
ctccacaacattccaccaagctctgctagatcccagagtgaggggcctatattttcctgctggtggctccagttccggaacagtaaaccctgttccgactactgcctcacccatatcgtcaatcttctcgaggactggggaccctgcaccgaacatggagaacacaacatcaggattcctaggacccctgctcgtgttacaggcggggtttttcttgttgacaagaatcctcacaataccacagagtctagactcgtggtggacttctctcaattttctagggggagcacccacgtgtcctggccaaaattcgcagtccccaacctccaatcactcaccaacctcttgtcctccaatttgtcctggctatcgctggatgtgtctgcggcgttttatcatattcctcttcatcctgctgctatgcctcatcttcttgttggttcttctggactaccaaggtatgttgcccgtttgtcctctacttccaggaacatcaaccaccagcacggggccatgcaagacctgcacgattcctgctcaaggaacctctatgtttccctcttgttgctgtacaaaaccttcggacggaaactgcacttgtattcccatcccatcatcctgggctttcgcaagattcctatgggagtgggcctcagtccgtttctcctggctcagtttactagtgccatttgttcagtggttcgtagggctttcccccactgtttggctttcagttatatggatgatgtggtattgggggccaagtctgtacaacatcttgagtccctttttacctctattaccaattttcttttgtctttgggtatacatttaaaccctaataaaaccaaacgttggggctactcccttaacttcatgggatatgtaattggaagttggggtactttaccgcaggaacatattgtactaaaactcaagcaatgttttcgaaaattacctgtaaatagacctattgattggaaagtctgtcaaagaattgtgggtcttttgggctttgctgccccttttacacaatgtggctatcctgccttgatgcctttatatgcatgtatacaatctaagcaggctttcactttctcgccaacttacaaggcctttctgtgtaaacaatatctgaacctttaccccgttgcccggcaacggtcaggtctctgccaagtgtttgctgacgcaacccccactggatggggcttggccataggccatcggcgcatgcgtggaacctttgtggctcctctgccgatccatactgcggaactcctagcagcttgtttcgctcgcagccggtctggagcgaaacttatcggcaccgacaactctgttgtcctctctcggaaatacacctcctttccatggctgctagggtgtgctgccaactggatcctgcgcgggacgtcctttgtctacgtcccgtcggcgctgaatcccgcggacgacccgtctcggggccgtttggggctctaccgtccccttcttcatctgccgttccggccgaccacggggcgcacctctctttacgcggtctccccgtctgtgccttctcatctgccggaccgtgtgcacttcgcttcacctctgcacgtcgcatggagaccaccgtgaacgcccaccaggtcttgcccaaggtcttacataagaggactcttggactctcagcaatgtcaacgaccgaccttgaggcatacttcaaagactgtgtgtttaaagactgggaggagttgggggaggagattaggttaaaggtctttgtactaggaggctgtaggcataaattggtctgttcaccagcaccatgcaactttttcacctctgcctaatcatctcatgttcatgtcctactgttcaagcctccaagctgtgccttgggtggctttggggcatggacattgacccgtataaagaatttggagcatctgtggagttactctcttttttgccttctgacttctttccttctattcgagatctcctcgacaccgcttctgctctgtatcgggaggccttagagtctccggaacattgttcacctcaccatacagcactcaggcaagctattctgtgttggggtgagttgatgaatctggccacctgggtgggaagtaatttggaagacccagcatccagggaattagtagtcagctatgtcaatgttaatatgggcctaaaaatcagacaactattgtggtttcacatttcctgtcttacttttggaagagaaactgttcttgagtatttggtatcttttggagtgtggattcgcactcctcccgcttacagaccaccaaatgcccctatcttatcaacacttccggaaactactgttgttagacgacgaggcaggtcccctagaagaagaactccctcgcctcgcagacgaagatctcaatcgccgcgtcgcagaagatctcaatctcgggaatctcaatgttagtatcccttggactcataaggtgggaaactttactgggctttattcttctactgtacctgtctttaatcccgagtggcaaactccctcctttcctcacattcatttacaggaggacattattaatagatgtcaacaatatgtgggccctcttacagttaatgaaaaaaggagattaaaattaattatgcctgctaggttctatcctaaccttaccaaatatttgcccttagacaaaggcattaaaccgtattatcctgaacatgcagttaatcattacttcaaaactaggcattatttacatactctgtggaaggctggcattctatataagagagaaactacacgcagcgcctcattttgtgggtcaccatattcttgggaacaagagctacagcatgggaggttggtcttccaaacctcgacaaggcatggggacgaatctttctgttcccaatcctctgggattctttcccgatcaccagttggaccctgcgttcggagccaactcaaacaatccagattgggacttcaaccccaacaaggatcactggccagaggcaaatcaggtaggagcgggagcattcgggccagggttcaccccaccacacggcggtcttttggggtggagccctcaggctcagggcatattgacaacagtgccagcagcacctcctcctgcctccaccaatcggcagtcaggaagacagcctactcccatctctccacctctaagagacagtcatcctcaggccatgcagtggaa

SEQ ID NO: 3 - DNA, 3182 bp, synthetic construct
  misc_feature 1..3182: note = HBV-D gene
  source 1..3182: mol_type = other DNA
ttccacaacctttcaccaaactctgcaagatcccagagtgagaggcctgtatttccctgctggtggctccagttcaggagcagtaaaccctgttccgactactgcctctcccttatcgtcaatcttctcgaggattggggaccctgcgctgaacatggagaacatcacatcaggattcctaggaccccttctcgtgttacaggcggggtttttcttgttgacaagaatcctcacaataccgcagagtctagactcgtggtggacttctctcaattttctagggggaactaccgtgtgtcttggccaaaattcgcagtccccaacctccaatcactcaccaacctcctgtcctccaacttgtcctggttatcgctggatgtgtctgcggcgttttatcatcttcctcttcatcctgctgctatgcctcatcttcttgttggttcttctggactatcaaggtatgttgcccgtttgtcctctaattccaggatcctcaaccaccagcacgggaccatgccgaacctgcatgactactgctcaaggaacctctatgtatccctcctgttgctgtaccaaaccttcggacggaaattgcacctgtattcccatcccatcatcctgggctttcggaaaattcctatgggagtgggcctcagcccgtttctcctggctcagtttactagtgccatttgttcagtggttcgtagggctttcccccactgtttggctttcagttatatggatgatgtggtattgggggccaagtctgtacagcatcttgagtccctttttaccgctgttaccaattttcttttgtctttgggtatacatttaaaccctaacaaaacaaagagatggggttactctctgaattttatgggttatgtcattggaagttatgggtccttgccacaagaacacatcatacaaaaaatcaaagaatgttttagaaaacttcctattaacaggcctattgattggaaagtatgtcaacgaattgtgggtcttttgggttttgctgccccatttacacaatgtggttatcctgcgttaatgcccttgtatgcatgtattcaatctaagcaggctttcactttctcgccaacttacaaggcctttctgtgtaaacaatacctgaacctttaccccgttgcccggcaacggccaggtctgtgccaagtgtttgctgacgcaacccccactggctggggcttggtcatgggccatcagcgcgtgcgtggaaccttttcggctcctctgccgatccatactgcggaactcctagccgcttgttttgctcgcagcaggtctggagcaaacattatcgggactgataactctgttgtcctctcccgcaaatatacatcgtatccatggctgctaggctgtgctgccaactggatcctgcgcgggacgtcctttgtttacgtcccgtcggcgctgaatcctgcggacgacccttctcggggtcgcttgggactctctcgtccccttctccgtctgccgttccgaccgaccacggggcgcacctctctttacgcggactccccgtctgtgccttctcatctgccggaccgtgtgcacttcgcttcacctctgcacgtcgcatggagaccaccgtgaacgcccaccgaatgttgcccaaggtcttacataagaggactcttggactctctgcaatgtcaacgaccgaccttgaggcatacttcaaagactgtttgtttaaagactgggaggagttgggggaggagattagattaaaggtctttgtactaggaggctgtaggcataaattggtctgcgcaccagcaccatgcaactttttcacctctgcctaatcatctcttgttcatgtcctactgttcaagcctccaagctgtgccttgggtggctttggggcatggacatcgacccttataaagaatttggagctactgtggagttactctcgtttttgccttctgacttctttccttcagtacgagatcttctagataccgcctcagctctgtatcgggaagccttagagtctcctgagcattgttcacctcaccatactgcactcaggcaagcaattctttgctggggggaactaatgactctagctacctgggtgggtgttaatttggaagatccagcatctagagacctagtagtcagttatgtcaacactaatatgggcctaaagttcaggcaactcttgtggtttcacatttcttgtctcacttttggaagagaaaccgttatagagtatttggtgtctttcggagtgtggattcgcactcctccagcttatagaccaccaaatgcccctatcctatcaacacttccggaaactactgttgttagacgacgaggcaggtcccctagaagaagaactccctcgcctcgcagacgaaggtctcaatcgccgcgtcgcagaagatctcaatctcgggaacctcaatgttagtattccttggactcataaggtggggaactttactggtctttattcttctactgtacctgtctttaatcctcattggaaaacaccatcttttcctaatatacatttacaccaagacattatcaaaaaatgtgaacagtttgtaggcccacttacagttaatgagaaaagaagattgcaattgattatgcctgctaggttttatccaaaggttaccaaatatttaccattggataagggtattaaaccttattatccagaacatctagttaatcattacttccaaactagacactatttacacactctatggaaggcgggtatattatataagagagaaacaacacatagcgcctcattttgtgggtcaccatattcttgggaacaagatctacagcatggggcagaatctttccaccagcaatcctctgggattctttcccgaccaccagttggatccagccttcagagcaaacacagcaaatccagattgggacttcaatcccaacaaggacacctggccagacgccaacaaggtaggagctggagcattcgggctgggtttcaccccaccgcacggaggccttttggggtggagccctcaggctcagggcatactacaaactttgccagcaaatccgcctcctgcctccaccaatcgccagacaggaaggcagcctaccccgctgtctccacctttgagaaacactcatcctcaggccatgcagtggaa

SEQ ID NO: 4 - DNA, 20 bp, synthetic construct
  misc_feature 1..20: note = HBV-sgRNA-0001
  source 1..20: mol_type = other DNA
aaaaaatcaaaatgtgtttt

SEQ ID NO: 5 - DNA, 20 bp, synthetic construct
  misc_feature 1..20: note = HBV-sgRNA-0002
  source 1..20: mol_type = other DNA
aaaaaatgtgaacagtttgt

SEQ ID NO: 6 - DNA, 20 bp, synthetic construct
  misc_feature 1..20: note = HBV-sgRNA-0003
  source 1..20: mol_type = other DNA
aaaatataggcccctcactc

SEQ ID NO: 7 - DNA, 20 bp, synthetic construct
  misc_feature 1..20: note = HBV-sgRNA-0004
  source 1..20: mol_type = other DNA
aaacaaaggacgtcccgcgc

SEQ ID NO: 8 - DNA, 20 bp, synthetic construct
  misc_feature 1..20: note = HBV-sgRNA-0005
  source 1..20: mol_type = other DNA
aaacacagcaaatccagatt

SEQ ID NO: 9 - DNA, 20 bp, synthetic construct
  misc_feature 1..20: note = HBV-sgRNA-0006
  source 1..20: mol_type = other DNA
aaagaaggagtttgccattt

SEQ ID NO: 10 - DNA, 20 bp, synthetic construct
  misc_feature 1..20: note = HBV-sgRNA-0007
  source 1..20: mol_type = other DNA
aaagaatcccagaggattgc

SEQ ID NO: 11 - DNA, 20 bp, synthetic construct
  misc_feature 1..20: note = HBV-sgRNA-0008
  source 1..20: mol_type = other DNA
aaagatggtgttttccaatg

SEQ ID NO: 12 - DNA, 20 bp, synthetic construct
  misc_feature 1..20: note = HBV-sgRNA-0009
  source 1..20: mol_type = other DNA
aaagcccaagatgatgggat

SEQ ID NO: 13 - DNA, 20 bp, synthetic construct
  misc_feature 1..20: note = HBV-sgRNA-0010
  source 1..20: mol_type = other DNA
aaagcccaggatgatgggat

SEQ ID NO: 14 - DNA, 20 bp, synthetic construct
  misc_feature 1..20: note = HBV-sgRNA-0011
  source 1..20: mol_type = other DNA
aaaggagggagtttgccact

SEQ ID NO: 15 - DNA, 20 bp, synthetic construct
  misc_feature 1..20: note = HBV-sgRNA-0012
  source 1..20: mol_type = other DNA
aaaggtggagacagcggggt

SEQ ID NO: 16 - DNA, 20 bp, synthetic construct
  misc_feature 1..20: note = HBV-sgRNA-0013
  source 1..20: mol_type = other DNA
aaagtacagggccctgactc

SEQ ID NO: 17 - DNA, 20 bp, synthetic construct
  misc_feature 1..20: note = HBV-sgRNA-0014
  source 1..20: mol_type = other DNA
aaagtatgtcaacgaattgt

SEQ ID NO: 18 - DNA, 20 bp, synthetic construct
  misc_feature 1..20: note = HBV-sgRNA-0015
  source 1..20: mol_type = other DNA
aaagtctgtcaaagaattgt

SEQ ID NO: 19 - DNA, 20 bp, synthetic construct
  misc_feature 1..20: note = HBV-sgRNA-0016
  source 1..20: mol_type = other DNA
aaatacaggcctctcactct

SEQ ID NO: 20 - DNA, 20 bp, synthetic construct
  misc_feature 1..20: note = HBV-sgRNA-0017
  source 1..20: mol_type = other DNA
aaatataggcccctcactct

SEQ ID NO: 21 - DNA, 20 bp, synthetic construct
  misc_feature 1..20: note = HBV-sgRNA-0018
  source 1..20: mol_type = other DNA
aaatatttaccattggataa

SEQ ID NO: 22 - DNA, 20 bp, synthetic construct
  misc_feature 1..20: note = HBV-sgRNA-0019
  source 1..20: mol_type = other DNA
aaatatttgcccttagacaa

SEQ ID NO: 23 - DNA, 20 bp, synthetic construct
  misc_feature 1..20: note = HBV-sgRNA-0020
  source 1..20: mol_type = other DNA
aaatatttgcccttagataa

SEQ ID NO: 24 - DNA, 20 bp, synthetic construct
  misc_feature 1..20: note = HBV-sgRNA-0021
  source 1..20: mol_type = other DNA
aaatgaatgtcaggaaaaga

SEQ ID NO: 25 - DNA, 20 bp, synthetic construct
  misc_feature 1..20: note = HBV-sgRNA-0022
  source 1..20: mol_type = other DNA
aaatgaatgtgaggaaagga

SEQ ID NO: 26 - DNA, 20 bp, synthetic construct
  misc_feature 1..20: note = HBV-sgRNA-0023
  source 1..20: mol_type = other DNA
aaatgtatattaggaaaaga

SEQ ID NO: 27 - DNA, 20 bp, synthetic construct
  misc_feature 1..20: note = HBV-sgRNA-0024
  source 1..20: mol_type = other DNA
aacaagagatgattaggcag

SEQ ID NO: 28 - DNA, 20 bp, synthetic construct
  misc_feature 1..20: note = HBV-sgRNA-0025
  source 1..20: mol_type = other DNA
aacaagagctacagcatggg

SEQ ID NO: 29 - DNA, 20 bp, synthetic construct
  misc_feature 1..20: note = HBV-sgRNA-0026
  source 1..20: mol_type = other DNA
aacaagatctacagcatggg

SEQ ID NO: 30 - DNA, 20 bp, synthetic construct
  misc_feature 1..20: note = HBV-sgRNA-0027
  source 1..20: mol_type = other DNA
aacacaacatcaggattcct

SEQ ID NO: 31 - DNA, 20 bp, synthetic construct
  misc_feature 1..20: note = HBV-sgRNA-0028
  source 1..20: mol_type = other DNA
aacatagaggttccttgagc

SEQ ID NO: 32 - DNA, 20 bp, synthetic construct
  misc_feature 1..20: note = HBV-sgRNA-0029
  source 1..20: mol_type = other DNA
aacatcacatcaggattcct

SEQ ID NO: 33 - DNA, 20 bp, synthetic construct
  misc_feature 1..20: note = HBV-sgRNA-0030
  source 1..20: mol_type = other DNA
aacatcgcatcaggactcct

SEQ ID NO: 34 - DNA, 20 bp, synthetic construct
  misc_feature 1..20: note = HBV-sgRNA-0031
  source 1..20: mol_type = other DNA
aacatgagatgattaggcag

SEQ ID NO: 35 - DNA, 20 bp, synthetic construct
  misc_feature 1..20: note = HBV-sgRNA-0032
  source 1..20: mol_type = other DNA
aacatggagaacacaacatc

SEQ ID NO: 36 - DNA, 20 bp, synthetic construct
  misc_feature 1..20: note = HBV-sgRNA-0033
  source 1..20: mol_type = other DNA
aacatggagaacatcacatc

SEQ ID NO: 37 - DNA, 20 bp, synthetic construct
  misc_feature 1..20: note = HBV-sgRNA-0034
  source 1..20: mol_type = other DNA
aacatggagaacatcgcatc

SEQ ID NO: 38 - DNA, 20 bp, synthetic construct
  misc_feature 1..20: note = HBV-sgRNA-0035
  source 1..20: mol_type = other DNA
aacccccactggatggggct

SEQ ID NO: 39 - DNA, 20 bp, synthetic construct
  misc_feature 1..20: note = HBV-sgRNA-0036
  source 1..20: mol_type = other DNA
aacccccactggctggggct

SEQ ID NO: 40 - DNA, 20 bp, synthetic construct
  misc_feature 1..20: note = HBV-sgRNA-0037
  source 1..20: mol_type = other DNA
aacccccactggttggggct

SEQ ID NO: 41 - DNA, 20 bp, synthetic construct
  misc_feature 1..20: note = HBV-sgRNA-0038
  source 1..20: mol_type = other DNA
aacgaattgtgggtcttttg

SEQ ID NO: 42 - DNA, 20 bp, synthetic construct
  misc_feature 1..20: note = HBV-sgRNA-0039
  source 1..20: mol_type = other DNA
aactaatgactctagctacc

SEQ ID NO: 43 - DNA, 20 bp, synthetic construct
  misc_feature 1..20: note = HBV-sgRNA-0040
  source 1..20: mol_type = other DNA
aactgaaagccaaacagtgg

SEQ ID NO: 44 - DNA, 20 bp, synthetic construct
  misc_feature 1..20: note = HBV-sgRNA-0041
  source 1..20: mol_type = other DNA
aactgaaagccagacagtgg

SEQ ID NO: 45 - DNA, 20 bp, synthetic construct
  misc_feature 1..20: note = HBV-sgRNA-0042
  source 1..20: mol_type = other DNA
aacttcatgggatatgtaat

SEQ ID NO: 46 - DNA, 20 bp, synthetic construct
  misc_feature 1..20: note = HBV-sgRNA-0043
  source 1..20: mol_type = other DNA
aagactgtgtgtttaaagac

SEQ ID NO: 47 - DNA, 20 bp, synthetic construct
  misc_feature 1..20: note = HBV-sgRNA-0044
  source 1..20: mol_type = other DNA
aagactgtgtgtttactgag

SEQ ID NO: 48 - DNA, 20 bp, synthetic construct
  misc_feature 1..20: note = HBV-sgRNA-0045
  source 1..20: mol_type = other DNA
aagactgtttgtttaaagac

SEQ ID NO: 49 - DNA, 20 bp, synthetic construct
  misc_feature 1..20: note = HBV-sgRNA-0046
  source 1..20: mol_type = other DNA
aagagtttggtggaaagtgg

SEQ ID NO: 50 - DNA, 20 bp, synthetic construct
  misc_feature 1..20: note = HBV-sgRNA-0047
  source 1..20: mol_type = other DNA
aagccacccaaggcacagct

SEQ ID NO: 51 - DNA, 20 bp, synthetic construct
  misc_feature 1..20: note = HBV-sgRNA-0048
  source 1..20: mol_type = other DNA
aagcctccaagctgtgcctt

SEQ ID NO: 52 - DNA, 20 bp, synthetic construct
  misc_feature 1..20: note = HBV-sgRNA-0049
  source 1..20: mol_type = other DNA
aagctccaaattctttatac

SEQ ID NO: 53 - DNA, 20 bp, synthetic construct
  misc_feature 1..20: note = HBV-sgRNA-0050
  source 1..20: mol_type = other DNA
aaggagggagtttgccactc

SEQ ID NO: 54 - DNA, 20 bp, synthetic construct
  misc_feature 1..20: note = HBV-sgRNA-0051
  source 1..20: mol_type = other DNA
aagggagtagccccaacgtt

SEQ ID NO: 55 - DNA, 20 bp, synthetic construct
  misc_feature 1..20: note = HBV-sgRNA-0052
  source 1..20: mol_type = other DNA
aaggtaggagctggagcatt

SEQ ID NO: 56 - DNA, 20 bp, synthetic construct
  misc_feature 1..20: note = HBV-sgRNA-0053
  source 1..20: mol_type = other DNA
aaggtgggagtgggagcatt

SEQ ID NO: 57 - DNA, 20 bp, synthetic construct
  misc_feature 1..20: note = HBV-sgRNA-0054
  source 1..20: mol_type = other DNA
aagtacagggccctgactct

SEQ ID NO: 58 - DNA, 20 bp, synthetic construct
  misc_feature 1..20: note = HBV-sgRNA-0055
  source 1..20: mol_type = other DNA
aagttggggtactttaccgc

SEQ ID NO: 59 - DNA, 20 bp, synthetic construct
  misc_feature 1..20: note = HBV-sgRNA-0056
  source 1..20: mol_type = other DNA
aatagatgtcaacaatatgt

SEQ ID NO: 60 - DNA, 20 bp, synthetic construct
  misc_feature 1..20: note = HBV-sgRNA-0057
  source 1..20: mol_type = other DNA
aatatttgcccttagataaa

SEQ ID NO: 61 - DNA, 20 bp, synthetic construct
  misc_feature 1..20: note = HBV-sgRNA-0058
  source 1..20: mol_type = other DNA
aatgactctagctacctggg

SEQ ID NO: 62 - DNA, 20 bp, synthetic construct
  misc_feature 1..20: note = HBV-sgRNA-0059
  source 1..20: mol_type = other DNA
aatgtcaacgaccgaccttg

SEQ ID NO: 63 - DNA, 20 bp, synthetic construct
  misc_feature 1..20: note = HBV-sgRNA-0060
  source 1..20: mol_type = other DNA
aattggtaacagcggcataa

SEQ ID NO: 64 - DNA, 20 bp, synthetic construct
  misc_feature 1..20: note = HBV-sgRNA-0061
  source 1..20: mol_type = other DNA
aattggtaacagcggtaaaa

SEQ ID NO: 65 - DNA, 20 bp, synthetic construct
  misc_feature 1..20: note = HBV-sgRNA-0062
  source 1..20: mol_type = other DNA
aattggtaatagaggtaaaa

SEQ ID NO: 66 - DNA, 20 bp, synthetic construct
  misc_feature 1..20: note = HBV-sgRNA-0063
  source 1..20: mol_type = other DNA
aattttatgggttatgtcat

SEQ ID NO: 67 - DNA, 20 bp, synthetic construct
  misc_feature 1..20: note = HBV-sgRNA-0064
  source 1..20: mol_type = other DNA
acaacaggttggtgagtgac

SEQ ID NO: 68 - DNA, 20 bp, synthetic construct
  misc_feature 1..20: note = HBV-sgRNA-0065
  source 1..20: mol_type = other DNA
acaactctgttgtcctctct

SEQ ID NO: 69 - DNA, 20 bp, synthetic construct
  misc_feature 1..20: note = HBV-sgRNA-0066
  source 1..20: mol_type = other DNA
acaagaggttggtgagtgat

SEQ ID NO: 70 - DNA, 20 bp, synthetic construct
  misc_feature 1..20: note = HBV-sgRNA-0067
  source 1..20: mol_type = other DNA
acaagagttgcctgaacttt

SEQ ID NO: 71 - DNA, 20 bp, synthetic construct
  misc_feature 1..20: note = HBV-sgRNA-0068
  source 1..20: mol_type = other DNA
acaagagttgtctgattttt

SEQ ID NO: 72 - DNA, 20 bp, synthetic construct
  misc_feature 1..20: note = HBV-sgRNA-0069
  source 1..20: mol_type = other DNA
acaataggcggagaagcggg

SEQ ID NO: 73 - DNA, 20 bp, synthetic construct
  misc_feature 1..20: note = HBV-sgRNA-0070
  source 1..20: mol_type = other DNA
acaatagttgtctgattttt

SEQ ID NO: 74 - DNA, 20 bp, synthetic construct
  misc_feature 1..20: note = HBV-sgRNA-0071
  source 1..20: mol_type = other DNA
acaatgctcaggagactcta

SEQ ID NO: 75 - DNA, 20 bp, synthetic construct
  misc_feature 1..20: note = HBV-sgRNA-0072
  source 1..20: mol_type = other DNA
acaatgttccggagactcta

SEQ ID NO: 76 - DNA, 20 bp, synthetic construct
  misc_feature 1..20: note = HBV-sgRNA-0073
  source 1..20: mol_type = other DNA
acacatagcgcctcattttg

SEQ ID NO: 77 - DNA, 20 bp, synthetic construct
  misc_feature 1..20: note = HBV-sgRNA-0074
  source 1..20: mol_type = other DNA
acaccctagcagccatggaa

SEQ ID NO: 78 - DNA, 20 bp, synthetic construct
  misc_feature 1..20: note = HBV-sgRNA-0075
  source 1..20: mol_type = other DNA
acaccgcctctgctctgtat

SEQ ID NO: 79 - DNA, 20 bp, synthetic construct
  misc_feature 1..20: note = HBV-sgRNA-0076
  source 1..20: mol_type = other DNA
acaccgcttctgctctgtat

SEQ ID NO: 80 - DNA, 20 bp, synthetic construct
  misc_feature 1..20: note = HBV-sgRNA-0077
  source 1..20: mol_type = other DNA
acacgcagcgcctcattttg

SEQ ID NO: 81 - DNA, 20 bp, synthetic construct
  misc_feature 1..20: note = HBV-sgRNA-0078
  source 1..20: mol_type = other DNA
acacggtccggcagatgaga

SEQ ID NO: 82 - DNA, 20 bp, synthetic construct
  misc_feature 1..20: note = HBV-sgRNA-0079
  source 1..20: mol_type = other DNA
acacgtagcgcctcattttg

SEQ ID NO: 83 - DNA, 20 bp, synthetic construct
  misc_feature 1..20: note = HBV-sgRNA-0080
  source 1..20: mol_type = other DNA
acagagcagaagcggtgtcg

SEQ ID NO: 84 - DNA, 20 bp, synthetic construct
  misc_feature 1..20: note = HBV-sgRNA-0081
  source 1..20: mol_type = other DNA
acagagcagaggcggtgtcg

SEQ ID NO: 85 - DNA, 20 bp, synthetic construct
  misc_feature 1..20: note = HBV-sgRNA-0082
  source 1..20: mol_type = other DNA
acaggaggttggtgagtgat

SEQ ID NO: 86 - DNA, 20 bp, synthetic construct
  misc_feature 1..20: note = HBV-sgRNA-0083
  source 1..20: mol_type = other DNA
acataaggtgggaaacttta

SEQ ID NO: 87 - DNA, 20 bp, synthetic construct
  misc_feature 1..20: note = HBV-sgRNA-0084
  source 1..20: mol_type = other DNA
acatcatttccatggctgct

SEQ ID NO: 88 - DNA, 20 bp, synthetic construct
  misc_feature 1..20: note = HBV-sgRNA-0085
  source 1..20: mol_type = other DNA
acatcgtatccatggctgct

SEQ ID NO: 89 - DNA, 20 bp, synthetic construct
  misc_feature 1..20: note = HBV-sgRNA-0086
  source 1..20: mol_type = other DNA
acatgcatataaaggcatca

SEQ ID NO: 90 - DNA, 20 bp, synthetic construct
  misc_feature 1..20: note = HBV-sgRNA-0087
  source 1..20: mol_type = other DNA
acattgggataaaacctagc

SEQ ID NO: 91 - DNA, 20 bp, synthetic construct
  misc_feature 1..20: note = HBV-sgRNA-0088
  source 1..20: mol_type = other DNA
acattgttcacctcaccata

SEQ ID NO: 92 - DNA, 20 bp, synthetic construct
  misc_feature 1..20: note = HBV-sgRNA-0089
  source 1..20: mol_type = other DNA
acatttcctgtcttactttt

SEQ ID NO: 93 - DNA, 20 bp, synthetic construct
  misc_feature 1..20: note = HBV-sgRNA-0090
  source 1..20: mol_type = other DNA
accaattttcttttgtcttt

SEQ ID NO: 94 - DNA, 20 bp, synthetic construct
  misc_feature 1..20: note = HBV-sgRNA-0091
  source 1..20: mol_type = other DNA
accaggacaagttggaggac

SEQ ID NO: 95 - DNA, 20 bp, synthetic construct
  misc_feature 1..20: note = HBV-sgRNA-0092
  source 1..20: mol_type = other DNA
accaggccgttgccgagcaa

SEQ ID NO: 96 - DNA, 20 bp, synthetic construct
  misc_feature 1..20: note = HBV-sgRNA-0093
  source 1..20: mol_type = other DNA
acccaaagacaaaagaaaat

SEQ ID NO: 97 - DNA, 20 bp, synthetic construct
  misc_feature 1..20: note = HBV-sgRNA-0094
  source 1..20: mol_type = other DNA
accccgcctgtaacacgaga

SEQ ID NO: 98 - DNA, 20 bp, synthetic construct
  misc_feature 1..20: note = HBV-sgRNA-0095
  source 1..20: mol_type = other DNA
accccgcctgtaacacgagc

SEQ ID NO: 99 - DNA, 20 bp, synthetic construct
  misc_feature 1..20: note = HBV-sgRNA-0096
  source 1..20: mol_type = other DNA
acccctgctcgtgttacagg

SEQ ID NO: 100 - DNA, 20 bp, synthetic construct
  misc_feature 1..20: note = HBV-sgRNA-0097
  source 1..20: mol_type = other DNA
accccttctcgtgttacagg

SEQ ID NO: 101 - DNA, 20 bp, synthetic construct
  misc_feature 1..20: note = HBV-sgRNA-0098
  source 1..20: mol_type = other DNA
acccgtctcggggccgtttg

SEQ ID NO: 102 - DNA, 20 bp, synthetic construct
  misc_feature 1..20: note = HBV-sgRNA-0099
  source 1..20: mol_type = other DNA
accctaacaaaacaaagaga

SEQ ID NO: 103 - DNA, 20 bp, synthetic construct
  misc_feature 1..20: note = HBV-sgRNA-0100
  source 1..20: mol_type = other DNA
accctaataaaaccaaacgt

SEQ ID NO: 104 - DNA, 20 bp, synthetic construct
  misc_feature 1..20: note = HBV-sgRNA-0101
  source 1..20: mol_type = other DNA
accctcacaaaacaaaaaga

SEQ ID NO: 105 - DNA, 20 bp, synthetic construct
  misc_feature 1..20: note = HBV-sgRNA-0102
  source 1..20: mol_type = other DNA
acctcaatgttagtattcct

SEQ ID NO: 106 - DNA, 20 bp, synthetic construct
  misc_feature 1..20: note = HBV-sgRNA-0103
  source 1..20: mol_type = other DNA
acctcctttccatggctgct

SEQ ID NO: 107 - DNA, 20 bp, synthetic construct
  misc_feature 1..20: note = HBV-sgRNA-0104
  source 1..20: mol_type = other DNA
acctgaccgttgccgggcaa

SEQ ID NO: 108 - DNA, 20 bp, synthetic construct
  misc_feature 1..20: note = HBV-sgRNA-0105
  source 1..20: mol_type = other DNA
acctgcacaactcctgctca

SEQ ID NO: 109 - DNA, 20 bp, synthetic construct
  misc_feature 1..20: note = HBV-sgRNA-0106
  source 1..20: mol_type = other DNA
acctgcacgattcctgctca

SEQ ID NO: 110 - DNA, 20 bp, synthetic construct
  misc_feature 1..20: note = HBV-sgRNA-0107
  source 1..20: mol_type = other DNA
acctgcatgactactgctca

SEQ ID NO: 111 - DNA, 20 bp, synthetic construct
  misc_feature 1..20: note = HBV-sgRNA-0108
  source 1..20: mol_type = other DNA
acctggccgttgccgggcaa

SEQ ID NO: 112 - DNA, 20 bp, synthetic construct
  misc_feature 1..20: note = HBV-sgRNA-0109
  source 1..20: mol_type = other DNA
acctttggataaaacctagc

SEQ ID NO: 113 - DNA, 20 bp, synthetic construct
  misc_feature 1..20: note = HBV-sgRNA-0110
  source 1..20: mol_type = other DNA
acgatgtatatttgcgggag

SEQ ID NO: 114 - DNA, 20 bp, synthetic construct
  misc_feature 1..20: note = HBV-sgRNA-0111
  source 1..20: mol_type = other DNA
acgcatgcgccgatggccta

SEQ ID NO: 115 - DNA, 20 bp, synthetic construct
  misc_feature 1..20: note = HBV-sgRNA-0112
  source 1..20: mol_type = other DNA
acgcatgcgctgatggccta

SEQ ID NO: 116 - DNA, 20 bp, synthetic construct
  misc_feature 1..20: note = HBV-sgRNA-0113
  source 1..20: mol_type = other DNA
acggcagatgaagaagggga

SEQ ID NO: 117 - DNA, 20 bp, synthetic construct
  misc_feature 1..20: note = HBV-sgRNA-0114
  source 1..20: mol_type = other DNA
actaatgactctagctacct

SEQ ID NO: 118 - DNA, 20 bp, synthetic construct
  misc_feature 1..20: note = HBV-sgRNA-0115
  source 1..20: mol_type = other DNA
actacatactctggataata

SEQ ID NO: 119 - DNA, 20 bp, synthetic construct
  misc_feature 1..20: note = HBV-sgRNA-0116
  source 1..20: mol_type = other DNA
actactaattccctggatgc

SEQ ID NO: 120 - DNA, 20 bp, synthetic construct
  misc_feature 1..20: note = HBV-sgRNA-0117
  source 1..20: mol_type = other DNA
actactaggtctctagatgc

SEQ ID NO: 121 - DNA, 20 bp, synthetic construct
  misc_feature 1..20: note = HBV-sgRNA-0118
  source 1..20: mol_type = other DNA
actactgttgttagacgacg

SEQ ID NO: 122 - DNA, 20 bp, synthetic construct
  misc_feature 1..20: note = HBV-sgRNA-0119
  source 1..20: mol_type = other DNA
actagatgttctggataata

SEQ ID NO: 123 - DNA, 20 bp, synthetic construct
  misc_feature 1..20: note = HBV-sgRNA-0120
  source 1..20: mol_type = other DNA
actcccaccttgttggcgtc

SEQ ID NO: 124 - DNA, 20 bp, synthetic construct
  misc_feature 1..20: note = HBV-sgRNA-0121
  source 1..20: mol_type = other DNA
actgaaggaaagaagtcaga

SEQ ID NO: 125 - DNA, 20 bp, synthetic construct
  misc_feature 1..20: note = HBV-sgRNA-0122
  source 1..20: mol_type = other DNA
actgcatgttcaggataata

SEQ ID NO: 126 - DNA, 20 bp, synthetic construct
  misc_feature 1..20: note = HBV-sgRNA-0123
  source 1..20: mol_type = other DNA
actggatggggcttggccat

SEQ ID NO: 127 - DNA, 20 bp, synthetic construct
  misc_feature 1..20: note = HBV-sgRNA-0124
  source 1..20: mol_type = other DNA
actggctggggcttggtcat

SEQ ID NO: 128 - DNA, 20 bp, synthetic construct
  misc_feature 1..20: note = HBV-sgRNA-0125
  source 1..20: mol_type = other DNA
actggttggggcttggccat

SEQ ID NO: 129 - DNA, 20 bp, synthetic construct
  misc_feature 1..20: note = HBV-sgRNA-0126
  source 1..20: mol_type = other DNA
actgttggggtggagccctc

SEQ ID NO: 130 - DNA, 20 bp, synthetic construct
  misc_feature 1..20: note = HBV-sgRNA-0127
  source 1..20: mol_type = other DNA
acttcatgggatatgtaatt

SEQ ID NO: 131 - DNA, 20 bp, synthetic construct
  misc_feature 1..20: note = HBV-sgRNA-0128
  source 1..20: mol_type = other DNA
acttctctcaattttctagg

SEQ ID NO: 132 - DNA, 20 bp, synthetic construct
  misc_feature 1..20: note = HBV-sgRNA-0129
  source 1..20: mol_type = other DNA
agaaaccgttatagagtatt

SEQ ID NO: 133 - DNA, 20 bp, synthetic construct
  misc_feature 1..20: note = HBV-sgRNA-0130
  source 1..20: mol_type = other DNA
agaaactgtccttgaatatt

SEQ ID NO: 134 - DNA, 20 bp, synthetic construct
  misc_feature 1..20: note = HBV-sgRNA-0131
  source 1..20: mol_type = other DNA
agaaactgttcttgagtatt

SEQ ID NO: 135 - DNA, 20 bp, synthetic construct
  misc_feature 1..20: note = HBV-sgRNA-0132
  source 1..20: mol_type = other DNA
agaagatgaggcatagcagc

SEQ ID NO: 136 - DNA, 20 bp, synthetic construct
  misc_feature 1..20: note = HBV-sgRNA-0133
  source 1..20: mol_type = other DNA
agacaaaggacgtcccgcgc

SEQ ID NO: 137 - DNA, 20 bp, synthetic construct
  misc_feature 1..20: note = HBV-sgRNA-0134
  source 1..20: mol_type = other DNA
agacacatccagcgataacc

SEQ ID NO: 138 - DNA, 20 bp, synthetic construct
  misc_feature 1..20: note = HBV-sgRNA-0135
  source 1..20: mol_type = other DNA
agacacatccagcgatagcc

SEQ ID NO: 139 - DNA, 20 bp, synthetic construct
  misc_feature 1..20: note = HBV-sgRNA-0136
  source 1..20: mol_type = other DNA
agacaccaaatactctataa

SEQ ID NO: 140 - DNA, 20 bp, synthetic construct
  misc_feature 1..20: note = HBV-sgRNA-0137
  source 1..20: mol_type = other DNA
agaccaccgtgaacgcccac

SEQ ID NO: 141 - DNA, 20 bp, synthetic construct
  misc_feature 1..20: note = HBV-sgRNA-0138
  source 1..20: mol_type = other DNA
agaccttcgtctgcgaggcg

SEQ ID NO: 142 - DNA, 20 bp, synthetic construct
  misc_feature 1..20: note = HBV-sgRNA-0139
  source 1..20: mol_type = other DNA
agaccttgggcaacattcgg

SEQ ID NO: 143 - DNA, 20 bp, synthetic construct
  misc_feature 1..20: note = HBV-sgRNA-0140
  source 1..20: mol_type = other DNA
agaccttgggcaagacctgg

SEQ ID NO: 144 - DNA, 20 bp, synthetic construct
  misc_feature 1..20: note = HBV-sgRNA-0141
  source 1..20: mol_type = other DNA
agaccttgggcaggttcctg

SEQ ID NO: 145 - DNA, 20 bp, synthetic construct
  misc_feature 1..20: note = HBV-sgRNA-0142
  source 1..20: mol_type = other DNA
agactgggaggagttggggg

SEQ ID NO: 146 - DNA, 20 bp, synthetic construct
  misc_feature 1..20: note = HBV-sgRNA-0143
  source 1..20: mol_type = other DNA
agactgtgtgtttaaagact

SEQ ID NO: 147 - DNA, 20 bp, synthetic construct
  misc_feature 1..20: note = HBV-sgRNA-0144
  source 1..20: mol_type = other DNA
agactgtgtgtttactgagt

SEQ ID NO: 148 - DNA, 20 bp, synthetic construct
  misc_feature 1..20: note = HBV-sgRNA-0145
  source 1..20: mol_type = other DNA
agactgtttgtttaaagact

SEQ ID NO: 149 - DNA, 20 bp, synthetic construct
  misc_feature 1..20: note = HBV-sgRNA-0146
  source 1..20: mol_type = other DNA
agagaggacaacagagttgt

SEQ ID NO: 150 - DNA, 20 bp, synthetic construct
  misc_feature 1..20: note = HBV-sgRNA-0147
  source 1..20: mol_type = other DNA
agagaggtgcgccccgtggt

SEQ ID NO: 151 - DNA, 20 bp, synthetic construct
  misc_feature 1..20: note = HBV-sgRNA-0148
  source 1..20: mol_type = other DNA
agagctacagcatgggaggt

SEQ ID NO: 152 - DNA, 20 bp, synthetic construct
  misc_feature 1..20: note = HBV-sgRNA-0149
  source 1..20: mol_type = other DNA
agaggcaaatcaggtaggag

SEQ ID NO: 153 - DNA, 20 bp, synthetic construct
  misc_feature 1..20: note = HBV-sgRNA-0150
  source 1..20: mol_type = other DNA
agaggcctgtatttccctgc

SEQ ID NO: 154 - DNA, 20 bp, synthetic construct
  misc_feature 1..20: note = HBV-sgRNA-0151
  source 1..20: mol_type = other DNA
agaggtggagagatgggagt

SEQ ID NO: 155 - DNA, 20 bp, synthetic construct
  misc_feature 1..20: note = HBV-sgRNA-0152
  source 1..20: mol_type = other DNA
agaggtggagataagggagt

SEQ ID NO: 156 - DNA, 20 bp, synthetic construct
  misc_feature 1..20: note = HBV-sgRNA-0153
  source 1..20: mol_type = other DNA
agaggttggtgagtgattgg

SEQ ID NO: 157 - DNA, 20 bp, synthetic construct
  misc_feature 1..20: note = HBV-sgRNA-0154
  source 1..20: mol_type = other DNA
agatctacagcatgggaggt

SEQ ID NO: 158 - DNA, 20 bp, synthetic construct
  misc_feature 1..20: note = HBV-sgRNA-0155
  source 1..20: mol_type = other DNA
agatcttcgtctgcgaggcg

SEQ ID NO: 159 - DNA, 20 bp, synthetic construct
  misc_feature 1..20: note = HBV-sgRNA-0156
  source 1..20: mol_type = other DNA
agatcttgttcccaagaata

SEQ ID NO: 160 - DNA, 20 bp, synthetic construct
  misc_feature 1..20: note = HBV-sgRNA-0157
  source 1..20: mol_type = other DNA
agatgatgggatgggaatac

SEQ ID NO: 161 - DNA, 20 bp, synthetic construct
  misc_feature 1..20: note = HBV-sgRNA-0158
  source 1..20: mol_type = other DNA
agattaaaggtctttgtact

SEQ ID NO: 162 - DNA, 20 bp, synthetic construct
  misc_feature 1..20: note = HBV-sgRNA-0159
  source 1..20: mol_type = other DNA
agattgaatacatgcataca

SEQ ID NO: 163 - DNA, 20 bp, synthetic construct
  misc_feature 1..20: note = HBV-sgRNA-0160
  source 1..20: mol_type = other DNA
agatttgggactgcgaattt

SEQ ID NO: 164 - DNA, 20 bp, synthetic construct
  misc_feature 1..20: note = HBV-sgRNA-0161
  source 1..20: mol_type = other DNA
agccaccagcaggaaaatat

SEQ ID NO: 165 - DNA, 20 bp, synthetic construct
  misc_feature 1..20: note = HBV-sgRNA-0162
  source 1..20: mol_type = other DNA
agccaccagcaggaaagtac

SEQ ID NO: 166 - DNA, 20 bp, synthetic construct
  misc_feature 1..20: note = HBV-sgRNA-0163
  source 1..20: mol_type = other DNA
agccaccagcagggaaatac

SEQ ID NO: 167 - DNA, 20 bp, synthetic construct
  misc_feature 1..20: note = HBV-sgRNA-0164
  source 1..20: mol_type = other DNA
agccccaaacggccccgaga

SEQ ID NO: 168 - DNA, 20 bp, synthetic construct
  misc_feature 1..20: note = HBV-sgRNA-0165
  source 1..20: mol_type = other DNA
agctatgtcaacgttaacat

SEQ ID NO: 169 - DNA, 20 bp, synthetic construct
  misc_feature 1..20: note = HBV-sgRNA-0166
  source 1..20: mol_type = other DNA
agctatgtcaatgttaatat

SEQ ID NO: 170 - DNA, 20 bp, synthetic construct
  misc_feature 1..20: note = HBV-sgRNA-0167
  source 1..20: mol_type = other DNA
agctcttgttcccaagaata

SEQ ID NO: 171 - DNA, 20 bp, synthetic construct
  misc_feature 1..20: note = HBV-sgRNA-0168
  source 1..20: mol_type = other DNA
agctgtgccttgggtggctt

SEQ ID NO: 172 - DNA, 20 bp, synthetic construct
  misc_feature 1..20: note = HBV-sgRNA-0169
  source 1..20: mol_type = other DNA
agcttggaggcttgaacagt

SEQ ID NO: 173 - DNA, 20 bp, synthetic construct
  misc_feature 1..20: note = HBV-sgRNA-0170
  source 1..20: mol_type = other DNA
aggaacatcaaccaccagca

SEQ ID NO: 174 - DNA, 20 bp, synthetic construct
  misc_feature 1..20: note = HBV-sgRNA-0171
  source 1..20: mol_type = other DNA
aggacaaattggaggacaac

SEQ ID NO: 175 - DNA, 20 bp, synthetic construct
  misc_feature 1..20: note = HBV-sgRNA-0172
  source 1..20: mol_type = other DNA
aggacaaattggaggacaag

SEQ ID NO: 176 - DNA, 20 bp, synthetic construct
  misc_feature 1..20: note = HBV-sgRNA-0173
  source 1..20: mol_type = other DNA
aggacaagttggaggacagg

SEQ ID NO: 177 - DNA, 20 bp, synthetic construct
  misc_feature 1..20: note = HBV-sgRNA-0174
  source 1..20: mol_type = other DNA
aggacccctgctcgtgttac

SEQ ID NO: 178 - DNA, 20 bp, synthetic construct
  misc_feature 1..20: note = HBV-sgRNA-0175
  source 1..20: mol_type = other DNA
aggaccccttctcgtgttac

SEQ ID NO: 179 - DNA, 20 bp, synthetic construct
  misc_feature 1..20: note = HBV-sgRNA-0176
  source 1..20: mol_type = other DNA
aggagctggagcattcgggc

SEQ ID NO: 180 - DNA, 20 bp, synthetic construct
  misc_feature 1..20: note = HBV-sgRNA-0177
  source 1..20: mol_type = other DNA
aggaggctgtaggcataaat

SEQ ID NO: 181 - DNA, 20 bp, synthetic construct
  misc_feature 1..20: note = HBV-sgRNA-0178
  source 1..20: mol_type = other DNA
aggaggtgtatttccgagag

SEQ ID NO: 182 - DNA, 20 bp, synthetic construct
  misc_feature 1..20: note = HBV-sgRNA-0179
  source 1..20: mol_type = other DNA
aggagttccgcagtatggat

SEQ ID NO: 183 - DNA, 20 bp, synthetic construct
  misc_feature 1..20: note = HBV-sgRNA-0180
  source 1..20: mol_type = other DNA
aggagttgggggaggagatt

SEQ ID NO: 184 - DNA, 20 bp, synthetic construct
  misc_feature 1..20: note = HBV-sgRNA-0181
  source 1..20: mol_type = other DNA
aggagttgggggaggaggtt

SEQ ID NO: 185 - DNA, 20 bp, synthetic construct
  misc_feature 1..20: note = HBV-sgRNA-0182
  source 1..20: mol_type = other DNA
aggatcctcaaccaccagca

SEQ ID NO: 186 - DNA, 20 bp, synthetic construct
  misc_feature 1..20: note = HBV-sgRNA-0183
  source 1..20: mol_type = other DNA
aggcaagcaattctttgctg

SEQ ID NO: 187 - DNA, 20 bp, synthetic construct
  misc_feature 1..20: note = HBV-sgRNA-0184
  source 1..20: mol_type = other DNA
aggcaagctatcctgtgttg

SEQ ID NO: 188 - DNA, 20 bp, synthetic construct
  misc_feature 1..20: note = HBV-sgRNA-0185
  source 1..20: mol_type = other DNA
aggcaagctattctgtgttg

SEQ ID NO: 189 - DNA, 20 bp, synthetic construct
  misc_feature 1..20: note = HBV-sgRNA-0186
  source 1..20: mol_type = other DNA
agggccctgtactttcctgc

SEQ ID NO: 190 - DNA, 20 bp, synthetic construct
  misc_feature 1..20: note = HBV-sgRNA-0187
  source 1..20: mol_type = other DNA
agggctcactgttcctgaac

SEQ ID NO: 191 - DNA, 20 bp, synthetic construct
  misc_feature 1..20: note = HBV-sgRNA-0188
  source 1..20: mol_type = other DNA
aggggcctatattttcctgc

SEQ ID NO: 192 - DNA, 20 bp, synthetic construct
  misc_feature 1..20: note = HBV-sgRNA-0189
  source 1..20: mol_type = other DNA
agggttcacccctccccatg

SEQ ID NO: 193 - DNA, 20 bp, synthetic construct
  misc_feature 1..20: note = HBV-sgRNA-0190
  source 1..20: mol_type = other DNA
agggtttactgctcctgaac

SEQ ID NO: 194 - DNA, 20 bp, synthetic construct
  misc_feature 1..20: note = HBV-sgRNA-0191
  source 1..20: mol_type = other DNA
agggtttactgttccggaac

SEQ ID NO: 195 - DNA, 20 bp, synthetic construct
  misc_feature 1..20: note = HBV-sgRNA-0192
  source 1..20: mol_type = other DNA
aggtaggagcgggagcattc

SEQ ID NO: 196 - DNA, 20 bp, synthetic construct
  misc_feature 1..20: note = HBV-sgRNA-0193
  source 1..20: mol_type = other DNA
aggtaggagctggagcattc

SEQ ID NO: 197 - DNA, 20 bp, synthetic construct
  misc_feature 1..20: note = HBV-sgRNA-0194
  source 1..20: mol_type = other DNA
aggtctggagcaaacattat

SEQ ID NO: 198 - DNA, 20 bp, synthetic construct
  misc_feature 1..20: note = HBV-sgRNA-0195
  source 1..20: mol_type = other DNA
aggtctggggcaaacctcat

SEQ ID NO: 199 - DNA, 20 bp, synthetic construct
  misc_feature 1..20: note = HBV-sgRNA-0196
  source 1..20: mol_type = other DNA
aggtgcgccccgtggtcggc

SEQ ID NO: 200 - DNA, 20 bp, synthetic construct
  misc_feature 1..20: note = HBV-sgRNA-0197
  source 1..20: mol_type = other DNA
aggtgcgccccgtggtcggt

SEQ ID NO: 201 - DNA, 20 bp, synthetic construct
  misc_feature 1..20: note = HBV-sgRNA-0198
  source 1..20: mol_type = other DNA
aggtgggagtgggagcattc

SEQ ID NO: 202 - DNA, 20 bp, synthetic construct
  misc_feature 1..20: note = HBV-sgRNA-0199
  source 1..20: mol_type = other DNA
aggttaaaggtctttgtact

SEQ ID NO: 203 - DNA, 20 bp, synthetic construct
  misc_feature 1..20: note = HBV-sgRNA-0200
  source 1..20: mol_type = other DNA
aggttaggatagaacctagc

SEQ ID NO: 204 - DNA, 20 bp, synthetic construct
  misc_feature 1..20: note = HBV-sgRNA-0201
  source 1..20: mol_type = other DNA
aggttccacgcacgcgctga

SEQ ID NO: 205 - DNA, 20 bp, synthetic construct
  misc_feature 1..20: note = HBV-sgRNA-0202
  source 1..20: mol_type = other DNA
aggttccacgcatgcgccga

SEQ ID NO: 206 - DNA, 20 bp, synthetic construct
  misc_feature 1..20: note = HBV-sgRNA-0203
  source 1..20: mol_type = other DNA
aggttccacgcatgcgctga

SEQ ID NO: 207 - DNA, 20 bp, synthetic construct
  misc_feature 1..20: note = HBV-sgRNA-0204
  source 1..20: mol_type = other DNA
aggttggggactgcgaattt

SEQ ID NO: 208 - DNA, 20 bp, synthetic construct
  misc_feature 1..20: note = HBV-sgRNA-0205
  source 1..20: mol_type = other DNA
aggtttggtacagcaacagg

SEQ ID NO: 209 - DNA, 20 bp, synthetic construct
  misc_feature 1..20: note = HBV-sgRNA-0206
  source 1..20: mol_type = other DNA
aggttttgtacagcaacaag

SEQ ID NO: 210 - DNA, 20 bp, synthetic construct
  misc_feature 1..20: note = HBV-sgRNA-0207
  source 1..20: mol_type = other DNA
aggttttgtacagcaacatg

SEQ ID NO: 211 - DNA, 20 bp, synthetic construct
  misc_feature 1..20: note = HBV-sgRNA-0208
  source 1..20: mol_type = other DNA
agtcccaagcgaccccgaga

SEQ ID NO: 212 - DNA, 20 bp, synthetic construct
  misc_feature 1..20: note = HBV-sgRNA-0209
  source 1..20: mol_type = other DNA
agtcccaagcggccccgaga

SEQ ID NO: 213 - DNA, 20 bp, synthetic construct
  misc_feature 1..20: note = HBV-sgRNA-0210
  source 1..20: mol_type = other DNA
agtcctcttatgcaagacct

SEQ ID NO: 214 - DNA, 20 bp, synthetic construct
  misc_feature 1..20: note = HBV-sgRNA-0211
  source 1..20: mol_type = other DNA
agtcctcttatgtaagacct

SEQ ID NO: 215 - DNA, 20 bp, synthetic construct
  misc_feature 1..20: note = HBV-sgRNA-0212
  source 1..20: mol_type = other DNA
agtctttgaagtatgcctca

SEQ ID NO: 216 - DNA, 20 bp, synthetic construct
  misc_feature 1..20: note = HBV-sgRNA-0213
  source 1..20: mol_type = other DNA
agttatgtcaacactaatat

SEQ ID NO: 217 - DNA, 20 bp, synthetic construct
  misc_feature 1..20: note = HBV-sgRNA-0214
  source 1..20: mol_type = other DNA
agttgatgaatctagctacc

SEQ ID NO: 218 - DNA, 20 bp, synthetic construct
  misc_feature 1..20: note = HBV-sgRNA-0215
  source 1..20: mol_type = other DNA
agttgatgaatctggccacc

SEQ ID NO: 219 - DNA, 20 bp, synthetic construct
  misc_feature 1..20: note = HBV-sgRNA-0216
  source 1..20: mol_type = other DNA
agttgtccttgtgcgggttg

SEQ ID NO: 220 - DNA, 20 bp, synthetic construct
  misc_feature 1..20: note = HBV-sgRNA-0217
  source 1..20: mol_type = other DNA
ataaccacattgtgtaaatg

SEQ ID NO: 221 - DNA, 20 bp, synthetic construct
  misc_feature 1..20: note = HBV-sgRNA-0218
  source 1..20: mol_type = other DNA
ataactgaaagccaaacagt

SEQ ID NO: 222 - DNA, 20 bp, synthetic construct
  misc_feature 1..20: note = HBV-sgRNA-0219
  source 1..20: mol_type = other DNA
ataactgaaagccagacagt

SEQ ID NO: 223 - DNA, 20 bp, synthetic construct
  misc_feature 1..20: note = HBV-sgRNA-0220
  source 1..20: mol_type = other DNA
ataaggtgggaaactttacg

SEQ ID NO: 224 - DNA, 20 bp, synthetic construct
  misc_feature 1..20: note = HBV-sgRNA-0221
  source 1..20: mol_type = other DNA
ataaggtgggaaactttact

SEQ ID NO: 225 - DNA, 20 bp, synthetic construct
  misc_feature 1..20: note = HBV-sgRNA-0222
  source 1..20: mol_type = other DNA
ataccgcctcagctctgtat

SEQ ID NO: 226 - DNA, 20 bp, synthetic construct
  misc_feature 1..20: note = HBV-sgRNA-0223
  source 1..20: mol_type = other DNA
atagaaggaaagaagtcaga

SEQ ID NO: 227 - DNA, 20 bp, synthetic construct
  misc_feature 1..20: note = HBV-sgRNA-0224
  source 1..20: mol_type = other DNA
atagagtatttggtgtcttt

SEQ ID NO: 228 - DNA, 20 bp, synthetic construct
  misc_feature 1..20: note = HBV-sgRNA-0225
  source 1..20: mol_type = other DNA
atagatgtaagcaatttgtg

SEQ ID NO: 229 - DNA, 20 bp, synthetic construct
  misc_feature 1..20: note = HBV-sgRNA-0226
  source 1..20: mol_type = other DNA
atagccacattgtgtaaaag

SEQ ID NO: 230 - DNA, 20 bp, synthetic construct
  misc_feature 1..20: note = HBV-sgRNA-0227
  source 1..20: mol_type = other DNA
atagctgactactaattccc

SEQ ID NO: 231 - DNA, 20 bp, synthetic construct
  misc_feature 1..20: note = HBV-sgRNA-0228
  source 1..20: mol_type = other DNA
ataggccatcagcgcatgcg

SEQ ID NO: 232 - DNA, 20 bp, synthetic construct
  misc_feature 1..20: note = HBV-sgRNA-0229
  source 1..20: mol_type = other DNA
ataggccatcggcgcatgcg

SEQ ID NO: 233 - DNA, 20 bp, synthetic construct
  misc_feature 1..20: note = HBV-sgRNA-0230
  source 1..20: mol_type = other DNA
atatccacattgcgtgaaag

SEQ ID NO: 234 - DNA, 20 bp, synthetic construct
  misc_feature 1..20: note = HBV-sgRNA-0231
  source 1..20: mol_type = other DNA
atatggatgatgtggtattg

SEQ ID NO: 235 - DNA, 20 bp, synthetic construct
  misc_feature 1..20: note = HBV-sgRNA-0232
  source 1..20: mol_type = other DNA
atatggatgatgtggttttg

SEQ ID NO: 236 - DNA, 20 bp, synthetic construct
  misc_feature 1..20: note = HBV-sgRNA-0233
  source 1..20: mol_type = other DNA
atatggtgacccacaaaatg

SEQ ID NO: 237 - DNA, 20 bp, synthetic construct
  misc_feature 1..20: note = HBV-sgRNA-0234
  source 1..20: mol_type = other DNA
atatggtgacccgcaaaatg

SEQ ID NO: 238 - DNA, 20 bp, synthetic construct
  misc_feature 1..20: note = HBV-sgRNA-0235
  source 1..20: mol_type = other DNA
atcccatcatcctgggcttt

SEQ ID NO: 239 - DNA, 20 bp, synthetic construct
  misc_feature 1..20: note = HBV-sgRNA-0236
  source 1..20: mol_type = other DNA
atcccgcggacgacccctct

SEQ ID NO: 240 - DNA, 20 bp, synthetic construct
  misc_feature 1..20: note = HBV-sgRNA-0237
  source 1..20: mol_type = other DNA
atcccgcggacgacccgtct

SEQ ID NO: 241 - DNA, 20 bp, synthetic construct
  misc_feature 1..20: note = HBV-sgRNA-0238
  source 1..20: mol_type = other DNA
atcccttggactcataaggt

SEQ ID NO: 242 - DNA, 20 bp, synthetic construct
  misc_feature 1..20: note = HBV-sgRNA-0239
  source 1..20: mol_type = other DNA
atcctgcggacgacccttct

SEQ ID NO: 243 - DNA, 20 bp, synthetic construct
  misc_feature 1..20: note = HBV-sgRNA-0240
  source 1..20: mol_type = other DNA
atcgacccttataaagaatt

SEQ ID NO: 244 - DNA, 20 bp, synthetic construct
  misc_feature 1..20: note = HBV-sgRNA-0241
  source 1..20: mol_type = other DNA
atctcaatgttagtatccct

SEQ ID NO: 245 - DNA, 20 bp, synthetic construct
  misc_feature 1..20: note = HBV-sgRNA-0242
  source 1..20: mol_type = other DNA
atctcaatgttagtattcct

SEQ ID NO: 246 - DNA, 20 bp, synthetic construct
  misc_feature 1..20: note = HBV-sgRNA-0243
  source 1..20: mol_type = other DNA
atcttgcagagtttggtgaa

SEQ ID NO: 247 - DNA, 20 bp, synthetic construct
  misc_feature 1..20: note = HBV-sgRNA-0244
  source 1..20: mol_type = other DNA
atgaatctagctacctgggt

SEQ ID NO: 248 - DNA, 20 bp, synthetic construct
  misc_feature 1..20: note = HBV-sgRNA-0245
  source 1..20: mol_type = other DNA
atgaatctggccacctgggt

SEQ ID NO: 249 - DNA, 20 bp, synthetic construct
  misc_feature 1..20: note = HBV-sgRNA-0246
  source 1..20: mol_type = other DNA
atgaccaagccccagccagt

SEQ ID NO: 250 - DNA, 20 bp, synthetic construct
  misc_feature 1..20: note = HBV-sgRNA-0247
  source 1..20: mol_type = other DNA
atgactctagctacctgggt

SEQ ID NO: 251 - DNA, 20 bp, synthetic construct
  misc_feature 1..20: note = HBV-sgRNA-0248
  source 1..20: mol_type = other DNA
atgatcggggaagaatccca

SEQ ID NO: 252 - DNA, 20 bp, synthetic construct
  misc_feature 1..20: note = HBV-sgRNA-0249
  source 1..20: mol_type = other DNA
atgctccaaattctttatac

SEQ ID NO: 253 - DNA, 20 bp, synthetic construct
  misc_feature 1..20: note = HBV-sgRNA-0250
  source 1..20: mol_type = other DNA
atggaaatgatgtatacttg

SEQ ID NO: 254 - DNA, 20 bp, synthetic construct
  misc_feature 1..20: note = HBV-sgRNA-0251
  source 1..20: mol_type = other DNA
atggatacgatgtatatttg

SEQ ID NO: 255 - DNA, 20 bp, synthetic construct
  misc_feature 1..20: note = HBV-sgRNA-0252
  source 1..20: mol_type = other DNA
atggccaagccccaaccagt

SEQ ID NO: 256 - DNA, 20 bp, synthetic construct
  misc_feature 1..20: note = HBV-sgRNA-0253
  source 1..20: mol_type = other DNA
atggccaagccccatccagt

SEQ ID NO: 257 - DNA, 20 bp, synthetic construct
  misc_feature 1..20: note = HBV-sgRNA-0254
  source 1..20: mol_type = other DNA
atgggccatcagcgcgtgcg

SEQ ID NO: 258 - DNA, 20 bp, synthetic construct
  misc_feature 1..20: note = HBV-sgRNA-0255
  source 1..20: mol_type = other DNA
atgttctccatgttcagcgc

SEQ ID NO: 259 - DNA, 20 bp, synthetic construct
  misc_feature 1..20: note = HBV-sgRNA-0256
  source 1..20: mol_type = other DNA
atgttctccatgttcggtac

SEQ ID NO: 260 - DNA, 20 bp, synthetic construct
  misc_feature 1..20: note = HBV-sgRNA-0257
  source 1..20: mol_type = other DNA
atgttgctgtacaaaaccta

SEQ ID NO: 261 - DNA, 20 bp, synthetic construct
  misc_feature 1..20: note = HBV-sgRNA-0258
  source 1..20: mol_type = other DNA
attccttggacacataaggt

SEQ ID NO: 262 - DNA, 20 bp, synthetic construct
  misc_feature 1..20: note = HBV-sgRNA-0259
  source 1..20: mol_type = other DNA
attccttggactcataaggt

SEQ ID NO: 263 - DNA, 20 bp, synthetic construct
  misc_feature 1..20: note = HBV-sgRNA-0260
  source 1..20: mol_type = other DNA
attcttccccgatcatcagt

SEQ ID NO: 264 - DNA, 20 bp, synthetic construct
  misc_feature 1..20: note = HBV-sgRNA-0261
  source 1..20: mol_type = other DNA
attctttcccgaccaccagt

SEQ ID NO: 265 - DNA, 20 bp, synthetic construct
  misc_feature 1..20: note = HBV-sgRNA-0262
  source 1..20: mol_type = other DNA
attctttcccgatcaccagt

SEQ ID NO: 266 - DNA, 20 bp, synthetic construct
  misc_feature 1..20: note = HBV-sgRNA-0263
  source 1..20: mol_type = other DNA
attgacccgtataaagaatt

SEQ ID NO: 267 - DNA, 20 bp, synthetic construct
  misc_feature 1..20: note = HBV-sgRNA-0264
  source 1..20: mol_type = other DNA
attggtaacagcggcataaa

SEQ ID NO: 268 - DNA, 20 bp, synthetic construct
  misc_feature 1..20: note = HBV-sgRNA-0265
  source 1..20: mol_type = other DNA
attggtaacagcggtaaaaa

SEQ ID NO: 269 - DNA, 20 bp, synthetic construct
  misc_feature 1..20: note = HBV-sgRNA-0266
  source 1..20: mol_type = other DNA
attggtaatagaggtaaaaa

SEQ ID NO: 270 - DNA, 20 bp, synthetic construct
  misc_feature 1..20: note = HBV-sgRNA-0267
  source 1..20: mol_type = other DNA
atttgctgtgtttgctctga

SEQ ID NO: 271 - DNA, 20 bp, synthetic construct
  misc_feature 1..20: note = HBV-sgRNA-0268
  source 1..20: mol_type = other DNA
atttggaagacccagcatcc

SEQ ID NO: 272 - DNA, 20 bp, synthetic construct
  misc_feature 1..20: note = HBV-sgRNA-0269
  source 1..20: mol_type = other DNA
atttggaagatccagcatcc

SEQ ID NO: 273 - DNA, 20 bp, synthetic construct
  misc_feature 1..20: note = HBV-sgRNA-0270
  source 1..20: mol_type = other DNA
atttggtatcttttggagtg

SEQ ID NO: 274 - DNA, 20 bp, synthetic construct
  misc_feature 1..20: note = HBV-sgRNA-0271
  source 1..20: mol_type = other DNA
atttggtgtctttcggagtg

SEQ ID NO: 275 - DNA, 20 bp, synthetic construct
  misc_feature 1..20: note = HBV-sgRNA-0272
  source 1..20: mol_type = other DNA
atttggtgtcttttggagtg

SEQ ID NO: 276 - DNA, 20 bp, synthetic construct
  misc_feature 1..20: note = HBV-sgRNA-0273
  source 1..20: mol_type = other DNA
caaaagaaaattggtaacag

SEQ ID NO: 277 - DNA, 20 bp, synthetic construct
  misc_feature 1..20: note = HBV-sgRNA-0274
  source 1..20: mol_type = other DNA
caaaagaaaattggtaatag

SEQ ID NO: 278 - DNA, 20 bp, synthetic construct
  misc_feature 1..20: note = HBV-sgRNA-0275
  source 1..20: mol_type = other DNA
caaaagacaccaaatattca

SEQ ID NO: 279 - DNA, 20 bp, synthetic construct
  misc_feature 1..20: note = HBV-sgRNA-0276
  source 1..20: mol_type = other DNA
caaaagaccgccgtgtggtg

SEQ ID NO: 280 - DNA, 20 bp, synthetic construct
  misc_feature 1..20: note = HBV-sgRNA-0277
  source 1..20: mol_type = other DNA
caaaaggcctccgtgcggtg

SEQ ID NO: 281 - DNA, 20 bp, synthetic construct
  misc_feature 1..20: note = HBV-sgRNA-0278
  source 1..20: mol_type = other DNA
caaacacagcaaatccagat

SEQ ID NO: 282 - DNA, 20 bp, synthetic construct
  misc_feature 1..20: note = HBV-sgRNA-0279
  source 1..20: mol_type = other DNA
caaagaattgtgggtctttt

SEQ ID NO: 283 - DNA, 20 bp, synthetic construct
  misc_feature 1..20: note = HBV-sgRNA-0280
  source 1..20: mol_type = other DNA
caaatatttaccattggata

SEQ ID NO: 284 - DNA, 20 bp, synthetic construct
  misc_feature 1..20: note = HBV-sgRNA-0281
  source 1..20: mol_type = other DNA
caaattacttcccacccagg

SEQ ID NO: 285 - DNA, 20 bp, synthetic construct
  misc_feature 1..20: note = HBV-sgRNA-0282
  source 1..20: mol_type = other DNA
caaattggaggacaacaggt

SEQ ID NO: 286 - DNA, 20 bp, synthetic construct
  misc_feature 1..20: note = HBV-sgRNA-0283
  source 1..20: mol_type = other DNA
caaattggaggacaagaggt

SEQ ID NO: 287 - DNA, 20 bp, synthetic construct
  misc_feature 1..20: note = HBV-sgRNA-0284
  source 1..20: mol_type = other DNA
caacaaggatcactggccag

SEQ ID NO: 288 - DNA, 20 bp, synthetic construct
  misc_feature 1..20: note = HBV-sgRNA-0285
  source 1..20: mol_type = other DNA
caacagtcccccatggggag

SEQ ID NO: 289 - DNA, 20 bp, synthetic construct
  misc_feature 1..20: note = HBV-sgRNA-0286
  source 1..20: mol_type = other DNA
caacattcggtgggcgttca

SEQ ID NO: 290 - DNA, 20 bp, synthetic construct
  misc_feature 1..20: note = HBV-sgRNA-0287
  source 1..20: mol_type = other DNA
caacgaattgtgggtctttt

SEQ ID NO: 291 - DNA, 20 bp, synthetic construct
  misc_feature 1..20: note = HBV-sgRNA-0288
  source 1..20: mol_type = other DNA
caactcaaacaatccagatt

SEQ ID NO: 292 - DNA, 20 bp, synthetic construct
  misc_feature 1..20: note = HBV-sgRNA-0289
  source 1..20: mol_type = other DNA
caactcagaaagtccagatt

SEQ ID NO: 293 - DNA, 20 bp, synthetic construct
  misc_feature 1..20: note = HBV-sgRNA-0290
  source 1..20: mol_type = other DNA
caactggccggacgccaaca

SEQ ID NO: 294 - DNA, 20 bp, synthetic construct
  misc_feature 1..20: note = HBV-sgRNA-0291
  source 1..20: mol_type = other DNA
caacttgtcctggttatcgc

SEQ ID NO: 295 - DNA, 20 bp, synthetic construct
  misc_feature 1..20: note = HBV-sgRNA-0292
  source 1..20: mol_type = other DNA
caagacctggtgggcgttca

SEQ ID NO: 296 - DNA, 20 bp, synthetic construct
  misc_feature 1..20: note = HBV-sgRNA-0293
  source 1..20: mol_type = other DNA
caagcctccaagctgtgcct

SEQ ID NO: 297 - DNA, 20 bp, synthetic construct
  misc_feature 1..20: note = HBV-sgRNA-0294
  source 1..20: mol_type = other DNA
caagtgcagtttccgtccga

SEQ ID NO: 298 - DNA, 20 bp, synthetic construct
  misc_feature 1..20: note = HBV-sgRNA-0295
  source 1..20: mol_type = other DNA
caagttggaggacaggaggt

SEQ ID NO: 299 - DNA, 20 bp, synthetic construct
  misc_feature 1..20: note = HBV-sgRNA-0296
  source 1..20: mol_type = other DNA
caatcaataggcctgttaat

SEQ ID NO: 300 - DNA, 20 bp, synthetic construct
  misc_feature 1..20: note = HBV-sgRNA-0297
  source 1..20: mol_type = other DNA
caatcaataggcctgtttac

SEQ ID NO: 301 - DNA, 20 bp, synthetic construct
  misc_feature 1..20: note = HBV-sgRNA-0298
  source 1..20: mol_type = other DNA
caatcaataggtctatttac

SEQ ID NO: 302 - DNA, 20 bp, synthetic construct
  misc_feature 1..20: note = HBV-sgRNA-0299
  source 1..20: mol_type = other DNA
caatttgtcctggctatcgc

SEQ ID NO: 303 - DNA, 20 bp, synthetic construct
  misc_feature 1..20: note = HBV-sgRNA-0300
  source 1..20: mol_type = other DNA
caatttgtcctggttatcgc

SEQ ID NO: 304 - DNA, 20 bp, synthetic construct
  misc_feature 1..20: note = HBV-sgRNA-0301
  source 1..20: mol_type = other DNA
cacacggcggtcttttgggg

SEQ ID NO: 305 - DNA, 20 bp, synthetic construct
  misc_feature 1..20: note = HBV-sgRNA-0302
  source 1..20: mol_type = other DNA
cacagaaaggccttgtaagt

SEQ ID NO: 306 - DNA, 20 bp, synthetic construct
  misc_feature 1..20: note = HBV-sgRNA-0303
  source 1..20: mol_type = other DNA
cacagagtctagactcgtgg

SEQ ID NO: 307 - DNA, 20 bp, synthetic construct
  misc_feature 1..20: note = HBV-sgRNA-0304
  source 1..20: mol_type = other DNA
cacatagcgcctcattttgt

SEQ ID NO: 308 - DNA, 20 bp, synthetic construct
  misc_feature 1..20: note = HBV-sgRNA-0305
  source 1..20: mol_type = other DNA
cacatttcctgtcttacttt

SEQ ID NO: 309 - DNA, 20 bp, synthetic construct
  misc_feature 1..20: note = HBV-sgRNA-0306
  source 1..20: mol_type = other DNA
cacatttcttgtctcacttt

SEQ ID NO: 310 - DNA, 20 bp, synthetic construct
  misc_feature 1..20: note = HBV-sgRNA-0307
  source 1..20: mol_type = other DNA
cacattttttgataatgtct

SEQ ID NO: 311 - DNA, 20 bp, synthetic construct
  misc_feature 1..20: note = HBV-sgRNA-0308
  source 1..20: mol_type = other DNA
caccacacggcggtcttttg

SEQ ID NO: 312 - DNA, 20 bp, synthetic construct
  misc_feature 1..20: note = HBV-sgRNA-0309
  source 1..20: mol_type = other DNA
caccacgagtctagactctg

SEQ ID NO: 313 - DNA, 20 bp, synthetic construct
  misc_feature 1..20: note = HBV-sgRNA-0310
  source 1..20: mol_type = other DNA
caccagttggaccctgcgtt

SEQ ID NO: 314 - DNA, 20 bp, synthetic construct
  misc_feature 1..20: note = HBV-sgRNA-0311
  source 1..20: mol_type = other DNA
caccccaaaagaccgccgtg

SEQ ID NO: 315 - DNA, 20 bp, synthetic construct
  misc_feature 1..20: note = HBV-sgRNA-0312
  source 1..20: mol_type = other DNA
caccccaaaaggcctccgtg

SEQ ID NO: 316 - DNA, 20 bp, synthetic construct
  misc_feature 1..20: note = HBV-sgRNA-0313
  source 1..20: mol_type = other DNA
caccccaacagtcccccatg

SEQ ID NO: 317 - DNA, 20 bp, synthetic construct
  misc_feature 1..20: note = HBV-sgRNA-0314
  source 1..20: mol_type = other DNA
caccgcacggaggccttttg

SEQ ID NO: 318 - DNA, 20 bp, synthetic construct
  misc_feature 1..20: note = HBV-sgRNA-0315
  source 1..20: mol_type = other DNA
caccgcctctgctctgtatc

SEQ ID NO: 319 - DNA, 20 bp, synthetic construct
  misc_feature 1..20: note = HBV-sgRNA-0316
  source 1..20: mol_type = other DNA
caccgcttctgctctgtatc

SEQ ID NO: 320 - DNA, 20 bp, synthetic construct
  misc_feature 1..20: note = HBV-sgRNA-0317
  source 1..20: mol_type = other DNA
cacctcaccatacagcactc

SEQ ID NO: 321 - DNA, 20 bp, synthetic construct
  misc_feature 1..20: note = HBV-sgRNA-0318
  source 1..20: mol_type = other DNA
cacctcaccatacggcactc

SEQ ID NO: 322 - DNA, 20 bp, synthetic construct
  misc_feature 1..20: note = HBV-sgRNA-0319
  source 1..20: mol_type = other DNA
cacctcaccatactgcactc

SEQ ID NO: 323 - DNA, 20 bp, synthetic construct
  misc_feature 1..20: note = HBV-sgRNA-0320
  source 1..20: mol_type = other DNA
cacctggccagacgccaaca

SEQ ID NO: 324 - DNA, 20 bp, synthetic construct
  misc_feature 1..20: note = HBV-sgRNA-0321
  source 1..20: mol_type = other DNA
cacctgggtgggaagtaatt

SEQ ID NO: 325 - DNA, 20 bp, synthetic construct
  misc_feature 1..20: note = HBV-sgRNA-0322
  source 1..20: mol_type = other DNA
cacgcagcgcctcattttgt

SEQ ID NO: 326 - DNA, 20 bp, synthetic construct
  misc_feature 1..20: note = HBV-sgRNA-0323
  source 1..20: mol_type = other DNA
cacgtagcgcctcattttgc

SEQ ID NO: 327 - DNA, 20 bp, synthetic construct
  misc_feature 1..20: note = HBV-sgRNA-0324
  source 1..20: mol_type = other DNA
cactggctggggcttggtca

SEQ ID NO: 328 - DNA, 20 bp, synthetic construct
  misc_feature 1..20: note = HBV-sgRNA-0325
  source 1..20: mol_type = other DNA
cactttctcgccaacttaca

SEQ ID NO: 329 - DNA, 20 bp, synthetic construct
  misc_feature 1..20: note = HBV-sgRNA-0326
  source 1..20: mol_type = other DNA
cagaattgtcagtcccgatg

SEQ ID NO: 330 - DNA, 20 bp, synthetic construct
  misc_feature 1..20: note = HBV-sgRNA-0327
  source 1..20: mol_type = other DNA
cagagacagtattctgagca

SEQ ID NO: 331 - DNA, 20 bp, synthetic construct
  misc_feature 1..20: note = HBV-sgRNA-0328
  source 1..20: mol_type = other DNA
cagagcttggtggaatgttg

SEQ ID NO: 332 - DNA, 20 bp, synthetic construct
  misc_feature 1..20: note = HBV-sgRNA-0329
  source 1..20: mol_type = other DNA
cagagtttggtgaaaggttg

SEQ ID NO: 333 - DNA, 20 bp, synthetic construct
  misc_feature 1..20: note = HBV-sgRNA-0330
  source 1..20: mol_type = other DNA
cagatactgtttacttagaa

SEQ ID NO: 334 - DNA, 20 bp, synthetic construct
  misc_feature 1..20: note = HBV-sgRNA-0331
  source 1..20: mol_type = other DNA
cagatattgtttacacagaa

SEQ ID NO: 335 - DNA, 20 bp, synthetic construct
  misc_feature 1..20: note = HBV-sgRNA-0332
  source 1..20: mol_type = other DNA
cagatgagaaggcacagacg

SEQ ID NO: 336 - DNA, 20 bp, synthetic construct
  misc_feature 1..20: note = HBV-sgRNA-0333
  source 1..20: mol_type = other DNA
cagcgataaccaggacaaat

SEQ ID NO: 337 - DNA, 20 bp, synthetic construct
  misc_feature 1..20: note = HBV-sgRNA-0334
  source 1..20: mol_type = other DNA
cagcgataaccaggacaagt

SEQ ID NO: 338 - DNA, 20 bp, synthetic construct
  misc_feature 1..20: note = HBV-sgRNA-0335
  source 1..20: mol_type = other DNA
cagcgatagccaggacaaat

SEQ ID NO: 339 - DNA, 20 bp, synthetic construct
  misc_feature 1..20: note = HBV-sgRNA-0336
  source 1..20: mol_type = other DNA
cagctatgtcaacgttaaca

SEQ ID NO: 340 - DNA, 20 bp, synthetic construct
  misc_feature 1..20: note = HBV-sgRNA-0337
  source 1..20: mol_type = other DNA
cagctatgtcaatgttaata

SEQ ID NO: 341 - DNA, 20 bp, synthetic construct
  misc_feature 1..20: note = HBV-sgRNA-0338
  source 1..20: mol_type = other DNA
cagcttgtttcgctcgcagc

SEQ ID NO: 342 - DNA, 20 bp, synthetic construct
  misc_feature 1..20: note = HBV-sgRNA-0339
  source 1..20: mol_type = other DNA
caggcaagcaattctttgct

SEQ ID NO: 343 - DNA, 20 bp, synthetic construct
  misc_feature 1..20: note = HBV-sgRNA-0340
  source 1..20: mol_type = other DNA
caggcaagctatcctgtgtt

SEQ ID NO: 344 - DNA, 20 bp, synthetic construct
  misc_feature 1..20: note = HBV-sgRNA-0341
  source 1..20: mol_type = other DNA
caggcaagctattctgtgtt

SEQ ID NO: 345 - DNA, 20 bp, synthetic construct
  misc_feature 1..20: note = HBV-sgRNA-0342
  source 1..20: mol_type = other DNA
caggccgttgccgagcaacg

SEQ ID NO: 346 - DNA, 20 bp, synthetic construct
  misc_feature 1..20: note = HBV-sgRNA-0343
  source 1..20: mol_type = other DNA
cagggtccaactgatgatcg

SEQ ID NO: 347 - DNA, 20 bp, synthetic construct
  misc_feature 1..20: note = HBV-sgRNA-0344
  source 1..20: mol_type = other DNA
cagggttcacccctccccat

SEQ ID NO: 348 - DNA, 20 bp, synthetic construct
  misc_feature 1..20: note = HBV-sgRNA-0345
  source 1..20: mol_type = other DNA
caggtaggagcgggagcatt

SEQ ID NO: 349 - DNA, 20 bp, synthetic construct
  misc_feature 1..20: note = HBV-sgRNA-0346
  source 1..20: mol_type = other DNA
caggtattgtttacacagaa

SEQ ID NO: 350 - DNA, 20 bp, synthetic construct
  misc_feature 1..20: note = HBV-sgRNA-0347
  source 1..20: mol_type = other DNA
caggtgcaatttccgtccga

SEQ ID NO: 351 - DNA, 20 bp, synthetic construct
  misc_feature 1..20: note = HBV-sgRNA-0348
  source 1..20: mol_type = other DNA
caggtgcagtttccgtccgt

SEQ ID NO: 352 - DNA, 20 bp, synthetic construct
  misc_feature 1..20: note = HBV-sgRNA-0349
  source 1..20: mol_type = other DNA
caggttcctgtgggcgttca

SEQ ID NO: 353 - DNA, 20 bp, synthetic construct
  misc_feature 1..20: note = HBV-sgRNA-0350
  source 1..20: mol_type = other DNA
cagttatgtcaacactaata

SEQ ID NO: 354 - DNA, 20 bp, synthetic construct
  misc_feature 1..20: note = HBV-sgRNA-0351
  source 1..20: mol_type = other DNA
cataaggtgggaaactttac

SEQ ID NO: 355 - DNA, 20 bp, synthetic construct
  misc_feature 1..20: note = HBV-sgRNA-0352
  source 1..20: mol_type = other DNA
cataaggtggggaactttac

SEQ ID NO: 356 - DNA, 20 bp, synthetic construct
  misc_feature 1..20: note = HBV-sgRNA-0353
  source 1..20: mol_type = other DNA
catcttcttgttggttcttc

SEQ ID NO: 357 - DNA, 20 bp, synthetic construct
  misc_feature 1..20: note = HBV-sgRNA-0354
  source 1..20: mol_type = other DNA
catgaccaagccccagccag

SEQ ID NO: 358 - DNA, 20 bp, synthetic construct
  misc_feature 1..20: note = HBV-sgRNA-0355
  source 1..20: mol_type = other DNA
cattcggtgggcgttcacgg

SEQ ID NO: 359 - DNA, 20 bp, synthetic construct
  misc_feature 1..20: note = HBV-sgRNA-0356
  source 1..20: mol_type = other DNA
catttgttcagtggttcgta

SEQ ID NO: 360 - DNA, 20 bp, synthetic construct
  misc_feature 1..20: note = HBV-sgRNA-0357
  source 1..20: mol_type = other DNA
ccaaaagaccgccgtgtggt

SEQ ID NO: 361 - DNA, 20 bp, synthetic construct
  misc_feature 1..20: note = HBV-sgRNA-0358
  source 1..20: mol_type = other DNA
ccaaaaggcctccgtgcggt

SEQ ID NO: 362 - DNA, 20 bp, synthetic construct
  misc_feature 1..20: note = HBV-sgRNA-0359
  source 1..20: mol_type = other DNA
ccaaacctcgaaaaggcatg

SEQ ID NO: 363 - DNA, 20 bp, synthetic construct
  misc_feature 1..20: note = HBV-sgRNA-0360
  source 1..20: mol_type = other DNA
ccaaacctcgacaaggcatg

SEQ ID NO: 364 - DNA, 20 bp, synthetic construct
  misc_feature 1..20: note = HBV-sgRNA-0361
  source 1..20: mol_type = other DNA
ccaacagtcccccatgggga

SEQ ID NO: 365 - DNA, 20 bp, synthetic construct
  misc_feature 1..20: note = HBV-sgRNA-0362
  source 1..20: mol_type = other DNA
ccaactcaaacaatccagat

SEQ ID NO: 366 - DNA, 20 bp, synthetic construct
  misc_feature 1..20: note = HBV-sgRNA-0363
  source 1..20: mol_type = other DNA
ccaactcagaaagtccagat

SEQ ID NO: 367 - DNA, 20 bp, synthetic construct
  misc_feature 1..20: note = HBV-sgRNA-0364
  source 1..20: mol_type = other DNA
ccaatctggactttctgagt

SEQ ID NO: 368 - DNA, 20 bp, synthetic construct
  misc_feature 1..20: note = HBV-sgRNA-0365
  source 1..20: mol_type = other DNA
ccaatctggattgtttgagt

SEQ ID NO: 369 - DNA, 20 bp, synthetic construct
  misc_feature 1..20: note = HBV-sgRNA-0366
  source 1..20: mol_type = other DNA
ccaccaatcgccagacagga

SEQ ID NO: 370 - DNA, 20 bp, synthetic construct
  misc_feature 1..20: note = HBV-sgRNA-0367
  source 1..20: mol_type = other DNA
ccaccaatcggcagtcagga

SEQ ID NO: 371 - DNA, 20 bp, synthetic construct
  misc_feature 1..20: note = HBV-sgRNA-0368
  source 1..20: mol_type = other DNA
ccaccacacggcggtctttt

SEQ ID NO: 372 - DNA, 20 bp, synthetic construct
  misc_feature 1..20: note = HBV-sgRNA-0369
  source 1..20: mol_type = other DNA
ccacccaaggcacagcttgg

SEQ ID NO: 373 - DNA, 20 bp, synthetic construct
  misc_feature 1..20: note = HBV-sgRNA-0370
  source 1..20: mol_type = other DNA
ccaccccaacagtcccccat

SEQ ID NO: 374 - DNA, 20 bp, synthetic construct
  misc_feature 1..20: note = HBV-sgRNA-0371
  source 1..20: mol_type = other DNA
ccaccgcacggaggcctttt

SEQ ID NO: 375 - DNA, 20 bp, synthetic construct
  misc_feature 1..20: note = HBV-sgRNA-0372
  source 1..20: mol_type = other DNA
ccaggccgttgccgagcaac

SEQ ID NO: 376 - DNA, 20 bp, synthetic construct
  misc_feature 1..20: note = HBV-sgRNA-0373
  source 1..20: mol_type = other DNA
ccagggttcaccccaccaca

SEQ ID NO: 377 - DNA, 20 bp, synthetic construct
  misc_feature 1..20: note = HBV-sgRNA-0374
  source 1..20: mol_type = other DNA
ccagggttcacccctcccca

SEQ ID NO: 378 - DNA, 20 bp, synthetic construct
  misc_feature 1..20: note = HBV-sgRNA-0375
  source 1..20: mol_type = other DNA
ccatatcgtcaatcttctcg

SEQ ID NO: 379 - DNA, 20 bp, synthetic construct
  misc_feature 1..20: note = HBV-sgRNA-0376
  source 1..20: mol_type = other DNA
ccatgccccaaagccaccca

SEQ ID NO: 380 - DNA, 20 bp, synthetic construct
  misc_feature 1..20: note = HBV-sgRNA-0377
  source 1..20: mol_type = other DNA
ccatggggaggggtgaaccc

SEQ ID NO: 381 - DNA, 20 bp, synthetic construct
  misc_feature 1..20: note = HBV-sgRNA-0378
  source 1..20: mol_type = other DNA
ccatttgttcagtggttcgt

SEQ ID NO: 382 - DNA, 20 bp, synthetic construct
  misc_feature 1..20: note = HBV-sgRNA-0379
  source 1..20: mol_type = other DNA
cccaaaagaccgccgtgtgg

SEQ ID NO: 383 - DNA, 20 bp, synthetic construct
  misc_feature 1..20: note = HBV-sgRNA-0380
  source 1..20: mol_type = other DNA
cccaaaaggcctccgtgcgg

SEQ ID NO: 384 - DNA, 20 bp, synthetic construct
  misc_feature 1..20: note = HBV-sgRNA-0381
  source 1..20: mol_type = other DNA
cccaacagtcccccatgggg

SEQ ID NO: 385 - DNA, 20 bp, synthetic construct
  misc_feature 1..20: note = HBV-sgRNA-0382
  source 1..20: mol_type = other DNA
cccaacgtttggttttatta

SEQ ID NO: 386 - DNA, 20 bp, synthetic construct
  misc_feature 1..20: note = HBV-sgRNA-0383
  source 1..20: mol_type = other DNA
cccaccacacggcggtcttt

SEQ ID NO: 387 - DNA, 20 bp, synthetic construct
  misc_feature 1..20: note = HBV-sgRNA-0384
  source 1..20: mol_type = other DNA
cccaccgcacggaggccttt

SEQ ID NO: 388 - DNA, 20 bp, synthetic construct
  misc_feature 1..20: note = HBV-sgRNA-0385
  source 1..20: mol_type = other DNA
cccatctctttgttttgtta

SEQ ID NO: 389 - DNA, 20 bp, synthetic construct
  misc_feature 1..20: note = HBV-sgRNA-0386
  source 1..20: mol_type = other DNA
cccatctttttgttttgtga

SEQ ID NO: 390 - DNA, 20 bp, synthetic construct
  misc_feature 1..20: note = HBV-sgRNA-0387
  source 1..20: mol_type = other DNA
cccatgggggactgttgggg

SEQ ID NO: 391 - DNA, 20 bp, synthetic construct
  misc_feature 1..20: note = HBV-sgRNA-0388
  source 1..20: mol_type = other DNA
ccccaacgtttggttttatt

SEQ ID NO: 392 - DNA, 20 bp, synthetic construct
  misc_feature 1..20: note = HBV-sgRNA-0389
  source 1..20: mol_type = other DNA
ccccatctctttgttttgtt

SEQ ID NO: 393 - DNA, 20 bp, synthetic construct
  misc_feature 1..20: note = HBV-sgRNA-0390
  source 1..20: mol_type = other DNA
ccccatctttttgttttgtg

SEQ ID NO: 394 - DNA, 20 bp, synthetic construct
  misc_feature 1..20: note = HBV-sgRNA-0391
  source 1..20: mol_type = other DNA
ccccatgccttgtcgaggtt

SEQ ID NO: 395 - DNA, 20 bp, synthetic construct
  misc_feature 1..20: note = HBV-sgRNA-0392
  source 1..20: mol_type = other DNA
ccccatgccttttcgaggtt

SEQ ID NO: 396 - DNA, 20 bp, synthetic construct
  misc_feature 1..20: note = HBV-sgRNA-0393
  source 1..20: mol_type = other DNA
ccccgagaagggtcgtccgc

SEQ ID NO: 397 - DNA, 20 bp, synthetic construct
  misc_feature 1..20: note = HBV-sgRNA-0394
  source 1..20: mol_type = other DNA
ccccgagacgggtcgtccgc

SEQ ID NO: 398 - DNA, 20 bp, synthetic construct
  misc_feature 1..20: note = HBV-sgRNA-0395
  source 1..20: mol_type = other DNA
ccccgagaggggtcgtccgc

SEQ ID NO: 399 - DNA, 20 bp, synthetic construct
  misc_feature 1..20: note = HBV-sgRNA-0396
  source 1..20: mol_type = other DNA
ccccgcctgtaacacgagaa

SEQ ID NO: 400 - DNA, 20 bp, synthetic construct
  misc_feature 1..20: note = HBV-sgRNA-0397
  source 1..20: mol_type = other DNA
ccccgcctgtaacacgagca

SEQ ID NO: 401 - DNA, 20 bp, synthetic construct
  misc_feature 1..20: note = HBV-sgRNA-0398
  source 1..20: mol_type = other DNA
cccctgctcgtgttacaggc

SEQ ID NO: 402 - DNA, 20 bp, synthetic construct
  misc_feature 1..20: note = HBV-sgRNA-0399
  source 1..20: mol_type = other DNA
ccccttctcgtgttacaggc

SEQ ID NO: 403 - DNA, 20 bp, synthetic construct
  misc_feature 1..20: note = HBV-sgRNA-0400
  source 1..20: mol_type = other DNA
cccgcacaaggacaactggc

SEQ ID NO: 404 - DNA, 20 bp, synthetic construct
  misc_feature 1..20: note = HBV-sgRNA-0401
  source 1..20: mol_type = other DNA
cccgcctgtaacacgagaag

SEQ ID NO: 405 - DNA, 20 bp, synthetic construct
  misc_feature 1..20: note = HBV-sgRNA-0402
  source 1..20: mol_type = other DNA
cccgcctgtaacacgagcag

SEQ ID NO: 406 - DNA, 20 bp, synthetic construct
  misc_feature 1..20: note = HBV-sgRNA-0403
  source 1..20: mol_type = other DNA
cccgcggacgacccctctcg

SEQ ID NO: 407 - DNA, 20 bp, synthetic construct
  misc_feature 1..20: note = HBV-sgRNA-0404
  source 1..20: mol_type = other DNA
cccgcggacgacccgtctcg

SEQ ID NO: 408 - DNA, 20 bp, synthetic construct
  misc_feature 1..20: note = HBV-sgRNA-0405
  source 1..20: mol_type = other DNA
cccgtcggcgctgaatcccg

SEQ ID NO: 409 - DNA, 20 bp, synthetic construct
  misc_feature 1..20: note = HBV-sgRNA-0406
  source 1..20: mol_type = other DNA
cccgtcggcgctgaatcctg

SEQ ID NO: 410 - DNA, 20 bp, synthetic construct
  misc_feature 1..20: note = HBV-sgRNA-0407
  source 1..20: mol_type = other DNA
cccgttgcccggcaacggcc

SEQ ID NO: 411 - DNA, 20 bp, synthetic construct
  misc_feature 1..20: note = HBV-sgRNA-0408
  source 1..20: mol_type = other DNA
cccgttgcccggcaacggtc

SEQ ID NO: 412 - DNA, 20 bp, synthetic construct
  misc_feature 1..20: note = HBV-sgRNA-0409
  source 1..20: mol_type = other DNA
cccgttgctcggcaacggcc

SEQ ID NO: 413 - DNA, 20 bp, synthetic construct
  misc_feature 1..20: note = HBV-sgRNA-0410
  source 1..20: mol_type = other DNA
cccgtttgtcctctaattcc

SEQ ID NO: 414 - DNA, 20 bp, synthetic construct
  misc_feature 1..20: note = HBV-sgRNA-0411
  source 1..20: mol_type = other DNA
cccgtttgtcctctacttcc

SEQ ID NO: 415 - DNA, 20 bp, synthetic construct
  misc_feature 1..20: note = HBV-sgRNA-0412
  source 1..20: mol_type = other DNA
ccctaacaaaacaaagagat

SEQ ID NO: 416 - DNA, 20 bp, synthetic construct
  misc_feature 1..20: note = HBV-sgRNA-0413
  source 1..20: mol_type = other DNA
ccctaataaaaccaaacgtt

SEQ ID NO: 417 - DNA, 20 bp, synthetic construct
  misc_feature 1..20: note = HBV-sgRNA-0414
  source 1..20: mol_type = other DNA
ccctagcagccatggaaagg

SEQ ID NO: 418 - DNA, 20 bp, synthetic construct
  misc_feature 1..20: note = HBV-sgRNA-0415
  source 1..20: mol_type = other DNA
ccctatcctatcaacacttc

SEQ ID NO: 419 - DNA, 20 bp, synthetic construct
  misc_feature 1..20: note = HBV-sgRNA-0416
  source 1..20: mol_type = other DNA
ccctatcttatcaacacttc

SEQ ID NO: 420 - DNA, 20 bp, synthetic construct
  misc_feature 1..20: note = HBV-sgRNA-0417
  source 1..20: mol_type = other DNA
ccctatcttatcaactcttc

SEQ ID NO: 421 - DNA, 20 bp, synthetic construct
  misc_feature 1..20: note = HBV-sgRNA-0418
  source 1..20: mol_type = other DNA
ccctcacaaaacaaaaagat

SEQ ID NO: 422 - DNA, 20 bp, synthetic construct
  misc_feature 1..20: note = HBV-sgRNA-0419
  source 1..20: mol_type = other DNA
ccctccccatgggggactgt

SEQ ID NO: 423 - DNA, 20 bp, synthetic construct
  misc_feature 1..20: note = HBV-sgRNA-0420
  source 1..20: mol_type = other DNA
ccctgctcgtgttacaggcg

SEQ ID NO: 424 - DNA, 20 bp, synthetic construct
  misc_feature 1..20: note = HBV-sgRNA-0421
  source 1..20: mol_type = other DNA
cccttacagtaaatgaaaac

SEQ ID NO: 425 - DNA, 20 bp, synthetic construct
  misc_feature 1..20: note = HBV-sgRNA-0422
  source 1..20: mol_type = other DNA
cccttctcgtgttacaggcg

SEQ ID NO: 426 - DNA, 20 bp, synthetic construct
  misc_feature 1..20: note = HBV-sgRNA-0423
  source 1..20: mol_type = other DNA
cccttcttcatctgccgttc

SEQ ID NO: 427 - DNA, 20 bp, synthetic construct
  misc_feature 1..20: note = HBV-sgRNA-0424
  source 1..20: mol_type = other DNA
ccgcaggattcagcgccgac

SEQ ID NO: 428 - DNA, 20 bp, synthetic construct
  misc_feature 1..20: note = HBV-sgRNA-0425
  source 1..20: mol_type = other DNA
ccgcgggattcagcgccgac

SEQ ID NO: 429 - DNA, 20 bp, synthetic construct
  misc_feature 1..20: note = HBV-sgRNA-0426
  source 1..20: mol_type = other DNA
ccgcttgttttgctcgcagc

SEQ ID NO: 430 - DNA, 20 bp, synthetic construct
  misc_feature 1..20: note = HBV-sgRNA-0427
  source 1..20: mol_type = other DNA
ccggaacggcagatgaagaa

SEQ ID NO: 431 - DNA, 20 bp, synthetic construct
  misc_feature 1..20: note = HBV-sgRNA-0428
  source 1..20: mol_type = other DNA
ccggaactggagccaccagc

SEQ ID NO: 432 - DNA, 20 bp, synthetic construct
  misc_feature 1..20: note = HBV-sgRNA-0429
  source 1..20: mol_type = other DNA
ccggaagagttgataagata

SEQ ID NO: 433 - DNA, 20 bp, synthetic construct
  misc_feature 1..20: note = HBV-sgRNA-0430
  source 1..20: mol_type = other DNA
ccggaagtgttgataagata

SEQ ID NO: 434 - DNA, 20 bp, synthetic construct
  misc_feature 1..20: note = HBV-sgRNA-0431
  source 1..20: mol_type = other DNA
ccggaagtgttgataggata

SEQ ID NO: 435 - DNA, 20 bp, synthetic construct
  misc_feature 1..20: note = HBV-sgRNA-0432
  source 1..20: mol_type = other DNA
ccggccagttgtccttgtgc

SEQ ID NO: 436 - DNA, 20 bp, synthetic construct
  misc_feature 1..20: note = HBV-sgRNA-0433
  source 1..20: mol_type = other DNA
ccgtggtcggccggtacaat

SEQ ID NO: 437 - DNA, 20 bp, synthetic construct
  misc_feature 1..20: note = HBV-sgRNA-0434
  source 1..20: mol_type = other DNA
ccgtgtggtggggtgaaccc

SEQ ID NO: 438 - DNA, 20 bp, synthetic construct
  misc_feature 1..20: note = HBV-sgRNA-0435
  source 1..20: mol_type = other DNA
cctaacaaaacaaagagatg

SEQ ID NO: 439 - DNA, 20 bp, synthetic construct
  misc_feature 1..20: note = HBV-sgRNA-0436
  source 1..20: mol_type = other DNA
cctaataaaaccaaacgttg

SEQ ID NO: 440 - DNA, 20 bp, synthetic construct
  misc_feature 1..20: note = HBV-sgRNA-0437
  source 1..20: mol_type = other DNA
cctacgaaccactgaacaaa

SEQ ID NO: 441 - DNA, 20 bp, synthetic construct
  misc_feature 1..20: note = HBV-sgRNA-0438
  source 1..20: mol_type = other DNA
cctattgtaccggccgacca

SEQ ID NO: 442 - DNA, 20 bp, synthetic construct
  misc_feature 1..20: note = HBV-sgRNA-0439
  source 1..20: mol_type = other DNA
cctcacaaaacaaaaagatg

SEQ ID NO: 443 - DNA, 20 bp, synthetic construct
  misc_feature 1..20: note = HBV-sgRNA-0440
  source 1..20: mol_type = other DNA
cctccaagctgtgccttggg

SEQ ID NO: 444 - DNA, 20 bp, synthetic construct
  misc_feature 1..20: note = HBV-sgRNA-0441
  source 1..20: mol_type = other DNA
cctccccatgggggactgtt

SEQ ID NO: 445 - DNA, 20 bp, synthetic construct
  misc_feature 1..20: note = HBV-sgRNA-0442
  source 1..20: mol_type = other DNA
cctcctttccatggctgcta

SEQ ID NO: 446 - DNA, 20 bp, synthetic construct
  misc_feature 1..20: note = HBV-sgRNA-0443
  source 1..20: mol_type = other DNA
cctcgagaagattgacgata

SEQ ID NO: 447 - DNA, 20 bp, synthetic construct
  misc_feature 1..20: note = HBV-sgRNA-0444
  source 1..20: mol_type = other DNA
cctgaactggagccaccagc

SEQ ID NO: 448 - DNA, 20 bp, synthetic construct
  misc_feature 1..20: note = HBV-sgRNA-0445
  source 1..20: mol_type = other DNA
cctgaccgttgccgggcaac

SEQ ID NO: 449 - DNA, 20 bp, synthetic construct
  misc_feature 1..20: note = HBV-sgRNA-0446
  source 1..20: mol_type = other DNA
cctgagggctccaccccaaa

SEQ ID NO: 450 - DNA, 20 bp, synthetic construct
  misc_feature 1..20: note = HBV-sgRNA-0447
  source 1..20: mol_type = other DNA
cctgcggacgacccttctcg

SEQ ID NO: 451 - DNA, 20 bp, synthetic construct
  misc_feature 1..20: note = HBV-sgRNA-0448
  source 1..20: mol_type = other DNA
cctgctgcgagcaaaacaag

SEQ ID NO: 452 - DNA, 20 bp, synthetic construct
  misc_feature 1..20: note = HBV-sgRNA-0449
  source 1..20: mol_type = other DNA
cctgctggtggctccagttc

SEQ ID NO: 453 - DNA, 20 bp, synthetic construct
  misc_feature 1..20: note = HBV-sgRNA-0450
  source 1..20: mol_type = other DNA
cctggaagtagaggacaaac

SEQ ID NO: 454 - DNA, 20 bp, synthetic construct
  misc_feature 1..20: note = HBV-sgRNA-0451
  source 1..20: mol_type = other DNA
cctggaattagaggacaaac

SEQ ID NO: 455 - DNA, 20 bp, synthetic construct
  misc_feature 1..20: note = HBV-sgRNA-0452
  source 1..20: mol_type = other DNA
cctggccgttgccgggcaac

SEQ ID NO: 456 - DNA, 20 bp, synthetic construct
  misc_feature 1..20: note = HBV-sgRNA-0453
  source 1..20: mol_type = other DNA
cctgttttcatttactgtaa

SEQ ID NO: 457 - DNA, 20 bp, synthetic construct
  misc_feature 1..20: note = HBV-sgRNA-0454
  source 1..20: mol_type = other DNA
ccttatcgtcaatcttctcg

SEQ ID NO: 458 - DNA, 20 bp, synthetic construct
  misc_feature 1..20: note = HBV-sgRNA-0455
  source 1..20: mol_type = other DNA
ccttcctgactgccgattgg

SEQ ID NO: 459 - DNA, 20 bp, synthetic construct
  misc_feature 1..20: note = HBV-sgRNA-0456
  source 1..20: mol_type = other DNA
ccttcctgtctggcgattgg

SEQ ID NO: 460 - DNA, 20 bp, synthetic construct
  misc_feature 1..20: note = HBV-sgRNA-0457
  source 1..20: mol_type = other DNA
ccttgggtggctttggggca

SEQ ID NO: 461 - DNA, 20 bp, synthetic construct
  misc_feature 1..20: note = HBV-sgRNA-0458
  source 1..20: mol_type = other DNA
ccttttggggtggagccctc

SEQ ID NO: 462 - DNA, 20 bp, synthetic construct
  misc_feature 1..20: note = HBV-sgRNA-0459
  source 1..20: mol_type = other DNA
cgaaggtttggtacagcaac

SEQ ID NO: 463 - DNA, 20 bp, synthetic construct
  misc_feature 1..20: note = HBV-sgRNA-0460
  source 1..20: mol_type = other DNA
cgaattttggccaagacaca

SEQ ID NO: 464 - DNA, 20 bp, synthetic construct
  misc_feature 1..20: note = HBV-sgRNA-0461
  source 1..20: mol_type = other DNA
cgaattttggccaggacacg

SEQ ID NO: 465 - DNA, 20 bp, synthetic construct
  misc_feature 1..20: note = HBV-sgRNA-0462
  source 1..20: mol_type = other DNA
cgacccctctcggggccgct

SEQ ID NO: 466 - DNA, 20 bp, synthetic construct
  misc_feature 1..20: note = HBV-sgRNA-0463
  source 1..20: mol_type = other DNA
cgacccgtctcggggccgtt

SEQ ID NO: 467 - DNA, 20 bp, synthetic construct
  misc_feature 1..20: note = HBV-sgRNA-0464
  source 1..20: mol_type = other DNA
cgacccttctcggggtcgct

SEQ ID NO: 468 - DNA, 20 bp, synthetic construct
  misc_feature 1..20: note = HBV-sgRNA-0465
  source 1..20: mol_type = other DNA
cgagggagttcttcttctag

SEQ ID NO: 469 - DNA, 20 bp, synthetic construct
  misc_feature 1..20: note = HBV-sgRNA-0466
  source 1..20: mol_type = other DNA
cgataaccaggacaaattgg

SEQ ID NO: 470 - DNA, 20 bp, synthetic construct
  misc_feature 1..20: note = HBV-sgRNA-0467
  source 1..20: mol_type = other DNA
cgataaccaggacaagttgg

SEQ ID NO: 471 - DNA, 20 bp, synthetic construct
  misc_feature 1..20: note = HBV-sgRNA-0468
  source 1..20: mol_type = other DNA
cgataagtttcgctccagac

SEQ ID NO: 472 - DNA, 20 bp, synthetic construct
  misc_feature 1..20: note = HBV-sgRNA-0469
  source 1..20: mol_type = other DNA
cgatagccaggacaaattgg

SEQ ID NO: 473 - DNA, 20 bp, synthetic construct
  misc_feature 1..20: note = HBV-sgRNA-0470
  source 1..20: mol_type = other DNA
cgattggtggaggcaggagg

SEQ ID NO: 474 - DNA, 20 bp, synthetic construct
  misc_feature 1..20: note = HBV-sgRNA-0471
  source 1..20: mol_type = other DNA
cgcaaaatacctatgggagt

SEQ ID NO: 475 - DNA, 20 bp, synthetic construct
  misc_feature 1..20: note = HBV-sgRNA-0472
  source 1..20: mol_type = other DNA
cgcaagattcctatgggagt

SEQ ID NO: 476 - DNA, 20 bp, synthetic construct
  misc_feature 1..20: note = HBV-sgRNA-0473
  source 1..20: mol_type = other DNA
cgcacggaggccttttgggg

SEQ ID NO: 477 - DNA, 20 bp, synthetic construct
  misc_feature 1..20: note = HBV-sgRNA-0474
  source 1..20: mol_type = other DNA
cgcagagtctagactcgtgg

SEQ ID NO: 478 - DNA, 20 bp, synthetic construct
  misc_feature 1..20: note = HBV-sgRNA-0475
  source 1..20: mol_type = other DNA
cgcagggtccaactggtgat

SEQ ID NO: 479 - DNA, 20 bp, synthetic construct
  misc_feature 1..20: note = HBV-sgRNA-0476
  source 1..20: mol_type = other DNA
cgcccacaggaacctgccca

SEQ ID NO: 480 - DNA, 20 bp, synthetic construct
  misc_feature 1..20: note = HBV-sgRNA-0477
  source 1..20: mol_type = other DNA
cgcccaccaggtcttgccca

SEQ ID NO: 481 - DNA, 20 bp, synthetic construct
  misc_feature 1..20: note = HBV-sgRNA-0478
  source 1..20: mol_type = other DNA
cgcccaccgaatgttgccca

SEQ ID NO: 482 - DNA, 20 bp, synthetic construct
  misc_feature 1..20: note = HBV-sgRNA-0479
  source 1..20: mol_type = other DNA
cgccccgtggtcggccggaa

SEQ ID NO: 483 - DNA, 20 bp, synthetic construct
  misc_feature 1..20: note = HBV-sgRNA-0480
  source 1..20: mol_type = other DNA
cgccccgtggtcggtcggaa

SEQ ID NO: 484 - DNA, 20 bp, synthetic construct
  misc_feature 1..20: note = HBV-sgRNA-0481
  source 1..20: mol_type = other DNA
cgccgacgggacgtaaacaa

SEQ ID NO: 485 - DNA, 20 bp, synthetic construct
  misc_feature 1..20: note = HBV-sgRNA-0482
  source 1..20: mol_type = other DNA
cgccgacgggacgtagacaa

SEQ ID NO: 486 - DNA, 20 bp, synthetic construct
  misc_feature 1..20: note = HBV-sgRNA-0483
  source 1..20: mol_type = other DNA
cgcctctgctctgtatcggg

SEQ ID NO: 487 - DNA, 20 bp, synthetic construct
  misc_feature 1..20: note = HBV-sgRNA-0484
  source 1..20: mol_type = other DNA
cgcttctccgcctattgtac

SEQ ID NO: 488 - DNA, 20 bp, synthetic construct
  misc_feature 1..20: note = HBV-sgRNA-0485
  source 1..20: mol_type = other DNA
cgcttctgctctgtatcggg

SEQ ID NO: 489 - DNA, 20 bp, synthetic construct
  misc_feature 1..20: note = HBV-sgRNA-0486
  source 1..20: mol_type = other DNA
cggaaaattcctatgggagt

SEQ ID NO: 490 - DNA, 20 bp, synthetic construct
  misc_feature 1..20: note = HBV-sgRNA-0487
  source 1..20: mol_type = other DNA
cggaacagggtttactgttc

SEQ ID NO: 491 - DNA, 20 bp, synthetic construct
  misc_feature 1..20: note = HBV-sgRNA-0488
  source 1..20: mol_type = other DNA
cggaacggcagacggagaag

SEQ ID NO: 492 - DNA, 20 bp, synthetic construct
  misc_feature 1..20: note = HBV-sgRNA-0489
  source 1..20: mol_type = other DNA
cggaacggcagatgaagaag

SEQ ID NO: 493 - DNA, 20 bp, synthetic construct
  misc_feature 1..20: note = HBV-sgRNA-0490
  source 1..20: mol_type = other DNA
cggaagagttgataagatag

SEQ ID NO: 494 - DNA, 20 bp, synthetic construct
  misc_feature 1..20: note = HBV-sgRNA-0491
  source 1..20: mol_type = other DNA
cggaagtgttgataagatag

SEQ ID NO: 495 - DNA, 20 bp, synthetic construct
  misc_feature 1..20: note = HBV-sgRNA-0492
  source 1..20: mol_type = other DNA
cggaagtgttgataggatag

SEQ ID NO: 496 - DNA, 20 bp, synthetic construct
  misc_feature 1..20: note = HBV-sgRNA-0493
  source 1..20: mol_type = other DNA
cggctaggagttccgcagta

SEQ ID NO: 497 - DNA, 20 bp, synthetic construct
  misc_feature 1..20: note = HBV-sgRNA-0494
  source 1..20: mol_type = other DNA
cggggagaccgcgtaaagag

SEQ ID NO: 498 - DNA, 20 bp, synthetic construct
  misc_feature 1..20: note = HBV-sgRNA-0495
  source 1..20: mol_type = other DNA
cggggagtccgcgtaaagag

SEQ ID NO: 499 - DNA, 20 bp, synthetic construct
  misc_feature 1..20: note = HBV-sgRNA-0496
  source 1..20: mol_type = other DNA
cggtacaataggcggagaag

SEQ ID NO: 500 - DNA, 20 bp, synthetic construct
  misc_feature 1..20: note = HBV-sgRNA-0497
  source 1..20: mol_type = other DNA
cggtctggagcgaaacttat

SEQ ID NO: 501 - DNA, 20 bp, synthetic construct
  misc_feature 1..20: note = HBV-sgRNA-0498
  source 1..20: mol_type = other DNA
cggtttaatgcctttgtcta

SEQ ID NO: 502 - DNA, 20 bp, synthetic construct
  misc_feature 1..20: note = HBV-sgRNA-0499
  source 1..20: mol_type = other DNA
cggtttgatccctttatcta

SEQ ID NO: 503 - DNA, 20 bp, synthetic construct
  misc_feature 1..20: note = HBV-sgRNA-0500
  source 1..20: mol_type = other DNA
cgtcaatcttatcgaagact

SEQ ID NO: 504 - DNA, 20 bp, synthetic construct
  misc_feature 1..20: note = HBV-sgRNA-0501
  source 1..20: mol_type = other DNA
cgtcaatcttctcgaggact

SEQ ID NO: 505 - DNA, 20 bp, synthetic construct
  misc_feature 1..20: note = HBV-sgRNA-0502
  source 1..20: mol_type = other DNA
cgtcaatcttctcgaggatt

SEQ ID NO: 506 - DNA, 20 bp, synthetic construct
  misc_feature 1..20: note = HBV-sgRNA-0503
  source 1..20: mol_type = other DNA
cgtcccgcgcaggatccagt

SEQ ID NO: 507 - DNA, 20 bp, synthetic construct
  misc_feature 1..20: note = HBV-sgRNA-0504
  source 1..20: mol_type = other DNA
cgtctaacaacagtagtttc

SEQ ID NO: 508 - DNA, 20 bp, synthetic construct
  misc_feature 1..20: note = HBV-sgRNA-0505
  source 1..20: mol_type = other DNA
ctaagggcaaatatttggta

SEQ ID NO: 509 - DNA, 20 bp, synthetic construct
  misc_feature 1..20: note = HBV-sgRNA-0506
  source 1..20: mol_type = other DNA
ctaatatgggcctaaagttc

SEQ ID NO: 510 - DNA, 20 bp, synthetic construct
  misc_feature 1..20: note = HBV-sgRNA-0507
  source 1..20: mol_type = other DNA
ctactaattccctggatgct

SEQ ID NO: 511 - DNA, 20 bp, synthetic construct
  misc_feature 1..20: note = HBV-sgRNA-0508
  source 1..20: mol_type = other DNA
ctagactctgcggtattgtg

SEQ ID NO: 512 - DNA, 20 bp, synthetic construct
  misc_feature 1..20: note = HBV-sgRNA-0509
  source 1..20: mol_type = other DNA
ctagactctgtggtattgtg

SEQ ID NO: 513 - DNA, 20 bp, synthetic construct
  misc_feature 1..20: note = HBV-sgRNA-0510
  source 1..20: mol_type = other DNA
ctattaacaggcctattgat

SEQ ID NO: 514 - DNA, 20 bp, synthetic construct
  misc_feature 1..20: note = HBV-sgRNA-0511
  source 1..20: mol_type = other DNA
ctattgtaccggccgaccac

SEQ ID NO: 515 - DNA, 20 bp, synthetic construct
  misc_feature 1..20: note = HBV-sgRNA-0512
  source 1..20: mol_type = other DNA
ctatttacacactctatgga

SEQ ID NO: 516 - DNA, 20 bp, synthetic construct
  misc_feature 1..20: note = HBV-sgRNA-0513
  source 1..20: mol_type = other DNA
ctcaagatgctgtacagact

SEQ ID NO: 517 - DNA, 20 bp, synthetic construct
  misc_feature 1..20: note = HBV-sgRNA-0514
  source 1..20: mol_type = other DNA
ctcaagatgttgtacagact

SEQ ID NO: 518 - DNA, 20 bp, synthetic construct
  misc_feature 1..20: note = HBV-sgRNA-0515
  source 1..20: mol_type = other DNA
ctcatcctcaggccatgcag

SEQ ID NO: 519 - DNA, 20 bp, synthetic construct
  misc_feature 1..20: note = HBV-sgRNA-0516
  source 1..20: mol_type = other DNA
ctccccatgggggactgttg

SEQ ID NO: 520 - DNA, 20 bp, synthetic construct
  misc_feature 1..20: note = HBV-sgRNA-0517
  source 1..20: mol_type = other DNA
ctcccgatacagagcagaag

SEQ ID NO: 521 - DNA, 20 bp, synthetic construct
  misc_feature 1..20: note = HBV-sgRNA-0518
  source 1..20: mol_type = other DNA
ctcccgatacagagcagagg

SEQ ID NO: 522 - DNA, 20 bp, synthetic construct
  misc_feature 1..20: note = HBV-sgRNA-0519
  source 1..20: mol_type = other DNA
ctccctcgcctcgcagacga

SEQ ID NO: 523 - DNA, 20 bp, synthetic construct
  misc_feature 1..20: note = HBV-sgRNA-0520
  source 1..20: mol_type = other DNA
ctcccttatctccacctcta

SEQ ID NO: 524 - DNA, 20 bp, synthetic construct
  misc_feature 1..20: note = HBV-sgRNA-0521
  source 1..20: mol_type = other DNA
ctccgaacgcagggtccaac

SEQ ID NO: 525 - DNA, 20 bp, synthetic construct
  misc_feature 1..20: note = HBV-sgRNA-0522
  source 1..20: mol_type = other DNA
ctcctcctgcctccaccaat

SEQ ID NO: 526 - DNA, 20 bp, synthetic construct
  misc_feature 1..20: note = HBV-sgRNA-0523
  source 1..20: mol_type = other DNA
ctcgagaagattgacgataa

SEQ ID NO: 527 - DNA, 20 bp, synthetic construct
  misc_feature 1..20: note = HBV-sgRNA-0524
  source 1..20: mol_type = other DNA
ctcgagaagattgacgatat

SEQ ID NO: 528 - DNA, 20 bp, synthetic construct
  misc_feature 1..20: note = HBV-sgRNA-0525
  source 1..20: mol_type = other DNA
ctctgaaggctggatccaac

SEQ ID NO: 529 - DNA, 20 bp, synthetic construct
  misc_feature 1..20: note = HBV-sgRNA-0526
  source 1..20: mol_type = other DNA
ctctgctagatcccagagtg

SEQ ID NO: 530 - DNA, 20 bp, synthetic construct
  misc_feature 1..20: note = HBV-sgRNA-0527
  source 1..20: mol_type = other DNA
ctctggccagtgatccttgt

SEQ ID NO: 531 - DNA, 20 bp, synthetic construct
  misc_feature 1..20: note = HBV-sgRNA-0528
  source 1..20: mol_type = other DNA
ctctgggatctagcagagct

SEQ ID NO: 532 - DNA, 20 bp, synthetic construct
  misc_feature 1..20: note = HBV-sgRNA-0529
  source 1..20: mol_type = other DNA
ctctgggatcttgaagagtt

SEQ ID NO: 533 - DNA, 20 bp, synthetic construct
  misc_feature 1..20: note = HBV-sgRNA-0530
  source 1..20: mol_type = other DNA
ctctgggatcttgcagagtt

SEQ ID NO: 534 - DNA, 20 bp, synthetic construct
  misc_feature 1..20: note = HBV-sgRNA-0531
  source 1..20: mol_type = other DNA
ctcttacagttaatgaaaaa

SEQ ID NO: 535 - DNA, 20 bp, synthetic construct
  misc_feature 1..20: note = HBV-sgRNA-0532
  source 1..20: mol_type = other DNA
ctcttcaagatcccagagtc

SEQ ID NO: 536 - DNA, 20 bp, synthetic construct
  misc_feature 1..20: note = HBV-sgRNA-0533
  source 1..20: mol_type = other DNA
ctgaactggagccaccagca

SEQ ID NO: 537 - DNA, 20 bp, synthetic construct
  misc_feature 1..20: note = HBV-sgRNA-0534
  source 1..20: mol_type = other DNA
ctgaccgttgccgggcaacg

SEQ ID NO: 538 - DNA, 20 bp, synthetic construct
  misc_feature 1..20: note = HBV-sgRNA-0535
  source 1..20: mol_type = other DNA
ctgacgcaacccccactgga

SEQ ID NO: 539 - DNA, 20 bp, synthetic construct
  misc_feature 1..20: note = HBV-sgRNA-0536
  source 1..20: mol_type = other DNA
ctgacgcaacccccactggc

SEQ ID NO: 540 - DNA, 20 bp, synthetic construct
  misc_feature 1..20: note = HBV-sgRNA-0537
  source 1..20: mol_type = other DNA
ctgacgcaacccccactggt

SEQ ID NO: 541 - DNA, 20 bp, synthetic construct
  misc_feature 1..20: note = HBV-sgRNA-0538
  source 1..20: mol_type = other DNA
ctgagttggctttgaatgca

SEQ ID NO: 542 - DNA, 20 bp, synthetic construct
  misc_feature 1..20: note = HBV-sgRNA-0539
  source 1..20: mol_type = other DNA
ctgcaagatcccagagtgag

SEQ ID NO: 543 - DNA, 20 bp, synthetic construct
  misc_feature 1..20: note = HBV-sgRNA-0540
  source 1..20: mol_type = other DNA
ctgccaactggatcctgcgc

SEQ ID NO: 544 - DNA, 20 bp, synthetic construct
  misc_feature 1..20: note = HBV-sgRNA-0541
  source 1..20: mol_type = other DNA
ctgccgttccgaccgaccac

SEQ ID NO: 545 - DNA, 20 bp, synthetic construct
  misc_feature 1..20: note = HBV-sgRNA-0542
  source 1..20: mol_type = other DNA
ctgccgttccggccgaccac

SEQ ID NO: 546 - DNA, 20 bp, synthetic construct
  misc_feature 1..20: note = HBV-sgRNA-0543
  source 1..20: mol_type = other DNA
ctgccttcctgactgccgat

SEQ ID NO: 547 - DNA, 20 bp, synthetic construct
  misc_feature 1..20: note = HBV-sgRNA-0544
  source 1..20: mol_type = other DNA
ctgccttcctgtctggcgat

SEQ ID NO: 548 - DNA, 20 bp, synthetic construct
  misc_feature 1..20: note = HBV-sgRNA-0545
  source 1..20: mol_type = other DNA
ctgctagatcccagagtgag

SEQ ID NO: 549 - DNA, 20 bp, synthetic construct
  misc_feature 1..20: note = HBV-sgRNA-0546
  source 1..20: mol_type = other DNA
ctgctaggagttccgcagta

SEQ ID NO: 550 - DNA, 20 bp, synthetic construct
  misc_feature 1..20: note = HBV-sgRNA-0547
  source 1..20: mol_type = other DNA
ctgctggcacagttgtgagt

SEQ ID NO: 551 - DNA, 20 bp, synthetic construct
  misc_feature 1..20: note = HBV-sgRNA-0548
  source 1..20: mol_type = other DNA
ctggccagtgatccttgttg

SEQ ID NO: 552 - DNA, 20 bp, synthetic construct
  misc_feature 1..20: note = HBV-sgRNA-0549
  source 1..20: mol_type = other DNA
ctggccggacgccaacaagg

SEQ ID NO: 553 - DNA, 20 bp, synthetic construct
  misc_feature 1..20: note = HBV-sgRNA-0550
  source 1..20: mol_type = other DNA
ctggccgttgccgggcaacg

SEQ ID NO: 554 - DNA, 20 bp, synthetic construct
  misc_feature 1..20: note = HBV-sgRNA-0551
  source 1..20: mol_type = other DNA
ctgggtttcaccccaccgca

SEQ ID NO: 555 - DNA, 20 bp, synthetic construct
  misc_feature 1..20: note = HBV-sgRNA-0552
  source 1..20: mol_type = other DNA
ctgtaaacaggcctattgat

SEQ ID NO: 556 - DNA, 20 bp, synthetic construct
  misc_feature 1..20: note = HBV-sgRNA-0553
  source 1..20: mol_type = other DNA
ctgtaaatagacctattgat

SEQ ID NO: 557 - DNA, 20 bp, synthetic construct
  misc_feature 1..20: note = HBV-sgRNA-0554
  source 1..20: mol_type = other DNA
ctgtaaatgaatgtgaggaa

SEQ ID NO: 558 - DNA, 20 bp, synthetic construct
  misc_feature 1..20: note = HBV-sgRNA-0555
  source 1..20: mol_type = other DNA
ctgtctggctttcagttata

SEQ ID NO: 559 - DNA, 20 bp, synthetic construct
  misc_feature 1..20: note = HBV-sgRNA-0556
  source 1..20: mol_type = other DNA
ctgtcttcctgactgccgat

SEQ ID NO: 560 - DNA, 20 bp, synthetic construct
  misc_feature 1..20: note = HBV-sgRNA-0557
  source 1..20: mol_type = other DNA
ctgtgccttgggtggctttg

SEQ ID NO: 561 - DNA, 20 bp, synthetic construct
  misc_feature 1..20: note = HBV-sgRNA-0558
  source 1..20: mol_type = other DNA
ctgtgtgtttaaagactggg

SEQ ID NO: 562 - DNA, 20 bp, synthetic construct
  misc_feature 1..20: note = HBV-sgRNA-0559
  source 1..20: mol_type = other DNA
ctgtgtgtttactgagtggg

SEQ ID NO: 563 - DNA, 20 bp, synthetic construct
  misc_feature 1..20: note = HBV-sgRNA-0560
  source 1..20: mol_type = other DNA
ctgttgctgtaccaaacctt

SEQ ID NO: 564 - DNA, 20 bp, synthetic construct
  misc_feature 1..20: note = HBV-sgRNA-0561
  source 1..20: mol_type = other DNA
ctgttgttagacgacgaggc

SEQ ID NO: 565 - DNA, 20 bp, synthetic construct
  misc_feature 1..20: note = HBV-sgRNA-0562
  source 1..20: mol_type = other DNA
ctgtttggctttcagttata

SEQ ID NO: 566 - DNA, 20 bp, synthetic construct
  misc_feature 1..20: note = HBV-sgRNA-0563
  source 1..20: mol_type = other DNA
ctgtttgtttaaagactggg

SEQ ID NO: 567 - DNA, 20 bp, synthetic construct
  misc_feature 1..20: note = HBV-sgRNA-0564
  source 1..20: mol_type = other DNA
ctgttttcatttactgtaag

SEQ ID NO: 568 - DNA, 20 bp, synthetic construct
  misc_feature 1..20: note = HBV-sgRNA-0565
  source 1..20: mol_type = other DNA
cttagaaaggccttgtaagt

SEQ ID NO: 569 - DNA, 20 bp, synthetic construct
  misc_feature 1..20: note = HBV-sgRNA-0566
  source 1..20: mol_type = other DNA
cttatccaatggtaaatatt

SEQ ID NO: 570 - DNA, 20 bp, synthetic construct
  misc_feature 1..20: note = HBV-sgRNA-0567
  source 1..20: mol_type = other DNA
cttcacctctgcacgtcgca

SEQ ID NO: 571 - DNA, 20 bp, synthetic construct
  misc_feature 1..20: note = HBV-sgRNA-0568
  source 1..20: mol_type = other DNA
cttcgataagattgacgata

SEQ ID NO: 572 - DNA, 20 bp, synthetic construct
  misc_feature 1..20: note = HBV-sgRNA-0569
  source 1..20: mol_type = other DNA
cttgaatatttggtgtcttt

SEQ ID NO: 573 - DNA, 20 bp, synthetic construct
  misc_feature 1..20: note = HBV-sgRNA-0570
  source 1..20: mol_type = other DNA
cttgagtatttggtatcttt

SEQ ID NO: 574 - DNA, 20 bp, synthetic construct
  misc_feature 1..20: note = HBV-sgRNA-0571
  source 1..20: mol_type = other DNA
cttgcatggccccgtgctgg

SEQ ID NO: 575 - DNA, 20 bp, synthetic construct
  misc_feature 1..20: note = HBV-sgRNA-0572
  source 1..20: mol_type = other DNA
cttgcgaaagcccaggatga

SEQ ID NO: 576 - DNA, 20 bp, synthetic construct
  misc_feature 1..20: note = HBV-sgRNA-0573
  source 1..20: mol_type = other DNA
ctttccaccagcaatcctct

SEQ ID NO: 577 - DNA, 20 bp, synthetic construct
  misc_feature 1..20: note = HBV-sgRNA-0574
  source 1..20: mol_type = other DNA
ctttcctcacattcatttac

SEQ ID NO: 578 - DNA, 20 bp, synthetic construct
  misc_feature 1..20: note = HBV-sgRNA-0575
  source 1..20: mol_type = other DNA
ctttctgtccccaatcccct

SEQ ID NO: 579 - DNA, 20 bp, synthetic construct
  misc_feature 1..20: note = HBV-sgRNA-0576
  source 1..20: mol_type = other DNA
ctttctgttcccaatcctct

SEQ ID NO: 580 - DNA, 20 bp, synthetic construct
  misc_feature 1..20: note = HBV-sgRNA-0577
  source 1..20: mol_type = other DNA
cttttctcattaactgtaag

SEQ ID NO: 581 - DNA, 20 bp, synthetic construct
  misc_feature 1..20: note = HBV-sgRNA-0578
  source 1..20: mol_type = other DNA
cttttttcattaactgtaag

SEQ ID NO: 582 - DNA, 20 bp, synthetic construct
  misc_feature 1..20: note = HBV-sgRNA-0579
  source 1..20: mol_type = other DNA
gaaagcccaagatgatggga

SEQ ID NO: 583 - DNA, 20 bp, synthetic construct
  misc_feature 1..20: note = HBV-sgRNA-0580
  source 1..20: mol_type = other DNA
gaaagcccaggatgatggga

SEQ ID NO: 584 - DNA, 20 bp, synthetic construct
  misc_feature 1..20: note = HBV-sgRNA-0581
  source 1..20: mol_type = other DNA
gaaagtatgtcaacgaattg

SEQ ID NO: 585 - DNA, 20 bp, synthetic construct
  misc_feature 1..20: note = HBV-sgRNA-0582
  source 1..20: mol_type = other DNA
gaaagtctgtcaaagaattg

SEQ ID NO: 586 - DNA, 20 bp, synthetic construct
  misc_feature 1..20: note = HBV-sgRNA-0583
  source 1..20: mol_type = other DNA
gaaatacaggcctctcactc

SEQ ID NO: 587 - DNA, 20 bp, synthetic construct
  misc_feature 1..20: note = HBV-sgRNA-0584
  source 1..20: mol_type = other DNA
gaacatcaaccaccagcacg

SEQ ID NO: 588 - DNA, 20 bp, synthetic construct
  misc_feature 1..20: note = HBV-sgRNA-0585
  source 1..20: mol_type = other DNA
gaagaaccaacaagaagatg

SEQ ID NO: 589 - DNA, 20 bp, synthetic construct
  misc_feature 1..20: note = HBV-sgRNA-0586
  source 1..20: mol_type = other DNA
gaagattgacgataagggag

SEQ ID NO: 590 - DNA, 20 bp, synthetic construct
  misc_feature 1..20: note = HBV-sgRNA-0587
  source 1..20: mol_type = other DNA
gaagattgacgatatgggtg

SEQ ID NO: 591 - DNA, 20 bp, synthetic construct
  misc_feature 1..20: note = HBV-sgRNA-0588
  source 1..20: mol_type = other DNA
gaagcgaagtgcacacggtc

SEQ ID NO: 592 - DNA, 20 bp, synthetic construct
  misc_feature 1..20: note = HBV-sgRNA-0589
  source 1..20: mol_type = other DNA
gaagctccaaattctttata

SEQ ID NO: 593 - DNA, 20 bp, synthetic construct
  misc_feature 1..20: note = HBV-sgRNA-0590
  source 1..20: mol_type = other DNA
gaatcccagaggattgctgg

SEQ ID NO: 594 - DNA, 20 bp, synthetic construct
  misc_feature 1..20: note = HBV-sgRNA-0591
  source 1..20: mol_type = other DNA
gaattttggccaagacacac

SEQ ID NO: 595 - DNA, 20 bp, synthetic construct
  misc_feature 1..20: note = HBV-sgRNA-0592
  source 1..20: mol_type = other DNA
gaattttggccaggacacgt

SEQ ID NO: 596 - DNA, 20 bp, synthetic construct
  misc_feature 1..20: note = HBV-sgRNA-0593
  source 1..20: mol_type = other DNA
gacaaacgggcaacatacct

SEQ ID NO: 597 - DNA, 20 bp, synthetic construct
  misc_feature 1..20: note = HBV-sgRNA-0594
  source 1..20: mol_type = other DNA
gacactatttacacactcta

SEQ ID NO: 598 - DNA, 20 bp, synthetic construct
  misc_feature 1..20: note = HBV-sgRNA-0595
  source 1..20: mol_type = other DNA
gacatgaacaagagatgatt

SEQ ID NO: 599 - DNA, 20 bp, synthetic construct
  misc_feature 1..20: note = HBV-sgRNA-0596
  source 1..20: mol_type = other DNA
gacatgaacatgagatgatt

SEQ ID NO: 600 - DNA, 20 bp, synthetic construct
  misc_feature 1..20: note = HBV-sgRNA-0597
  source 1..20: mol_type = other DNA
gacattatttacacactctt

SEQ ID NO: 601 - DNA, 20 bp, synthetic construct
  misc_feature 1..20: note = HBV-sgRNA-0598
  source 1..20: mol_type = other DNA
gaccaagccccagccagtgg

SEQ ID NO: 602 - DNA, 20 bp, synthetic construct
  misc_feature 1..20: note = HBV-sgRNA-0599
  source 1..20: mol_type = other DNA
gaccaccgtgaacgcccacc

SEQ ID NO: 603 - DNA, 20 bp, synthetic construct
  misc_feature 1..20: note = HBV-sgRNA-0600
  source 1..20: mol_type = other DNA
gacccctctcggggccgctt

SEQ ID NO: 604 - DNA, 20 bp, synthetic construct
  misc_feature 1..20: note = HBV-sgRNA-0601
  source 1..20: mol_type = other DNA
gacccgtctcggggccgttt

SEQ ID NO: 605 - DNA, 20 bp, synthetic construct
  misc_feature 1..20: note = HBV-sgRNA-0602
  source 1..20: mol_type = other DNA
gacccttctcggggtcgctt

SEQ ID NO: 606 - DNA, 20 bp, synthetic construct
  misc_feature 1..20: note = HBV-sgRNA-0603
  source 1..20: mol_type = other DNA
gacctggtgggcgttcacgg

SEQ ID NO: 607 - DNA, 20 bp, synthetic construct
  misc_feature 1..20: note = HBV-sgRNA-0604
  source 1..20: mol_type = other DNA
gaccttcgtctgcgaggcga

SEQ ID NO: 608 - DNA, 20 bp, synthetic construct
  misc_feature 1..20: note = HBV-sgRNA-0605
  source 1..20: mol_type = other DNA
gaccttgggcaacattcggt

SEQ ID NO: 609 - DNA, 20 bp, synthetic construct
  misc_feature 1..20: note = HBV-sgRNA-0606
  source 1..20: mol_type = other DNA
gaccttgggcaagacctggt

SEQ ID NO: 610 - DNA, 20 bp, synthetic construct
  misc_feature 1..20: note = HBV-sgRNA-0607
  source 1..20: mol_type = other DNA
gaccttgggcaggttcctgt

SEQ ID NO: 611 - DNA, 20 bp, synthetic construct
  misc_feature 1..20: note = HBV-sgRNA-0608
  source 1..20: mol_type = other DNA
gacgcaacccccactggatg

SEQ ID NO: 612 - DNA, 20 bp, synthetic construct
  misc_feature 1..20: note = HBV-sgRNA-0609
  source 1..20: mol_type = other DNA
gacgcaacccccactggctg

SEQ ID NO: 613 - DNA, 20 bp, synthetic construct
  misc_feature 1..20: note = HBV-sgRNA-0610
  source 1..20: mol_type = other DNA
gacgcaacccccactggttg

SEQ ID NO: 614 - DNA, 20 bp, synthetic construct
  misc_feature 1..20: note = HBV-sgRNA-0611
  source 1..20: mol_type = other DNA
gacgccaacaaggtaggagc

SEQ ID NO: 615 - DNA, 20 bp, synthetic construct
  misc_feature 1..20: note = HBV-sgRNA-0612
  source 1..20: mol_type = other DNA
gacgccaacaaggtgggagt

SEQ ID NO: 616 - DNA, 20 bp, synthetic construct
  misc_feature 1..20: note = HBV-sgRNA-0613
  source 1..20: mol_type = other DNA
gactgccgattggtggaggc

SEQ ID NO: 617 - DNA, 20 bp, synthetic construct
  misc_feature 1..20: note = HBV-sgRNA-0614
  source 1..20: mol_type = other DNA
gacttctctcaattttctag

SEQ ID NO: 618 - DNA, 20 bp, synthetic construct
  misc_feature 1..20: note = HBV-sgRNA-0615
  source 1..20: mol_type = other DNA
gagaggcagtagtcggaaca

SEQ ID NO: 619 - DNA, 20 bp, synthetic construct
  misc_feature 1..20: note = HBV-sgRNA-0616
  source 1..20: mol_type = other DNA
gagcagtagtcatgcaggtt

SEQ ID NO: 620 - DNA, 20 bp, synthetic construct
  misc_feature 1..20: note = HBV-sgRNA-0617
  source 1..20: mol_type = other DNA
gagccaagagaaacggactg

SEQ ID NO: 621 - DNA, 20 bp, synthetic construct
  misc_feature 1..20: note = HBV-sgRNA-0618
  source 1..20: mol_type = other DNA
gagccaggagaaacggactg

SEQ ID NO: 622 - DNA, 20 bp, synthetic construct
  misc_feature 1..20: note = HBV-sgRNA-0619
  source 1..20: mol_type = other DNA
gagccaggagaaacgggctg

SEQ ID NO: 623 - DNA, 20 bp, synthetic construct
  misc_feature 1..20: note = HBV-sgRNA-0620
  source 1..20: mol_type = other DNA
gagcgggagcattcgggcca

SEQ ID NO: 624 - DNA, 20 bp, synthetic construct
  misc_feature 1..20: note = HBV-sgRNA-0621
  source 1..20: mol_type = other DNA
gaggcaaatcaggtaggagc

SEQ ID NO: 625 - DNA, 20 bp, synthetic construct
  misc_feature 1..20: note = HBV-sgRNA-0622
  source 1..20: mol_type = other DNA
gaggcaggaggaggagctgc

SEQ ID NO: 626 - DNA, 20 bp, synthetic construct
  misc_feature 1..20: note = HBV-sgRNA-0623
  source 1..20: mol_type = other DNA
gaggcaggaggaggtgctgc

SEQ ID NO: 627 - DNA, 20 bp, synthetic construct
  misc_feature 1..20: note = HBV-sgRNA-0624
  source 1..20: mol_type = other DNA
gaggcaggaggcggatttgc

SEQ ID NO: 628 - DNA, 20 bp, synthetic construct
  misc_feature 1..20: note = HBV-sgRNA-0625
  source 1..20: mol_type = other DNA
gaggtgaagcgaagtgcaca

SEQ ID NO: 629 - DNA, 20 bp, synthetic construct
  misc_feature 1..20: note = HBV-sgRNA-0626
  source 1..20: mol_type = other DNA
gagtcccaagcggccccgag

SEQ ID NO: 630 - DNA, 20 bp, synthetic construct
  misc_feature 1..20: note = HBV-sgRNA-0627
  source 1..20: mol_type = other DNA
gagtgggagcattcgggcca

SEQ ID NO: 631 - DNA, 20 bp, synthetic construct
  misc_feature 1..20: note = HBV-sgRNA-0628
  source 1..20: mol_type = other DNA
gagttggggcacattgccac

SEQ ID NO: 632 - DNA, 20 bp, synthetic construct
  misc_feature 1..20: note = HBV-sgRNA-0629
  source 1..20: mol_type = other DNA
gataaccacattgtgtaaat

SEQ ID NO: 633 - DNA, 20 bp, synthetic construct
  misc_feature 1..20: note = HBV-sgRNA-0630
  source 1..20: mol_type = other DNA
gataagataggggcatttgg

SEQ ID NO: 634 - DNA, 20 bp, synthetic construct
  misc_feature 1..20: note = HBV-sgRNA-0631
  source 1..20: mol_type = other DNA
gataagggagaggcagtagt

SEQ ID NO: 635 - DNA, 20 bp, synthetic construct
  misc_feature 1..20: note = HBV-sgRNA-0632
  source 1..20: mol_type = other DNA
gatagatgtaagcaatttgt

SEQ ID NO: 636 - DNA, 20 bp, synthetic construct
  misc_feature 1..20: note = HBV-sgRNA-0633
  source 1..20: mol_type = other DNA
gatagccacattgtgtaaaa

SEQ ID NO: 637 - DNA, 20 bp, synthetic construct
  misc_feature 1..20: note = HBV-sgRNA-0634
  source 1..20: mol_type = other DNA
gataggataggggcatttgg

SEQ ID NO: 638 - DNA, 20 bp, synthetic construct
  misc_feature 1..20: note = HBV-sgRNA-0635
  source 1..20: mol_type = other DNA
gatatccacattgcgtgaaa

SEQ ID NO: 639 - DNA, 20 bp, synthetic construct
  misc_feature 1..20: note = HBV-sgRNA-0636
  source 1..20: mol_type = other DNA
gatatgggtgaggcagtagt

SEQ ID NO: 640 - DNA, 20 bp, synthetic construct
  misc_feature 1..20: note = HBV-sgRNA-0637
  source 1..20: mol_type = other DNA
gatcggcagaggagccacaa

SEQ ID NO: 641 - DNA, 20 bp, synthetic construct
  misc_feature 1..20: note = HBV-sgRNA-0638
  source 1..20: mol_type = other DNA
gatcggcagaggagccgaaa

SEQ ID NO: 642 - DNA, 20 bp, synthetic construct
  misc_feature 1..20: note = HBV-sgRNA-0639
  source 1..20: mol_type = other DNA
gatcggtagaggagacacaa

SEQ ID NO: 643 - DNA, 20 bp, synthetic construct
  misc_feature 1..20: note = HBV-sgRNA-0640
  source 1..20: mol_type = other DNA
gatcttcgtctgcgaggcga

SEQ ID NO: 644 - DNA, 20 bp, synthetic construct
  misc_feature 1..20: note = HBV-sgRNA-0641
  source 1..20: mol_type = other DNA
gatgaatctagctacctggg

SEQ ID NO: 645 - DNA, 20 bp, synthetic construct
  misc_feature 1..20: note = HBV-sgRNA-0642
  source 1..20: mol_type = other DNA
gatgaatctggccacctggg

SEQ ID NO: 646 - DNA, 20 bp, synthetic construct
  misc_feature 1..20: note = HBV-sgRNA-0643
  source 1..20: mol_type = other DNA
gatgatcggggaagaatccc

SEQ ID NO: 647 - DNA, 20 bp, synthetic construct
  misc_feature 1..20: note = HBV-sgRNA-0644
  source 1..20: mol_type = other DNA
gatgcgatgttctccatgtt

SEQ ID NO: 648 - DNA, 20 bp, synthetic construct
  misc_feature 1..20: note = HBV-sgRNA-0645
  source 1..20: mol_type = other DNA
gatgctccaaattctttata

SEQ ID NO: 649 - DNA, 20 bp, synthetic construct
  misc_feature 1..20: note = HBV-sgRNA-0646
  source 1..20: mol_type = other DNA
gatgttgtgttctccatgtt

SEQ ID NO: 650 - DNA, 20 bp, synthetic construct
  misc_feature 1..20: note = HBV-sgRNA-0647
  source 1..20: mol_type = other DNA
gattgaatacatgcatacaa

SEQ ID NO: 651 - DNA, 20 bp, synthetic construct
  misc_feature 1..20: note = HBV-sgRNA-0648
  source 1..20: mol_type = other DNA
gattgagaccttcgtctgcg

SEQ ID NO: 652 - DNA, 20 bp, synthetic construct
  misc_feature 1..20: note = HBV-sgRNA-0649
  source 1..20: mol_type = other DNA
gattgagatcttcgtctgcg

SEQ ID NO: 653 - DNA, 20 bp, synthetic construct
  misc_feature 1..20: note = HBV-sgRNA-0650
  source 1..20: mol_type = other DNA
gattgagatcttctgcgacg

SEQ ID NO: 654 - DNA, 20 bp, synthetic construct
  misc_feature 1..20: note = HBV-sgRNA-0651
  source 1..20: mol_type = other DNA
gattgatatcttctgcgacg

SEQ ID NO: 655 - DNA, 20 bp, synthetic construct
  misc_feature 1..20: note = HBV-sgRNA-0652
  source 1..20: mol_type = other DNA
gattgtatacatgcatataa

SEQ ID NO: 656 - DNA, 20 bp, synthetic construct
  misc_feature 1..20: note = HBV-sgRNA-0653
  source 1..20: mol_type = other DNA
gcaaaatgaggcgctacgtg

SEQ ID NO: 657 - DNA, 20 bp, synthetic construct
  misc_feature 1..20: note = HBV-sgRNA-0654
  source 1..20: mol_type = other DNA
gcaaacacttggcacagacc

SEQ ID NO: 658 - DNA, 20 bp, synthetic construct
  misc_feature 1..20: note = HBV-sgRNA-0655
  source 1..20: mol_type = other DNA
gcaaatatacatcgtatcca

SEQ ID NO: 659 - DNA, 20 bp, synthetic construct
  misc_feature 1..20: note = HBV-sgRNA-0656
  source 1..20: mol_type = other DNA
gcaacaagagggaaacatag

SEQ ID NO: 660 - DNA, 20 bp, synthetic construct
  misc_feature 1..20: note = HBV-sgRNA-0657
  source 1..20: mol_type = other DNA
gcaacaggagggatacatag

SEQ ID NO: 661 - DNA, 20 bp, synthetic construct
  misc_feature 1..20: note = HBV-sgRNA-0658
  source 1..20: mol_type = other DNA
gcaacatgagggaaacatag

SEQ ID NO: 662 - DNA, 20 bp, synthetic construct
  misc_feature 1..20: note = HBV-sgRNA-0659
  source 1..20: mol_type = other DNA
gcaagcaattctttgctggg

SEQ ID NO: 663 - DNA, 20 bp, synthetic construct
  misc_feature 1..20: note = HBV-sgRNA-0660
  source 1..20: mol_type = other DNA
gcaagtatacatcatttcca

SEQ ID NO: 664 - DNA, 20 bp, synthetic construct
  misc_feature 1..20: note = HBV-sgRNA-0661
  source 1..20: mol_type = other DNA
gcaatttccgtccgaaggtt

SEQ ID NO: 665 - DNA, 20 bp, synthetic construct
  misc_feature 1..20: note = HBV-sgRNA-0662
  source 1..20: mol_type = other DNA
gcacagacctggccgttgcc

SEQ ID NO: 666 - DNA, 20 bp, synthetic construct
  misc_feature 1..20: note = HBV-sgRNA-0663
  source 1..20: mol_type = other DNA
gcagagacagtattctgagc

SEQ ID NO: 667 - DNA, 20 bp, synthetic construct
  misc_feature 1..20: note = HBV-sgRNA-0664
  source 1..20: mol_type = other DNA
gcagagacctgaccgttgcc

SEQ ID NO: 668 - DNA, 20 bp, synthetic construct
  misc_feature 1..20: note = HBV-sgRNA-0665
  source 1..20: mol_type = other DNA
gcagaggtgaaaaagttgca

SEQ ID NO: 669 - DNA, 20 bp, synthetic construct
  misc_feature 1..20: note = HBV-sgRNA-0666
  source 1..20: mol_type = other DNA
gcagatgagaaggcacagac

SEQ ID NO: 670 - DNA, 20 bp, synthetic construct
  misc_feature 1..20: note = HBV-sgRNA-0667
  source 1..20: mol_type = other DNA
gcagcacaccctagcagcca

SEQ ID NO: 671 - DNA, 20 bp, synthetic construct
  misc_feature 1..20: note = HBV-sgRNA-0668
  source 1..20: mol_type = other DNA
gcagcacagcctagcagcca

SEQ ID NO: 672 - DNA, 20 bp, synthetic construct
  misc_feature 1..20: note = HBV-sgRNA-0669
  source 1..20: mol_type = other DNA
gcagggtccaactgatgatc

SEQ ID NO: 673 - DNA, 20 bp, synthetic construct
  misc_feature 1..20: note = HBV-sgRNA-0670
  source 1..20: mol_type = other DNA
gcagggtccaactggtgatc

SEQ ID NO: 674 - DNA, 20 bp, synthetic construct
  misc_feature 1..20: note = HBV-sgRNA-0671
  source 1..20: mol_type = other DNA
gcatacaagggcattaacgc

SEQ ID NO: 675 - DNA, 20 bp, synthetic construct
  misc_feature 1..20: note = HBV-sgRNA-0672
  source 1..20: mol_type = other DNA
gcatataaaggcatcaaggc

SEQ ID NO: 676 - DNA, 20 bp, synthetic construct
  misc_feature 1..20: note = HBV-sgRNA-0673
  source 1..20: mol_type = other DNA
gcatataaaggcattaaagc

SEQ ID NO: 677 - DNA, 20 bp, synthetic construct
  misc_feature 1..20: note = HBV-sgRNA-0674
  source 1..20: mol_type = other DNA
gcatttggtggtctataagc

SEQ ID NO: 678 - DNA, 20 bp, synthetic construct
  misc_feature 1..20: note = HBV-sgRNA-0675
  source 1..20: mol_type = other DNA
gcatttggtggtctatatgc

SEQ ID NO: 679 - DNA, 20 bp, synthetic construct
  misc_feature 1..20: note = HBV-sgRNA-0676
  source 1..20: mol_type = other DNA
gcatttggtggtctgtaagc

SEQ ID NO: 680 - DNA, 20 bp, synthetic construct
  misc_feature 1..20: note = HBV-sgRNA-0677
  source 1..20: mol_type = other DNA
gccaccagcaggaaagtaca

SEQ ID NO: 681 - DNA, 20 bp, synthetic construct
  misc_feature 1..20: note = HBV-sgRNA-0678
  source 1..20: mol_type = other DNA
gccccaaacggccccgagac

SEQ ID NO: 682 - DNA, 20 bp, synthetic construct
  misc_feature 1..20: note = HBV-sgRNA-0679
  source 1..20: mol_type = other DNA
gccccgagacgggtcgtccg

SEQ ID NO: 683 - DNA, 20 bp, synthetic construct
  misc_feature 1..20: note = HBV-sgRNA-0680
  source 1..20: mol_type = other DNA
gccccgagaggggtcgtccg

SEQ ID NO: 684 - DNA, 20 bp, synthetic construct
  misc_feature 1..20: note = HBV-sgRNA-0681
  source 1..20: mol_type = other DNA
gccctgtactttcctgctgg

SEQ ID NO: 685 - DNA, 20 bp, synthetic construct
  misc_feature 1..20: note = HBV-sgRNA-0682
  source 1..20: mol_type = other DNA
gccgcccctttcacgcaatg

SEQ ID NO: 686 - DNA, 20 bp, synthetic construct
  misc_feature 1..20: note = HBV-sgRNA-0683
  source 1..20: mol_type = other DNA
gccggaacggcagatgaaga

SEQ ID NO: 687 - DNA, 20 bp, synthetic construct
  misc_feature 1..20: note = HBV-sgRNA-0684
  source 1..20: mol_type = other DNA
gcctccaccaatcgccagac

SEQ ID NO: 688 - DNA, 20 bp, synthetic construct
  misc_feature 1..20: note = HBV-sgRNA-0685
  source 1..20: mol_type = other DNA
gcctccaccaatcggcagtc

SEQ ID NO: 689 - DNA, 20 bp, synthetic construct
  misc_feature 1..20: note = HBV-sgRNA-0686
  source 1..20: mol_type = other DNA
gcctgctaggttttatccaa

SEQ ID NO: 690 - DNA, 20 bp, synthetic construct
  misc_feature 1..20: note = HBV-sgRNA-0687
  source 1..20: mol_type = other DNA
gcgagggagttcttcttcta

SEQ ID NO: 691 - DNA, 20 bp, synthetic construct
  misc_feature 1..20: note = HBV-sgRNA-0688
  source 1..20: mol_type = other DNA
gcgcatgcgtggaacctttg

SEQ ID NO: 692 - DNA, 20 bp, synthetic construct
  misc_feature 1..20: note = HBV-sgRNA-0689
  source 1..20: mol_type = other DNA
gcgcgtgcgtggaacctttt

SEQ ID NO: 693 - DNA, 20 bp, synthetic construct
  misc_feature 1..20: note = HBV-sgRNA-0690
  source 1..20: mol_type = other DNA
gcgggcggtagagtcccaag

SEQ ID NO: 694 - DNA, 20 bp, synthetic construct
  misc_feature 1..20: note = HBV-sgRNA-0691
  source 1..20: mol_type = other DNA
gctatcgctggatgtgtctg

SEQ ID NO: 695 - DNA, 20 bp, synthetic construct
  misc_feature 1..20: note = HBV-sgRNA-0692
  source 1..20: mol_type = other DNA
gctatgcctcatcttcttgt

SEQ ID NO: 696 - DNA, 20 bp, synthetic construct
  misc_feature 1..20: note = HBV-sgRNA-0693
  source 1..20: mol_type = other DNA
gctcctacctgatttgcctc

SEQ ID NO: 697 - DNA, 20 bp, synthetic construct
  misc_feature 1..20: note = HBV-sgRNA-0694
  source 1..20: mol_type = other DNA
gctcctaccttgttggcgtc

SEQ ID NO: 698 - DNA, 20 bp, synthetic construct
  misc_feature 1..20: note = HBV-sgRNA-0695
  source 1..20: mol_type = other DNA
gctgccaactggatcctgcg

SEQ ID NO: 699 - DNA, 20 bp, synthetic construct
  misc_feature 1..20: note = HBV-sgRNA-0696
  source 1..20: mol_type = other DNA
gctgccccatttacacaatg

SEQ ID NO: 700 - DNA, 20 bp, synthetic construct
  misc_feature 1..20: note = HBV-sgRNA-0697
  source 1..20: mol_type = other DNA
gctgccccttttacacaatg

SEQ ID NO: 701 - DNA, 20 bp, synthetic construct
  misc_feature 1..20: note = HBV-sgRNA-0698
  source 1..20: mol_type = other DNA
gctggatccaactggtggtc

SEQ ID NO: 702 - DNA, 20 bp, synthetic construct
  misc_feature 1..20: note = HBV-sgRNA-0699
  source 1..20: mol_type = other DNA
gctgtgccttgggtggcttt

SEQ ID NO: 703 - DNA, 20 bp, synthetic construct
  misc_feature 1..20: note = HBV-sgRNA-0700
  source 1..20: mol_type = other DNA
gctgtgtttgctctgaaggc

SEQ ID NO: 704 - DNA, 20 bp, synthetic construct
  misc_feature 1..20: note = HBV-sgRNA-0701
  source 1..20: mol_type = other DNA
gcttgtatacatgcatataa

SEQ ID NO: 705 - DNA, 20 bp, synthetic construct
  misc_feature 1..20: note = HBV-sgRNA-0702
  source 1..20: mol_type = other DNA
ggaaagaatcccagaggatt

SEQ ID NO: 706 - DNA, 20 bp, synthetic construct
  misc_feature 1..20: note = HBV-sgRNA-0703
  source 1..20: mol_type = other DNA
ggaaatacacctcctttcca

SEQ ID NO: 707 - DNA, 20 bp, synthetic construct
  misc_feature 1..20: note = HBV-sgRNA-0704
  source 1..20: mol_type = other DNA
ggaacaagatctacagcatg

SEQ ID NO: 708 - DNA, 20 bp, synthetic construct
  misc_feature 1..20: note = HBV-sgRNA-0705
  source 1..20: mol_type = other DNA
ggaacatcaaccaccagcac

SEQ ID NO: 709 - DNA, 20 bp, synthetic construct
  misc_feature 1..20: note = HBV-sgRNA-0706
  source 1..20: mol_type = other DNA
ggaagaatcccaggggattg

SEQ ID NO: 710 - DNA, 20 bp, synthetic construct
  misc_feature 1..20: note = HBV-sgRNA-0707
  source 1..20: mol_type = other DNA
ggaatcgtgcaggtcttgca

SEQ ID NO: 711 - DNA, 20 bp, synthetic construct
  misc_feature 1..20: note = HBV-sgRNA-0708
  source 1..20: mol_type = other DNA
ggacgccaacaaggtgggag

SEQ ID NO: 712 - DNA, 20 bp, synthetic construct
  misc_feature 1..20: note = HBV-sgRNA-0709
  source 1..20: mol_type = other DNA
ggactgaggcccactcccat

SEQ ID NO: 713 - DNA, 20 bp, synthetic construct
  misc_feature 1..20: note = HBV-sgRNA-0710
  source 1..20: mol_type = other DNA
ggacttctctcaattttcta

SEQ ID NO: 714 - DNA, 20 bp, synthetic construct
  misc_feature 1..20: note = HBV-sgRNA-0711
  source 1..20: mol_type = other DNA
ggagaggcagtagtcggaac

SEQ ID NO: 715 - DNA, 20 bp, synthetic construct
  misc_feature 1..20: note = HBV-sgRNA-0712
  source 1..20: mol_type = other DNA
ggagcgggagcattcgggcc

SEQ ID NO: 716 - DNA, 20 bp, synthetic construct
  misc_feature 1..20: note = HBV-sgRNA-0713
  source 1..20: mol_type = other DNA
ggagctggagcattcgggct

SEQ ID NO: 717 - DNA, 20 bp, synthetic construct
  misc_feature 1..20: note = HBV-sgRNA-0714
  source 1..20: mol_type = other DNA
ggaggttggtgagtgattgg

SEQ ID NO: 718 - DNA, 20 bp, synthetic construct
  misc_feature 1..20: note = HBV-sgRNA-0715
  source 1..20: mol_type = other DNA
ggagtgggagcattcgggcc

SEQ ID NO: 719 - DNA, 20 bp, synthetic construct
  misc_feature 1..20: note = HBV-sgRNA-0716
  source 1..20: mol_type = other DNA
ggagttgtgcaggttttgca

SEQ ID NO: 720 - DNA, 20 bp, synthetic construct
  misc_feature 1..20: note = HBV-sgRNA-0717
  source 1..20: mol_type = other DNA
ggataaccacattgtgtaaa

SEQ ID NO: 721 - DNA, 20 bp, synthetic construct
  misc_feature 1..20: note = HBV-sgRNA-0718
  source 1..20: mol_type = other DNA
ggatagccacattgtgtaaa

SEQ ID NO: 722 - DNA, 20 bp, synthetic construct
  misc_feature 1..20: note = HBV-sgRNA-0719
  source 1..20: mol_type = other DNA
ggatatccacattgcgtgaa

SEQ ID NO: 723 - DNA, 20 bp, synthetic construct
  misc_feature 1..20: note = HBV-sgRNA-0720
  source 1..20: mol_type = other DNA
ggatatgtaattggaagttg

SEQ ID NO: 724 - DNA, 20 bp, synthetic construct
  misc_feature 1..20: note = HBV-sgRNA-0721
  source 1..20: mol_type = other DNA
ggatatgtaattgggagttg

SEQ ID NO: 725 - DNA, 20 bp, synthetic construct
  misc_feature 1..20: note = HBV-sgRNA-0722
  source 1..20: mol_type = other DNA
ggatattcccttaacttcat

SEQ ID NO: 726 - DNA, 20 bp, synthetic construct
  misc_feature 1..20: note = HBV-sgRNA-0723
  source 1..20: mol_type = other DNA
ggatcatcaacaaccagcac

SEQ ID NO: 727 - DNA, 20 bp, synthetic construct
  misc_feature 1..20: note = HBV-sgRNA-0724
  source 1..20: mol_type = other DNA
ggatcctcaaccaccagcac

SEQ ID NO: 728 - DNA, 20 bp, synthetic construct
  misc_feature 1..20: note = HBV-sgRNA-0725
  source 1..20: mol_type = other DNA
ggatgactgtctcttagagg

SEQ ID NO: 729 - DNA, 20 bp, synthetic construct
  misc_feature 1..20: note = HBV-sgRNA-0726
  source 1..20: mol_type = other DNA
ggatgagtgtcccttagagg

SEQ ID NO: 730 - DNA, 20 bp, synthetic construct
  misc_feature 1..20: note = HBV-sgRNA-0727
  source 1..20: mol_type = other DNA
ggatgagtgtttctcaaagg

SEQ ID NO: 731 - DNA, 20 bp, synthetic construct
  misc_feature 1..20: note = HBV-sgRNA-0728
  source 1..20: mol_type = other DNA
ggatgatgggatgggaatac

SEQ ID NO: 732 - DNA, 20 bp, synthetic construct
  misc_feature 1..20: note = HBV-sgRNA-0729
  source 1..20: mol_type = other DNA
ggcaaatatttagtaacatt

SEQ ID NO: 733 - DNA, 20 bp, synthetic construct
  misc_feature 1..20: note = HBV-sgRNA-0730
  source 1..20: mol_type = other DNA
ggcaaatatttggtaaggtt

SEQ ID NO: 734 - DNA, 20 bp, synthetic construct
  misc_feature 1..20: note = HBV-sgRNA-0731
  source 1..20: mol_type = other DNA
ggcaagcaattctttgctgg

SEQ ID NO: 735 - DNA, 20 bp, synthetic construct
  misc_feature 1..20: note = HBV-sgRNA-0732
  source 1..20: mol_type = other DNA
ggcacagacctggccgttgc

SEQ ID NO: 736 - DNA, 20 bp, synthetic construct
  misc_feature 1..20: note = HBV-sgRNA-0733
  source 1..20: mol_type = other DNA
ggcagagacctgaccgttgc

SEQ ID NO: 737 - DNA, 20 bp, synthetic construct
  misc_feature 1..20: note = HBV-sgRNA-0734
  source 1..20: mol_type = other DNA
ggcagatgagaaggcacaga

SEQ ID NO: 738 - DNA, 20 bp, synthetic construct
  misc_feature 1..20: note = HBV-sgRNA-0735
  source 1..20: mol_type = other DNA
ggcatagcagcaggatgaag

SEQ ID NO: 739 - DNA, 20 bp, synthetic construct
  misc_feature 1..20: note = HBV-sgRNA-0736
  source 1..20: mol_type = other DNA
ggcatagcagcaggatgcag

SEQ ID NO: 740 - DNA, 20 bp, synthetic construct
  misc_feature 1..20: note = HBV-sgRNA-0737
  source 1..20: mol_type = other DNA
ggcattatttacatactctg

SEQ ID NO: 741 - DNA, 20 bp, synthetic construct
  misc_feature 1..20: note = HBV-sgRNA-0738
  source 1..20: mol_type = other DNA
ggcatttggtggtctgtaag

SEQ ID NO: 742 - DNA, 20 bp, synthetic construct
  misc_feature 1..20: note = HBV-sgRNA-0739
  source 1..20: mol_type = other DNA
ggccaagccccaaccagtgg

SEQ ID NO: 743 - DNA, 20 bp, synthetic construct
  misc_feature 1..20: note = HBV-sgRNA-0740
  source 1..20: mol_type = other DNA
ggccaagccccatccagtgg

SEQ ID NO: 744 - DNA, 20 bp, synthetic construct
  misc_feature 1..20: note = HBV-sgRNA-0741
  source 1..20: mol_type = other DNA
ggcctatattttcctgctgg

SEQ ID NO: 745 - DNA, 20 bp, synthetic construct
  misc_feature 1..20: note = HBV-sgRNA-0742
  source 1..20: mol_type = other DNA
ggcctcccgatacagagcag

SEQ ID NO: 746 - DNA, 20 bp, synthetic construct
  misc_feature 1..20: note = HBV-sgRNA-0743
  source 1..20: mol_type = other DNA
ggcctgtatttccctgctgg

SEQ ID NO: 747 - DNA, 20 bp, synthetic construct
  misc_feature 1..20: note = HBV-sgRNA-0744
  source 1..20: mol_type = other DNA
ggcgagggagttcttcttct

SEQ ID NO: 748 - DNA, 20 bp, synthetic construct
  misc_feature 1..20: note = HBV-sgRNA-0745
  source 1..20: mol_type = other DNA
ggctactcccttaacttcat

SEQ ID NO: 749 - DNA, 20 bp, synthetic construct
  misc_feature 1..20: note = HBV-sgRNA-0746
  source 1..20: mol_type = other DNA
ggctggatccaactggtggt

SEQ ID NO: 750 - DNA, 20 bp, synthetic construct
  misc_feature 1..20: note = HBV-sgRNA-0747
  source 1..20: mol_type = other DNA
ggcttcccgatacagagctg

SEQ ID NO: 751 - DNA, 20 bp, synthetic construct
  misc_feature 1..20: note = HBV-sgRNA-0748
  source 1..20: mol_type = other DNA
ggctttcgcaaaatacctat

SEQ ID NO: 752 - DNA, 20 bp, synthetic construct
  misc_feature 1..20: note = HBV-sgRNA-0749
  source 1..20: mol_type = other DNA
ggctttcgcaagattcctat

SEQ ID NO: 753 - DNA, 20 bp, synthetic construct
  misc_feature 1..20: note = HBV-sgRNA-0750
  source 1..20: mol_type = other DNA
ggctttcggaaaattcctat

SEQ ID NO: 754 - DNA, 20 bp, synthetic construct
  misc_feature 1..20: note = HBV-sgRNA-0751
  source 1..20: mol_type = other DNA
gggaaagaatcccagaggat

SEQ ID NO: 755 - DNA, 20 bp, synthetic construct
  misc_feature 1..20: note = HBV-sgRNA-0752
  source 1..20: mol_type = other DNA
gggaacaagagctacagcat

SEQ ID NO: 756 - DNA, 20 bp, synthetic construct
  misc_feature 1..20: note = HBV-sgRNA-0753
  source 1..20: mol_type = other DNA
gggaacaagatctacagcat

SEQ ID NO: 757 - DNA, 20 bp, synthetic construct
  misc_feature 1..20: note = HBV-sgRNA-0754
  source 1..20: mol_type = other DNA
gggaagaatcccaggggatt

SEQ ID NO: 758 - DNA, 20 bp, synthetic construct
  misc_feature 1..20: note = HBV-sgRNA-0755
  source 1..20: mol_type = other DNA
gggatatgtaattggaagtt

SEQ ID NO: 759 - DNA, 20 bp, synthetic construct
  misc_feature 1..20: note = HBV-sgRNA-0756
  source 1..20: mol_type = other DNA
gggatatgtaattgggagtt

SEQ ID NO: 760 - DNA, 20 bp, synthetic construct
  misc_feature 1..20: note = HBV-sgRNA-0757
  source 1..20: mol_type = other DNA
gggatattcccttaacttca

SEQ ID NO: 761 - DNA, 20 bp, synthetic construct
  misc_feature 1..20: note = HBV-sgRNA-0758
  source 1..20: mol_type = other DNA
gggcaaatatttagtaacat

SEQ ID NO: 762 - DNA, 20 bp, synthetic construct
  misc_feature 1..20: note = HBV-sgRNA-0759
  source 1..20: mol_type = other DNA
gggcaacggggtaaaggttc

SEQ ID NO: 763 - DNA, 20 bp, synthetic construct
  misc_feature 1..20: note = HBV-sgRNA-0760
  source 1..20: mol_type = other DNA
gggcctcagcccgtttctcc

SEQ ID NO: 764 - DNA, 20 bp, synthetic construct
  misc_feature 1..20: note = HBV-sgRNA-0761
  source 1..20: mol_type = other DNA
gggcctcagtccgtttctcc

SEQ ID NO: 765 - DNA, 20 bp, synthetic construct
  misc_feature 1..20: note = HBV-sgRNA-0762
  source 1..20: mol_type = other DNA
gggcctcagtccgtttctct

SEQ ID NO: 766 - DNA, 20 bp, synthetic construct
  misc_feature 1..20: note = HBV-sgRNA-0763
  source 1..20: mol_type = other DNA
gggctactcccttaacttca

SEQ ID NO: 767 - DNA, 20 bp, synthetic construct
  misc_feature 1..20: note = HBV-sgRNA-0764
  source 1..20: mol_type = other DNA
gggctgaggcccactcccat

SEQ ID NO: 768 - DNA, 20 bp, synthetic construct
  misc_feature 1..20: note = HBV-sgRNA-0765
  source 1..20: mol_type = other DNA
gggctttcgcaaaataccta

SEQ ID NO: 769 - DNA, 20 bp, synthetic construct
  misc_feature 1..20: note = HBV-sgRNA-0766
  source 1..20: mol_type = other DNA
gggctttcgcaagattccta

SEQ ID NO: 770 - DNA, 20 bp, synthetic construct
  misc_feature 1..20: note = HBV-sgRNA-0767
  source 1..20: mol_type = other DNA
gggctttcggaaaattccta

SEQ ID NO: 771 - DNA, 20 bp, synthetic construct
  misc_feature 1..20: note = HBV-sgRNA-0768
  source 1..20: mol_type = other DNA
ggggaagaatcccaggggat

SEQ ID NO: 772 - DNA, 20 bp, synthetic construct
  misc_feature 1..20: note = HBV-sgRNA-0769
  source 1..20: mol_type = other DNA
ggggacggtagagccccaaa

SEQ ID NO: 773 - DNA, 20 bp, synthetic construct
  misc_feature 1..20: note = HBV-sgRNA-0770
  source 1..20: mol_type = other DNA
ggggactgcgaattttggcc

SEQ ID NO: 774 - DNA, 20 bp, synthetic construct
  misc_feature 1..20: note = HBV-sgRNA-0771
  source 1..20: mol_type = other DNA
ggggcgcacctctctttacg

SEQ ID NO: 775 - DNA, 20 bp, synthetic construct
  misc_feature 1..20: note = HBV-sgRNA-0772
  source 1..20: mol_type = other DNA
ggggcttggccataggccat

SEQ ID NO: 776 - DNA, 20 bp, synthetic construct
  misc_feature 1..20: note = HBV-sgRNA-0773
  source 1..20: mol_type = other DNA
gggggaacacccgtgtgtct

SEQ ID NO: 777 - DNA, 20 bp, synthetic construct
  misc_feature 1..20: note = HBV-sgRNA-0774
  source 1..20: mol_type = other DNA
gggggaactaccgtgtgtct

SEQ ID NO: 778 - DNA, 20 bp, synthetic construct
  misc_feature 1..20: note = HBV-sgRNA-0775
  source 1..20: mol_type = other DNA
gggggagcacccacgtgtcc

SEQ ID NO: 779 - DNA, 20 bp, synthetic construct
  misc_feature 1..20: note = HBV-sgRNA-0776
  source 1..20: mol_type = other DNA
gggggaggagattagattaa

SEQ ID NO: 780 - DNA, 20 bp, synthetic construct
  misc_feature 1..20: note = HBV-sgRNA-0777
  source 1..20: mol_type = other DNA
gggggaggagattaggttaa

SEQ ID NO: 781 - DNA, 20 bp, synthetic construct
  misc_feature 1..20: note = HBV-sgRNA-0778
  source 1..20: mol_type = other DNA
gggggaggaggttaggttaa

SEQ ID NO: 782 - DNA, 20 bp, synthetic construct
  misc_feature 1..20: note = HBV-sgRNA-0779
  source 1..20: mol_type = other DNA
ggggtggagccctcaggctc

SEQ ID NO: 783 - DNA, 20 bp, synthetic construct
  misc_feature 1..20: note = HBV-sgRNA-0780
  source 1..20: mol_type = other DNA
gggtaggctgccttcctgtc

SEQ ID NO: 784 - DNA, 20 bp, synthetic construct
  misc_feature 1..20: note = HBV-sgRNA-0781
  source 1..20: mol_type = other DNA
gggtggagccctcaggctca

SEQ ID NO: 785 - DNA, 20 bp, synthetic construct
  misc_feature 1..20: note = HBV-sgRNA-0782
  source 1..20: mol_type = other DNA
gggttactctctgaatttta

SEQ ID NO: 786 - DNA, 20 bp, synthetic construct
  misc_feature 1..20: note = HBV-sgRNA-0783
  source 1..20: mol_type = other DNA
gggttcaccccaccacacgg

SEQ ID NO: 787 - DNA, 20 bp, synthetic construct
  misc_feature 1..20: note = HBV-sgRNA-0784
  source 1..20: mol_type = other DNA
gggttcacccctccccatgg

SEQ ID NO: 788 - DNA, 20 bp, synthetic construct
  misc_feature 1..20: note = HBV-sgRNA-0785
  source 1..20: mol_type = other DNA
gggttgcgtcagcaaacact

SEQ ID NO: 789 - DNA, 20 bp, synthetic construct
  misc_feature 1..20: note = HBV-sgRNA-0786
  source 1..20: mol_type = other DNA
ggtaaatatttggtaacctt

SEQ ID NO: 790 - DNA, 20 bp, synthetic construct
  misc_feature 1..20: note = HBV-sgRNA-0787
  source 1..20: mol_type = other DNA
ggtacaataggcggagaagc

SEQ ID NO: 791 - DNA, 20 bp, synthetic construct
  misc_feature 1..20: note = HBV-sgRNA-0788
  source 1..20: mol_type = other DNA
ggtctccatgcgacgtgcag

SEQ ID NO: 792 - DNA, 20 bp, synthetic construct
  misc_feature 1..20: note = HBV-sgRNA-0789
  source 1..20: mol_type = other DNA
ggtctggagcaaacattatc

SEQ ID NO: 793 - DNA, 20 bp, synthetic construct
  misc_feature 1..20: note = HBV-sgRNA-0790
  source 1..20: mol_type = other DNA
ggtctggggcaaacctcatc

SEQ ID NO: 794 - DNA, 20 bp, synthetic construct
  misc_feature 1..20: note = HBV-sgRNA-0791
  source 1..20: mol_type = other DNA
ggtcttgcatggccccgtgc

SEQ ID NO: 795 - DNA, 20 bp, synthetic construct
  misc_feature 1..20: note = HBV-sgRNA-0792
  source 1..20: mol_type = other DNA
ggtgaggcagtagtcggaac

SEQ ID NO: 796 - DNA, 20 bp, synthetic construct
  misc_feature 1..20: note = HBV-sgRNA-0793
  source 1..20: mol_type = other DNA
ggttaccaaatatttaccat

SEQ ID NO: 797 - DNA, 20 bp, synthetic construct
  misc_feature 1..20: note = HBV-sgRNA-0794
  source 1..20: mol_type = other DNA
ggttactctctgaattttat

SEQ ID NO: 798 - DNA, 20 bp, synthetic construct
  misc_feature 1..20: note = HBV-sgRNA-0795
  source 1..20: mol_type = other DNA
ggttatgtcattggaagtta

SEQ ID NO: 799 - DNA, 20 bp, synthetic construct
  misc_feature 1..20: note = HBV-sgRNA-0796
  source 1..20: mol_type = other DNA
ggttcggcatggtcccgtgc

SEQ ID NO: 800 - DNA, 20 bp, synthetic construct
  misc_feature 1..20: note = HBV-sgRNA-0797
  source 1..20: mol_type = other DNA
ggtttaatacccttatccaa

SEQ ID NO: 801 - DNA, 20 bp, synthetic construct
  misc_feature 1..20: note = HBV-sgRNA-0798
  source 1..20: mol_type = other DNA
ggtttaatgcctttgtctaa

SEQ ID NO: 802 - DNA, 20 bp, synthetic construct
  misc_feature 1..20: note = HBV-sgRNA-0799
  source 1..20: mol_type = other DNA
ggtttcaccccaccgcacgg

SEQ ID NO: 803 - DNA, 20 bp, synthetic construct
  misc_feature 1..20: note = HBV-sgRNA-0800
  source 1..20: mol_type = other DNA
ggtttgatccctttatctaa

SEQ ID NO: 804 - DNA, 20 bp, synthetic construct
  misc_feature 1..20: note = HBV-sgRNA-0801
  source 1..20: mol_type = other DNA
ggtttggtacagcaacagga

SEQ ID NO: 805 - DNA, 20 bp, synthetic construct
  misc_feature 1..20: note = HBV-sgRNA-0802
  source 1..20: mol_type = other DNA
ggttttgcatggtccggtgc

SEQ ID NO: 806 - DNA, 20 bp, synthetic construct
  misc_feature 1..20: note = HBV-sgRNA-0803
  source 1..20: mol_type = other DNA
ggttttgtacagcaacaaga

SEQ ID NO: 807 - DNA, 20 bp, synthetic construct
  misc_feature 1..20: note = HBV-sgRNA-0804
  source 1..20: mol_type = other DNA
ggttttgtacagcaacatga

SEQ ID NO: 808 - DNA, 20 bp, synthetic construct
  misc_feature 1..20: note = HBV-sgRNA-0805
  source 1..20: mol_type = other DNA
gtaaactgagccaagagaaa

SEQ ID NO: 809 - DNA, 20 bp, synthetic construct
  misc_feature 1..20: note = HBV-sgRNA-0806
  source 1..20: mol_type = other DNA
gtaaactgagccaggagaaa

SEQ ID NO: 810 - DNA, 20 bp, synthetic construct
  misc_feature 1..20: note = HBV-sgRNA-0807
  source 1..20: mol_type = other DNA
gtaaagagaggtgcgccccg

SEQ ID NO: 811 - DNA, 20 bp, synthetic construct
  misc_feature 1..20: note = HBV-sgRNA-0808
  source 1..20: mol_type = other DNA
gtaacacgagaaggggtcct

SEQ ID NO: 812 - DNA, 20 bp, synthetic construct
  misc_feature 1..20: note = HBV-sgRNA-0809
  source 1..20: mol_type = other DNA
gtaacacgagcaggggtcct

SEQ ID NO: 813 - DNA, 20 bp, synthetic construct
  misc_feature 1..20: note = HBV-sgRNA-0810
  source 1..20: mol_type = other DNA
gtaagaccttgggcaacatt

SEQ ID NO: 814 - DNA, 20 bp, synthetic construct
  misc_feature 1..20: note = HBV-sgRNA-0811
  source 1..20: mol_type = other DNA
gtaagaccttgggcaagacc

SEQ ID NO: 815 - DNA, 20 bp, synthetic construct
  misc_feature 1..20: note = HBV-sgRNA-0812
  source 1..20: mol_type = other DNA
gtagctccaaattctttata

SEQ ID NO: 816 - DNA, 20 bp, synthetic construct
  misc_feature 1..20: note = HBV-sgRNA-0813
  source 1..20: mol_type = other DNA
gtagtatgccctgagcctga

SEQ ID NO: 817 - DNA, 20 bp, synthetic construct
  misc_feature 1..20: note = HBV-sgRNA-0814
  source 1..20: mol_type = other DNA
gtagtcatgcaggttcggca

SEQ ID NO: 818 - DNA, 20 bp, synthetic construct
  misc_feature 1..20: note = HBV-sgRNA-0815
  source 1..20: mol_type = other DNA
gtattcccatcccatcatcc

SEQ ID NO: 819 - DNA, 20 bp, synthetic construct
  misc_feature 1..20: note = HBV-sgRNA-0816
  source 1..20: mol_type = other DNA
gtattcccatcccatcatct

SEQ ID NO: 820 - DNA, 20 bp, synthetic construct
  misc_feature 1..20: note = HBV-sgRNA-0817
  source 1..20: mol_type = other DNA
gtcaatatgccctgagcctg

SEQ ID NO: 821 - DNA, 20 bp, synthetic construct
  misc_feature 1..20: note = HBV-sgRNA-0818
  source 1..20: mol_type = other DNA
gtcaatcttatcgaagactg

SEQ ID NO: 822 - DNA, 20 bp, synthetic construct
  misc_feature 1..20: note = HBV-sgRNA-0819
  source 1..20: mol_type = other DNA
gtcaatcttctcgaggactg

SEQ ID NO: 823 - DNA, 20 bp, synthetic construct
  misc_feature 1..20: note = HBV-sgRNA-0820
  source 1..20: mol_type = other DNA
gtcaatcttctcgaggattg

SEQ ID NO: 824 - DNA, 20 bp, synthetic construct
  misc_feature 1..20: note = HBV-sgRNA-0821
  source 1..20: mol_type = other DNA
gtcatcctcaggccatgcag

SEQ ID NO: 825 - DNA, 20 bp, synthetic construct
  misc_feature 1..20: note = HBV-sgRNA-0822
  source 1..20: mol_type = other DNA
gtcccaagcgaccccgagaa

SEQ ID NO: 826 - DNA, 20 bp, synthetic construct
  misc_feature 1..20: note = HBV-sgRNA-0823
  source 1..20: mol_type = other DNA
gtcccaagcggccccgagag

SEQ ID NO: 827 - DNA, 20 bp, synthetic construct
  misc_feature 1..20: note = HBV-sgRNA-0824
  source 1..20: mol_type = other DNA
gtcccttagaggtggagata

SEQ ID NO: 828 - DNA, 20 bp, synthetic construct
  misc_feature 1..20: note = HBV-sgRNA-0825
  source 1..20: mol_type = other DNA
gtcctcttatgcaagacctt

SEQ ID NO: 829 - DNA, 20 bp, synthetic construct
  misc_feature 1..20: note = HBV-sgRNA-0826
  source 1..20: mol_type = other DNA
gtcctcttatgtaagacctt

SEQ ID NO: 830 - DNA, 20 bp, synthetic construct
  misc_feature 1..20: note = HBV-sgRNA-0827
  source 1..20: mol_type = other DNA
gtcctttgtctacgtcccgt

SEQ ID NO: 831 - DNA, 20 bp, synthetic construct
  misc_feature 1..20: note = HBV-sgRNA-0828
  source 1..20: mol_type = other DNA
gtcctttgtttacgtcccgt

SEQ ID NO: 832 - DNA, 20 bp, synthetic construct
  misc_feature 1..20: note = HBV-sgRNA-0829
  source 1..20: mol_type = other DNA
gtcgcagaagatatcaatct

SEQ ID NO: 833 - DNA, 20 bp, synthetic construct
  misc_feature 1..20: note = HBV-sgRNA-0830
  source 1..20: mol_type = other DNA
gtcgcagaagatctcaatct

SEQ ID NO: 834 - DNA, 20 bp, synthetic construct
  misc_feature 1..20: note = HBV-sgRNA-0831
  source 1..20: mol_type = other DNA
gtcggaacggcagacggaga

SEQ ID NO: 835 - DNA, 20 bp, synthetic construct
  misc_feature 1..20: note = HBV-sgRNA-0832
  source 1..20: mol_type = other DNA
gtctcttagaggtggagaga

SEQ ID NO: 836 - DNA, 20 bp, synthetic construct
  misc_feature 1..20: note = HBV-sgRNA-0833
  source 1..20: mol_type = other DNA
gtctggccaggtgtccttgt

SEQ ID NO: 837 - DNA, 20 bp, synthetic construct
  misc_feature 1..20: note = HBV-sgRNA-0834
  source 1..20: mol_type = other DNA
gtctggcgattggtggaggc

SEQ ID NO: 838 - DNA, 20 bp, synthetic construct
  misc_feature 1..20: note = HBV-sgRNA-0835
  source 1..20: mol_type = other DNA
gtctgtgccttctcatctgc

SEQ ID NO: 839 - DNA, 20 bp, synthetic construct
  misc_feature 1..20: note = HBV-sgRNA-0836
  source 1..20: mol_type = other DNA
gtcttacataagaggactct

SEQ ID NO: 840 - DNA, 20 bp, synthetic construct
  misc_feature 1..20: note = HBV-sgRNA-0837
  source 1..20: mol_type = other DNA
gtcttgcataagaggactct

SEQ ID NO: 841 - DNA, 20 bp, synthetic construct
  misc_feature 1..20: note = HBV-sgRNA-0838
  source 1..20: mol_type = other DNA
gtgaaaaagttgcatggtgc

SEQ ID NO: 842 - DNA, 20 bp, synthetic construct
  misc_feature 1..20: note = HBV-sgRNA-0839
  source 1..20: mol_type = other DNA
gtgaggcagtagtcggaaca

SEQ ID NO: 843 - DNA, 20 bp, synthetic construct
  misc_feature 1..20: note = HBV-sgRNA-0840
  source 1..20: mol_type = other DNA
gtgagtaggccctgagcctg

SEQ ID NO: 844 - DNA, 20 bp, synthetic construct
  misc_feature 1..20: note = HBV-sgRNA-0841
  source 1..20: mol_type = other DNA
gtgctggtggttgaggatcc

SEQ ID NO: 845 - DNA, 20 bp, synthetic construct
  misc_feature 1..20: note = HBV-sgRNA-0842
  source 1..20: mol_type = other DNA
gtgctggtggttgatgttcc

SEQ ID NO: 846 - DNA, 20 bp, synthetic construct
  misc_feature 1..20: note = HBV-sgRNA-0843
  source 1..20: mol_type = other DNA
gtgctggttgttgatgatcc

SEQ ID NO: 847 - DNA, 20 bp, synthetic construct
  misc_feature 1..20: note = HBV-sgRNA-0844
  source 1..20: mol_type = other DNA
gtgggaggagttgggggagg

SEQ ID NO: 848 - DNA, 20 bp, synthetic construct
  misc_feature 1..20: note = HBV-sgRNA-0845
  source 1..20: mol_type = other DNA
gtgttctccatgttcggtgc

SEQ ID NO: 849 - DNA, 20 bp, synthetic construct
  misc_feature 1..20: note = HBV-sgRNA-0846
  source 1..20: mol_type = other DNA
gttatcgctggatgtgtctg

SEQ ID NO: 850 - DNA, 20 bp, synthetic construct
  misc_feature 1..20: note = HBV-sgRNA-0847
  source 1..20: mol_type = other DNA
gttatgtcattggaagttat

SEQ ID NO: 851 - DNA, 20 bp, synthetic construct
  misc_feature 1..20: note = HBV-sgRNA-0848
  source 1..20: mol_type = other DNA
gttcctgtgggcgttcacgg

SEQ ID NO: 852 - DNA, 20 bp, synthetic construct
  misc_feature 1..20: note = HBV-sgRNA-0849
  source 1..20: mol_type = other DNA
gttgaggatcctggaattag

SEQ ID NO: 853 - DNA, 20 bp, synthetic construct
  misc_feature 1..20: note = HBV-sgRNA-0850
  source 1..20: mol_type = other DNA
gttgataagataggggcatt

SEQ ID NO: 854 - DNA, 20 bp, synthetic construct
  misc_feature 1..20: note = HBV-sgRNA-0851
  source 1..20: mol_type = other DNA
gttgataggataggggcatt

SEQ ID NO: 855 - DNA, 20 bp, synthetic construct
  misc_feature 1..20: note = HBV-sgRNA-0852
  source 1..20: mol_type = other DNA
gttgatgaatctagctacct

SEQ ID NO: 856 - DNA, 20 bp, synthetic construct
  misc_feature 1..20: note = HBV-sgRNA-0853
  source 1..20: mol_type = other DNA
gttgatgaatctggccacct

SEQ ID NO: 857 - DNA, 20 bp, synthetic construct
  misc_feature 1..20: note = HBV-sgRNA-0854
  source 1..20: mol_type = other DNA
gttgatgatcctggaattag

SEQ ID NO: 858 - DNA, 20 bp, synthetic construct
  misc_feature 1..20: note = HBV-sgRNA-0855
  source 1..20: mol_type = other DNA
gttgatgttcctggaagtag

SEQ ID NO: 859 - DNA, 20 bp, synthetic construct
  misc_feature 1..20: note = HBV-sgRNA-0856
  source 1..20: mol_type = other DNA
gttgccgagcaacggggtaa

SEQ ID NO: 860 - DNA, 20 bp, synthetic construct
  misc_feature 1..20: note = HBV-sgRNA-0857
  source 1..20: mol_type = other DNA
gttgccgggcaacggggtaa

SEQ ID NO: 861 - DNA, 20 bp, synthetic construct
  misc_feature 1..20: note = HBV-sgRNA-0858
  source 1..20: mol_type = other DNA
gttggtgagtgattggaggt

SEQ ID NO: 862 - DNA, 20 bp, synthetic construct
  misc_feature 1..20: note = HBV-sgRNA-0859
  source 1..20: mol_type = other DNA
gtttaaagactgggaggagt

SEQ ID NO: 863 - DNA, 20 bp, synthetic construct
  misc_feature 1..20: note = HBV-sgRNA-0860
  source 1..20: mol_type = other DNA
gtttactgagtgggaggagt

SEQ ID NO: 864 - DNA, 20 bp, synthetic construct
  misc_feature 1..20: note = HBV-sgRNA-0861
  source 1..20: mol_type = other DNA
gttttgctcgcagcaggtct

SEQ ID NO: 865 - DNA, 20 bp, synthetic construct
  misc_feature 1..20: note = HBV-sgRNA-0862
  source 1..20: mol_type = other DNA
taaaaatcagacaactattg

SEQ ID NO: 866 - DNA, 20 bp, synthetic construct
  misc_feature 1..20: note = HBV-sgRNA-0863
  source 1..20: mol_type = other DNA
taaaaatcagacaactcttg

SEQ ID NO: 867 - DNA, 20 bp, synthetic construct
  misc_feature 1..20: note = HBV-sgRNA-0864
  source 1..20: mol_type = other DNA
taaaattaattatgcctgct

SEQ ID NO: 868 - DNA, 20 bp, synthetic construct
  misc_feature 1..20: note = HBV-sgRNA-0865
  source 1..20: mol_type = other DNA
taaactgagccaggagaaac

SEQ ID NO: 869 - DNA, 20 bp, synthetic construct
  misc_feature 1..20: note = HBV-sgRNA-0866
  source 1..20: mol_type = other DNA
taaagaatttggagcatctg

SEQ ID NO: 870 - DNA, 20 bp, synthetic construct
  misc_feature 1..20: note = HBV-sgRNA-0867
  source 1..20: mol_type = other DNA
taaagaatttggagctactg

SEQ ID NO: 871 - DNA, 20 bp, synthetic construct
  misc_feature 1..20: note = HBV-sgRNA-0868
  source 1..20: mol_type = other DNA
taaagaatttggagcttctg

SEQ ID NO: 872 - DNA, 20 bp, synthetic construct
  misc_feature 1..20: note = HBV-sgRNA-0869
  source 1..20: mol_type = other DNA
taaagactgggaggagttgg

SEQ ID NO: 873 - DNA, 20 bp, synthetic construct
  misc_feature 1..20: note = HBV-sgRNA-0870
  source 1..20: mol_type = other DNA
taaagttcaggcaactcttg

SEQ ID NO: 874 - DNA, 20 bp, synthetic construct
  misc_feature 1..20: note = HBV-sgRNA-0871
  source 1..20: mol_type = other DNA
taaatgaatgtgaggaaagg

SEQ ID NO: 875 - DNA, 20 bp, synthetic construct
  misc_feature 1..20: note = HBV-sgRNA-0872
  source 1..20: mol_type = other DNA
taactgaaagccaaacagtg

SEQ ID NO: 876 - DNA, 20 bp, synthetic construct
  misc_feature 1..20: note = HBV-sgRNA-0873
  source 1..20: mol_type = other DNA
taactgaaagccagacagtg

SEQ ID NO: 877 - DNA, 20 bp, synthetic construct
  misc_feature 1..20: note = HBV-sgRNA-0874
  source 1..20: mol_type = other DNA
taatagatgtcaacaatatg

SEQ ID NO: 878 - DNA, 20 bp, synthetic construct
  misc_feature 1..20: note = HBV-sgRNA-0875
  source 1..20: mol_type = other DNA
taatgattaactacatactc

SEQ ID NO: 879 - DNA, 20 bp, synthetic construct
  misc_feature 1..20: note = HBV-sgRNA-0876
  source 1..20: mol_type = other DNA
taatgattaactagatgttc

SEQ ID NO: 880 - DNA, 20 bp, synthetic construct
  misc_feature 1..20: note = HBV-sgRNA-0877
  source 1..20: mol_type = other DNA
taatgattaactgcatgttc

SEQ ID NO: 881 - DNA, 20 bp, synthetic construct
  misc_feature 1..20: note = HBV-sgRNA-0878
  source 1..20: mol_type = other DNA
tacacactctttggaaggcg

SEQ ID NO: 882 - DNA, 20 bp, synthetic construct
  misc_feature 1..20: note = HBV-sgRNA-0879
  source 1..20: mol_type = other DNA
tacatatcccatgaagttaa

SEQ ID NO: 883 - DNA, 20 bp, synthetic construct
  misc_feature 1..20: note = HBV-sgRNA-0880
  source 1..20: mol_type = other DNA
taccaattttcttttgtctt

SEQ ID NO: 884 - DNA, 20 bp, synthetic construct
  misc_feature 1..20: note = HBV-sgRNA-0881
  source 1..20: mol_type = other DNA
taccacagagtctagactcg

SEQ ID NO: 885 - DNA, 20 bp, synthetic construct
  misc_feature 1..20: note = HBV-sgRNA-0882
  source 1..20: mol_type = other DNA
taccgcagagtctagactcg

SEQ ID NO: 886 - DNA, 20 bp, synthetic construct
  misc_feature 1..20: note = HBV-sgRNA-0883
  source 1..20: mol_type = other DNA
taccgcctcagctctgtatc

SEQ ID NO: 887 - DNA, 20 bp, synthetic construct
  misc_feature 1..20: note = HBV-sgRNA-0884
  source 1..20: mol_type = other DNA
tacctgggtgggaagtaatt

SEQ ID NO: 888 - DNA, 20 bp, synthetic construct
  misc_feature 1..20: note = HBV-sgRNA-0885
  source 1..20: mol_type = other DNA
tacctgggtgggtgttaatt

SEQ ID NO: 889 - DNA, 20 bp, synthetic construct
  misc_feature 1..20: note = HBV-sgRNA-0886
  source 1..20: mol_type = other DNA
tacctgtctttaatcccgag

SEQ ID NO: 890 - DNA, 20 bp, synthetic construct
  misc_feature 1..20: note = HBV-sgRNA-0887
  source 1..20: mol_type = other DNA
tacctgtctttaatcctcat

SEQ ID NO: 891 - DNA, 20 bp, synthetic construct
  misc_feature 1..20: note = HBV-sgRNA-0888
  source 1..20: mol_type = other DNA
taccttgctttaatcctaaa

SEQ ID NO: 892 - DNA, 20 bp, synthetic construct
  misc_feature 1..20: note = HBV-sgRNA-0889
  source 1..20: mol_type = other DNA
taccttgttggcgtctggcc

SEQ ID NO: 893 - DNA, 20 bp, synthetic construct
  misc_feature 1..20: note = HBV-sgRNA-0890
  source 1..20: mol_type = other DNA
tacggggctttattcttcta

SEQ ID NO: 894 - DNA, 20 bp, synthetic construct
  misc_feature 1..20: note = HBV-sgRNA-0891
  source 1..20: mol_type = other DNA
tactagtgccatttgttcag

SEQ ID NO: 895 - DNA, 20 bp, synthetic construct
  misc_feature 1..20: note = HBV-sgRNA-0892
  source 1..20: mol_type = other DNA
tactgagtgggaggagttgg

SEQ ID NO: 896 - DNA, 20 bp, synthetic construct
  misc_feature 1..20: note = HBV-sgRNA-0893
  source 1..20: mol_type = other DNA
tactttctcgccaacttaca

SEQ ID NO: 897 - DNA, 20 bp, synthetic construct
  misc_feature 1..20: note = HBV-sgRNA-0894
  source 1..20: mol_type = other DNA
tagctccaaattctttataa

SEQ ID NO: 898 - DNA, 20 bp, synthetic construct
  misc_feature 1..20: note = HBV-sgRNA-0895
  source 1..20: mol_type = other DNA
tagcttgcctgagtgccgta

SEQ ID NO: 899 - DNA, 20 bp, synthetic construct
  misc_feature 1..20: note = HBV-sgRNA-0896
  source 1..20: mol_type = other DNA
tagcttgcctgagtgctgta

SEQ ID NO: 900 - DNA, 20 bp, synthetic construct
  misc_feature 1..20: note = HBV-sgRNA-0897
  source 1..20: mol_type = other DNA
taggaatcttgcgaaagccc

SEQ ID NO: 901 - DNA, 20 bp, synthetic construct
  misc_feature 1..20: note = HBV-sgRNA-0898
  source 1..20: mol_type = other DNA
taggaattttccgaaagccc

SEQ ID NO: 902 - DNA, 20 bp, synthetic construct
  misc_feature 1..20: note = HBV-sgRNA-0899
  source 1..20: mol_type = other DNA
tagggctttcccccactgtc

SEQ ID NO: 903 - DNA, 20 bp, synthetic construct
  misc_feature 1..20: note = HBV-sgRNA-0900
  source 1..20: mol_type = other DNA
tagggctttcccccactgtt

SEQ ID NO: 904 - DNA, 20 bp, synthetic construct
  misc_feature 1..20: note = HBV-sgRNA-0901
  source 1..20: mol_type = other DNA
tagtatcccttggactcata

SEQ ID NO: 905 - DNA, 20 bp, synthetic construct
  misc_feature 1..20: note = HBV-sgRNA-0902
  source 1..20: mol_type = other DNA
tagtattccttggacacata

SEQ ID NO: 906 - DNA, 20 bp, synthetic construct
  misc_feature 1..20: note = HBV-sgRNA-0903
  source 1..20: mol_type = other DNA
tagtattccttggactcata

SEQ ID NO: 907 - DNA, 20 bp, synthetic construct
  misc_feature 1..20: note = HBV-sgRNA-0904
  source 1..20: mol_type = other DNA
tagtttccggaagtgttgat

SEQ ID NO: 908 - DNA, 20 bp, synthetic construct
  misc_feature 1..20: note = HBV-sgRNA-0905
  source 1..20: mol_type = other DNA
tataactgaaagccaaacag

SEQ ID NO: 909 - DNA, 20 bp, synthetic construct
  misc_feature 1..20: note = HBV-sgRNA-0906
  source 1..20: mol_type = other DNA
tataactgaaagccagacag

SEQ ID NO: 910 - DNA, 20 bp, synthetic construct
  misc_feature 1..20: note = HBV-sgRNA-0907
  source 1..20: mol_type = other DNA
tatatggatgatgtggtatt

SEQ ID NO: 911 - DNA, 20 bp, synthetic construct
  misc_feature 1..20: note = HBV-sgRNA-0908
  source 1..20: mol_type = other DNA
tatatggatgatgtggtttt

SEQ ID NO: 912 - DNA, 20 bp, synthetic construct
  misc_feature 1..20: note = HBV-sgRNA-0909
  source 1..20: mol_type = other DNA
tatcccttggactcataagg

SEQ ID NO: 913 - DNA, 20 bp, synthetic construct
  misc_feature 1..20: note = HBV-sgRNA-0910
  source 1..20: mol_type = other DNA
tatgatgtgttcttgtggca

SEQ ID NO: 914 - DNA, 20 bp, synthetic construct
  misc_feature 1..20: note = HBV-sgRNA-0911
  source 1..20: mol_type = other DNA
tatggatgatgtggtattgg

SEQ ID NO: 915 - DNA, 20 bp, synthetic construct
  misc_feature 1..20: note = HBV-sgRNA-0912
  source 1..20: mol_type = other DNA
tatggatgatgtggttttgg

SEQ ID NO: 916 - DNA, 20 bp, synthetic construct
  misc_feature 1..20: note = HBV-sgRNA-0913
  source 1..20: mol_type = other DNA
tatggccaagccccaaccag

SEQ ID NO: 917 - DNA, 20 bp, synthetic construct
  misc_feature 1..20: note = HBV-sgRNA-0914
  source 1..20: mol_type = other DNA
tatggccaagccccatccag

SEQ ID NO: 918 - DNA, 20 bp, synthetic construct
  misc_feature 1..20: note = HBV-sgRNA-0915
  source 1..20: mol_type = other DNA
tattcccatcccatcatcct

SEQ ID NO: 919 - DNA, 20 bp, synthetic construct
  misc_feature 1..20: note = HBV-sgRNA-0916
  source 1..20: mol_type = other DNA
tattcccatcccatcatctt

SEQ ID NO: 920 - DNA, 20 bp, synthetic construct
  misc_feature 1..20: note = HBV-sgRNA-0917
  source 1..20: mol_type = other DNA
tattccttggacacataagg

SEQ ID NO: 921 - DNA, 20 bp, synthetic construct
  misc_feature 1..20: note = HBV-sgRNA-0918
  source 1..20: mol_type = other DNA
tattccttggactcataagg

SEQ ID NO: 922 - DNA, 20 bp, synthetic construct
  misc_feature 1..20: note = HBV-sgRNA-0919
  source 1..20: mol_type = other DNA
tattgtaccggccgaccacg

SEQ ID NO: 923 - DNA, 20 bp, synthetic construct
  misc_feature 1..20: note = HBV-sgRNA-0920
  source 1..20: mol_type = other DNA
tcaaagaattgtgggtcttt

SEQ ID NO: 924 - DNA, 20 bp, synthetic construct
  misc_feature 1..20: note = HBV-sgRNA-0921
  source 1..20: mol_type = other DNA
tcaaccccaacaaggatcac

SEQ ID NO: 925 - DNA, 20 bp, synthetic construct
  misc_feature 1..20: note = HBV-sgRNA-0922
  source 1..20: mol_type = other DNA
tcaacccgcacaaggacaac

SEQ ID NO: 926 - DNA, 20 bp, synthetic construct
  misc_feature 1..20: note = HBV-sgRNA-0923
  source 1..20: mol_type = other DNA
tcaacgaattgtgggtcttt

SEQ ID NO: 927 - DNA, 20 bp, synthetic construct
  misc_feature 1..20: note = HBV-sgRNA-0924
  source 1..20: mol_type = other DNA
tcaatatgccctgagcctga

SEQ ID NO: 928 - DNA, 20 bp, synthetic construct
  misc_feature 1..20: note = HBV-sgRNA-0925
  source 1..20: mol_type = other DNA
tcaatcccaacaaggacacc

SEQ ID NO: 929 - DNA, 20 bp, synthetic construct
  misc_feature 1..20: note = HBV-sgRNA-0926
  source 1..20: mol_type = other DNA
tcactggccagaggcaaatc

SEQ ID NO: 930 - DNA, 20 bp, synthetic construct
  misc_feature 1..20: note = HBV-sgRNA-0927
  source 1..20: mol_type = other DNA
tcaggcaagcaattctttgc

SEQ ID NO: 931 - DNA, 20 bp, synthetic construct
  misc_feature 1..20: note = HBV-sgRNA-0928
  source 1..20: mol_type = other DNA
tcaggcaagctatcctgtgt

SEQ ID NO: 932 - DNA, 20 bp, synthetic construct
  misc_feature 1..20: note = HBV-sgRNA-0929
  source 1..20: mol_type = other DNA
tcaggcaagctattctgtgt

SEQ ID NO: 933 - DNA, 20 bp, synthetic construct
  misc_feature 1..20: note = HBV-sgRNA-0930
  source 1..20: mol_type = other DNA
tcatcaactcaccccaacac

SEQ ID NO: 934 - DNA, 20 bp, synthetic construct
  misc_feature 1..20: note = HBV-sgRNA-0931
  source 1..20: mol_type = other DNA
tccaaacctcgaaaaggcat

SEQ ID NO: 935 - DNA, 20 bp, synthetic construct
  misc_feature 1..20: note = HBV-sgRNA-0932
  source 1..20: mol_type = other DNA
tccaaacctcgacaaggcat

SEQ ID NO: 936 - DNA, 20 bp, synthetic construct
  misc_feature 1..20: note = HBV-sgRNA-0933
  source 1..20: mol_type = other DNA
tccaaggaatactaacattg

SEQ ID NO: 937 - DNA, 20 bp, synthetic construct
  misc_feature 1..20: note = HBV-sgRNA-0934
  source 1..20: mol_type = other DNA
tccacattgcgtgaaagggg

SEQ ID NO: 938 - DNA, 20 bp, synthetic construct
  misc_feature 1..20: note = HBV-sgRNA-0935
  source 1..20: mol_type = other DNA
tccaccccaacagtccccca

SEQ ID NO: 939 - DNA, 20 bp, synthetic construct
  misc_feature 1..20: note = HBV-sgRNA-0936
  source 1..20: mol_type = other DNA
tcccgcggacgacccctctc

SEQ ID NO: 940 - DNA, 20 bp, synthetic construct
  misc_feature 1..20: note = HBV-sgRNA-0937
  source 1..20: mol_type = other DNA
tcccgcggacgacccgtctc

SEQ ID NO: 941 - DNA, 20 bp, synthetic construct
  misc_feature 1..20: note = HBV-sgRNA-0938
  source 1..20: mol_type = other DNA
tcccttagaggtggagataa

SEQ ID NO: 942 - DNA, 20 bp, synthetic construct
  misc_feature 1..20: note = HBV-sgRNA-0939
  source 1..20: mol_type = other DNA
tcccttatctccacctctaa

SEQ ID NO: 943 - DNA, 20 bp, synthetic construct
  misc_feature 1..20: note = HBV-sgRNA-0940
  source 1..20: mol_type = other DNA
tccgcaggattcagcgccga

SEQ ID NO: 944 - DNA, 20 bp, synthetic construct
  misc_feature 1..20: note = HBV-sgRNA-0941
  source 1..20: mol_type = other DNA
tccgcagtatggatcggcag

SEQ ID NO: 945 - DNA, 20 bp, synthetic construct
  misc_feature 1..20: note = HBV-sgRNA-0942
  source 1..20: mol_type = other DNA
tccgcagtatggatcggtag

SEQ ID NO: 946 - DNA, 20 bp, synthetic construct
  misc_feature 1..20: note = HBV-sgRNA-0943
  source 1..20: mol_type = other DNA
tccgcgggattcagcgccga

SEQ ID NO: 947 - DNA, 20 bp, synthetic construct
  misc_feature 1..20: note = HBV-sgRNA-0944
  source 1..20: mol_type = other DNA
tccggaagagttgataagat

SEQ ID NO: 948 - DNA, 20 bp, synthetic construct
  misc_feature 1..20: note = HBV-sgRNA-0945
  source 1..20: mol_type = other DNA
tccggaagtgttgataagat

SEQ ID NO: 949 - DNA, 20 bp, synthetic construct
  misc_feature 1..20: note = HBV-sgRNA-0946
  source 1..20: mol_type = other DNA
tccggaagtgttgataggat

SEQ ID NO: 950 - DNA, 20 bp, synthetic construct
  misc_feature 1..20: note = HBV-sgRNA-0947
  source 1..20: mol_type = other DNA
tccggccagttgtccttgtg

SEQ ID NO: 951 - DNA, 20 bp, synthetic construct
  misc_feature 1..20: note = HBV-sgRNA-0948
  source 1..20: mol_type = other DNA
tcctcacattcatttacagg

SEQ ID NO: 952 - DNA, 20 bp, synthetic construct
  misc_feature 1..20: note = HBV-sgRNA-0949
  source 1..20: mol_type = other DNA
tcctcctgcaaatgaatgtc

SEQ ID NO: 953 - DNA, 20 bp, synthetic construct
  misc_feature 1..20: note = HBV-sgRNA-0950
  source 1..20: mol_type = other DNA
tcctcctgtaaatgaatgtg

SEQ ID NO: 954 - DNA, 20 bp, synthetic construct
  misc_feature 1..20: note = HBV-sgRNA-0951
  source 1..20: mol_type = other DNA
tcctctaccgatccatactg

SEQ ID NO: 955 - DNA, 20 bp, synthetic construct
  misc_feature 1..20: note = HBV-sgRNA-0952
  source 1..20: mol_type = other DNA
tcctctgccgatccatactg

SEQ ID NO: 956 - DNA, 20 bp, synthetic construct
  misc_feature 1..20: note = HBV-sgRNA-0953
  source 1..20: mol_type = other DNA
tcctgacattcatttgcagg

SEQ ID NO: 957 - DNA, 20 bp, synthetic construct
  misc_feature 1..20: note = HBV-sgRNA-0954
  source 1..20: mol_type = other DNA
tcctgactgccgattggtgg

SEQ ID NO: 958 - DNA, 20 bp, synthetic construct
  misc_feature 1..20: note = HBV-sgRNA-0955
  source 1..20: mol_type = other DNA
tcctgcggacgacccttctc

SEQ ID NO: 959 - DNA, 20 bp, synthetic construct
  misc_feature 1..20: note = HBV-sgRNA-0956
  source 1..20: mol_type = other DNA
tcctggaagtagaggacaaa

SEQ ID NO: 960 - DNA, 20 bp, synthetic construct
  misc_feature 1..20: note = HBV-sgRNA-0957
  source 1..20: mol_type = other DNA
tcctggaattagaggacaaa

SEQ ID NO: 961 - DNA, 20 bp, synthetic construct
  misc_feature 1..20: note = HBV-sgRNA-0958
  source 1..20: mol_type = other DNA
tcctgtcctccaacttgtcc

SEQ ID NO: 962 - DNA, 20 bp, synthetic construct
  misc_feature 1..20: note = HBV-sgRNA-0959
  source 1..20: mol_type = other DNA
tcctgtctggcgattggtgg

SEQ ID NO: 963 - DNA, 20 bp, synthetic construct
  misc_feature 1..20: note = HBV-sgRNA-0960
  source 1..20: mol_type = other DNA
tcctgttttcatttactgta

SEQ ID NO: 964 - DNA, 20 bp, synthetic construct
  misc_feature 1..20: note = HBV-sgRNA-0961
  source 1..20: mol_type = other DNA
tccttgagcaggaatcgtgc

SEQ ID NO: 965 - DNA, 20 bp, synthetic construct
  misc_feature 1..20: note = HBV-sgRNA-0962
  source 1..20: mol_type = other DNA
tccttgagcaggagttgtgc

SEQ ID NO: 966 - DNA, 20 bp, synthetic construct
  misc_feature 1..20: note = HBV-sgRNA-0963
  source 1..20: mol_type = other DNA
tccttgagcagtagtcatgc

SEQ ID NO: 967 - DNA, 20 bp, synthetic construct
  misc_feature 1..20: note = HBV-sgRNA-0964
  source 1..20: mol_type = other DNA
tcgaggagatctcgaataga

SEQ ID NO: 968 - DNA, 20 bp, synthetic construct
  misc_feature 1..20: note = HBV-sgRNA-0965
  source 1..20: mol_type = other DNA
tcgcaaaatacctatgggag

SEQ ID NO: 969 - DNA, 20 bp, synthetic construct
  misc_feature 1..20: note = HBV-sgRNA-0966
  source 1..20: mol_type = other DNA
tcgcaagattcctatgggag

SEQ ID NO: 970 - DNA, 20 bp, synthetic construct
  misc_feature 1..20: note = HBV-sgRNA-0967
  source 1..20: mol_type = other DNA
tcgcagaagatatcaatctc

SEQ ID NO: 971 - DNA, 20 bp, synthetic construct
  misc_feature 1..20: note = HBV-sgRNA-0968
  source 1..20: mol_type = other DNA
tcgcagaagatctcaatctc

SEQ ID NO: 972 - DNA, 20 bp, synthetic construct
  misc_feature 1..20: note = HBV-sgRNA-0969
  source 1..20: mol_type = other DNA
tcggaaaattcctatgggag

SEQ ID NO: 973 - DNA, 20 bp, synthetic construct
  misc_feature 1..20: note = HBV-sgRNA-0970
  source 1..20: mol_type = other DNA
tcggaacggcagacggagaa

SEQ ID NO: 974 - DNA, 20 bp, synthetic construct
  misc_feature 1..20: note = HBV-sgRNA-0971
  source 1..20: mol_type = other DNA
tcggcatggtcccgtgctgg

SEQ ID NO: 975 - DNA, 20 bp, synthetic construct
  misc_feature 1..20: note = HBV-sgRNA-0972
  source 1..20: mol_type = other DNA
tcgggaggccttagagtctc

SEQ ID NO: 976 - DNA, 20 bp, synthetic construct
  misc_feature 1..20: note = HBV-sgRNA-0973
  source 1..20: mol_type = other DNA
tcgtcaatcttatcgaagac

SEQ ID NO: 977 - DNA, 20 bp, synthetic construct
  misc_feature 1..20: note = HBV-sgRNA-0974
  source 1..20: mol_type = other DNA
tcgtcaatcttctcgaggac

SEQ ID NO: 978 - DNA, 20 bp, synthetic construct
  misc_feature 1..20: note = HBV-sgRNA-0975
  source 1..20: mol_type = other DNA
tcgtcaatcttctcgaggat

SEQ ID NO: 979 - DNA, 20 bp, synthetic construct
  misc_feature 1..20: note = HBV-sgRNA-0976
  source 1..20: mol_type = other DNA
tctaagagacagtcatcctc

SEQ ID NO: 980 - DNA, 20 bp, synthetic construct
  misc_feature 1..20: note = HBV-sgRNA-0977
  source 1..20: mol_type = other DNA
tctaagggacactcatcctc

SEQ ID NO: 981 - DNA, 20 bp, synthetic construct
  misc_feature 1..20: note = HBV-sgRNA-0978
  source 1..20: mol_type = other DNA
tctagaagatctcgtactga

SEQ ID NO: 982 - DNA, 20 bp, synthetic construct
  misc_feature 1..20: note = HBV-sgRNA-0979
  source 1..20: mol_type = other DNA
tctcaaaggtggagacagcg

SEQ ID NO: 983 - DNA, 20 bp, synthetic construct
  misc_feature 1..20: note = HBV-sgRNA-0980
  source 1..20: mol_type = other DNA
tctcttagaggtggagagat

SEQ ID NO: 984 - DNA, 20 bp, synthetic construct
  misc_feature 1..20: note = HBV-sgRNA-0981
  source 1..20: mol_type = other DNA
tctgagttggctttgaatgc

SEQ ID NO: 985 - DNA, 20 bp, synthetic construct
  misc_feature 1..20: note = HBV-sgRNA-0982
  source 1..20: mol_type = other DNA
tctgccgttccgaccgacca

SEQ ID NO: 986 - DNA, 20 bp, synthetic construct
  misc_feature 1..20: note = HBV-sgRNA-0983
  source 1..20: mol_type = other DNA
tctgccgttccggccgacca

SEQ ID NO: 987 - DNA, 20 bp, synthetic construct
  misc_feature 1..20: note = HBV-sgRNA-0984
  source 1..20: mol_type = other DNA
tctgctagatcccagagtga

SEQ ID NO: 988 - DNA, 20 bp, synthetic construct
  misc_feature 1..20: note = HBV-sgRNA-0985
  source 1..20: mol_type = other DNA
tctggccaggtgtccttgtt

SEQ ID NO: 989 - DNA, 20 bp, synthetic construct
  misc_feature 1..20: note = HBV-sgRNA-0986
  source 1..20: mol_type = other DNA
tctggccagtgatccttgtt

SEQ ID NO: 990 - DNA, 20 bp, synthetic construct
  misc_feature 1..20: note = HBV-sgRNA-0987
  source 1..20: mol_type = other DNA
tcttatgcaagaccttgggc

SEQ ID NO: 991 - DNA, 20 bp, synthetic construct
  misc_feature 1..20: note = HBV-sgRNA-0988
  source 1..20: mol_type = other DNA
tcttcaagatcccagagtca

SEQ ID NO: 992 - DNA, 20 bp, synthetic construct
  misc_feature 1..20: note = HBV-sgRNA-0989
  source 1..20: mol_type = other DNA
tcttcctgactgccgattgg

SEQ ID NO: 993 - DNA, 20 bp, synthetic construct
  misc_feature 1..20: note = HBV-sgRNA-0990
  source 1..20: mol_type = other DNA
tcttggtgtaaatgtatatt

SEQ ID NO: 994 - DNA, 20 bp, synthetic construct
  misc_feature 1..20: note = HBV-sgRNA-0991
  source 1..20: mol_type = other DNA
tcttgtcctccaatttgtcc

SEQ ID NO: 995 - DNA, 20 bp, synthetic construct
  misc_feature 1..20: note = HBV-sgRNA-0992
  source 1..20: mol_type = other DNA
tctttccaccagcaatcctc

SEQ ID NO: 996 - DNA, 20 bp, synthetic construct
  misc_feature 1..20: note = HBV-sgRNA-0993
  source 1..20: mol_type = other DNA
tctttctgtccccaatcccc

SEQ ID NO: 997 - DNA, 20 bp, synthetic construct
  misc_feature 1..20: note = HBV-sgRNA-0994
  source 1..20: mol_type = other DNA
tctttctgttcccaatcctc

SEQ ID NO: 998 - DNA, 20 bp, synthetic construct
  misc_feature 1..20: note = HBV-sgRNA-0995
  source 1..20: mol_type = other DNA
tctttgtactaggaggctgt

SEQ ID NO: 999 - DNA, 20 bp, synthetic construct
  misc_feature 1..20: note = HBV-sgRNA-0996
  source 1..20: mol_type = other DNA
tcttttggggtggagccctc

SEQ ID NO: 1000 - DNA, 20 bp, synthetic construct
  misc_feature 1..20: note = HBV-sgRNA-0997
  source 1..20: mol_type = other DNA
tgaaattaattatgcctgct

SEQ ID NO: 1001 - DNA, 20 bp, synthetic construct
  misc_feature 1..20: note = HBV-sgRNA-0998
  source 1..20: mol_type = other DNA
tgaacctttaccccgttgcc

SEQ ID NO: 1002 - DNA, 20 bp, synthetic construct
  misc_feature 1..20: note = HBV-sgRNA-0999
  source 1..20: mol_type = other DNA
tgaacctttaccccgttgct

SEQ ID NO: 1003 - DNA, 20 bp, synthetic construct
  misc_feature 1..20: note = HBV-sgRNA-1000
  source 1..20: mol_type = other DNA
tgaaggctggatccaactgg

SEQ ID NO: 1004 - DNA, 20 bp, synthetic construct
  misc_feature 1..20: note = HBV-sgRNA-1001
  source 1..20: mol_type = other DNA
tgacagactttccaatcaat

SEQ ID NO: 1005 - DNA, 20 bp, synthetic construct
  misc_feature 1..20: note = HBV-sgRNA-1002
  source 1..20: mol_type = other DNA
tgacatactttccaatcaat

SEQ ID NO: 1006 - DNA, 20 bp, synthetic construct
  misc_feature 1..20: note = HBV-sgRNA-1003
  source 1..20: mol_type = other DNA
tgaccaagccccagccagtg

SEQ ID NO: 1007 - DNA, 20 bp, synthetic construct
  misc_feature 1..20: note = HBV-sgRNA-1004
  source 1..20: mol_type = other DNA
tgacgcaacccccactggat

SEQ ID NO: 1008 - DNA, 20 bp, synthetic construct
  misc_feature 1..20: note = HBV-sgRNA-1005
  source 1..20: mol_type = other DNA
tgacgcaacccccactggct

SEQ ID NO: 1009 - DNA, 20 bp, synthetic construct
  misc_feature 1..20: note = HBV-sgRNA-1006
  source 1..20: mol_type = other DNA
tgacgcaacccccactggtt

SEQ ID NO: 1010 - DNA, 20 bp, synthetic construct
  misc_feature 1..20: note = HBV-sgRNA-1007
  source 1..20: mol_type = other DNA
tgaggatgactgtctcttag

SEQ ID NO: 1011 - DNA, 20 bp, synthetic construct
  misc_feature 1..20: note = HBV-sgRNA-1008
  source 1..20: mol_type = other DNA
tgaggatgagtgtcccttag

SEQ ID NO: 1012 - DNA, 20 bp, synthetic construct
  misc_feature 1..20: note = HBV-sgRNA-1009
  source 1..20: mol_type = other DNA
tgaggatgagtgtttctcaa

SEQ ID NO: 1013 - DNA, 20 bp, synthetic construct
  misc_feature 1..20: note = HBV-sgRNA-1010
  source 1..20: mol_type = other DNA
tgagtaggccctgagcctga

SEQ ID NO: 1014 - DNA, 20 bp, synthetic construct
  misc_feature 1..20: note = HBV-sgRNA-1011
  source 1..20: mol_type = other DNA
tgagtgggaggagttggggg

SEQ ID NO: 1015 - DNA, 20 bp, synthetic construct
  misc_feature 1..20: note = HBV-sgRNA-1012
  source 1..20: mol_type = other DNA
tgatagatgtaagcaatttg

SEQ ID NO: 1016 - DNA, 20 bp, synthetic construct
  misc_feature 1..20: note = HBV-sgRNA-1013
  source 1..20: mol_type = other DNA
tgatcgggaaagaatcccag

SEQ ID NO: 1017 - DNA, 20 bp, synthetic construct
  misc_feature 1..20: note = HBV-sgRNA-1014
  source 1..20: mol_type = other DNA
tgatcggggaagaatcccag

SEQ ID NO: 1018 - DNA, 20 bp, synthetic construct
  misc_feature 1..20: note = HBV-sgRNA-1015
  source 1..20: mol_type = other DNA
tgcaattgattatgcctgct

SEQ ID NO: 1019 - DNA, 20 bp, synthetic construct
  misc_feature 1..20: note = HBV-sgRNA-1016
  source 1..20: mol_type = other DNA
tgcagggtccaactgatgat

SEQ ID NO: 1020 - DNA, 20 bp, synthetic construct
  misc_feature 1..20: note = HBV-sgRNA-1017
  source 1..20: mol_type = other DNA
tgcatgtatacaagcgaaac

SEQ ID NO: 1021 - DNA, 20 bp, synthetic construct
  misc_feature 1..20: note = HBV-sgRNA-1018
  source 1..20: mol_type = other DNA
tgcatgtatacaatctaagc

SEQ ID NO: 1022 - DNA, 20 bp, synthetic construct
  misc_feature 1..20: note = HBV-sgRNA-1019
  source 1..20: mol_type = other DNA
tgcatgtattcaatctaagc

SEQ ID NO: 1023 - DNA, 20 bp, synthetic construct
  misc_feature 1..20: note = HBV-sgRNA-1020
  source 1..20: mol_type = other DNA
tgccactcgggattaaagac

SEQ ID NO: 1024 - DNA, 20 bp, synthetic construct
  misc_feature 1..20: note = HBV-sgRNA-1021
  source 1..20: mol_type = other DNA
tgccatttaggattaaagca

SEQ ID NO: 1025 - DNA, 20 bp, synthetic construct
  misc_feature 1..20: note = HBV-sgRNA-1022
  source 1..20: mol_type = other DNA
tgcccaaggtcttacataag

SEQ ID NO: 1026 - DNA, 20 bp, synthetic construct
  misc_feature 1..20: note = HBV-sgRNA-1023
  source 1..20: mol_type = other DNA
tgcccaaggtcttgcataag

SEQ ID NO: 1027 - DNA, 20 bp, synthetic construct
  misc_feature 1..20: note = HBV-sgRNA-1024
  source 1..20: mol_type = other DNA
tgccgattggtggaggcagg

SEQ ID NO: 1028 - DNA, 20 bp, synthetic construct
  misc_feature 1..20: note = HBV-sgRNA-1025
  source 1..20: mol_type = other DNA
tgccgttccgaccgaccacg

SEQ ID NO: 1029 - DNA, 20 bp, synthetic construct
  misc_feature 1..20: note = HBV-sgRNA-1026
  source 1..20: mol_type = other DNA
tgccgttccggccgaccacg

SEQ ID NO: 1030 - DNA, 20 bp, synthetic construct
  misc_feature 1..20: note = HBV-sgRNA-1027
  source 1..20: mol_type = other DNA
tgcctgagtgcagtatggtg

SEQ ID NO: 1031 - DNA, 20 bp, synthetic construct
  misc_feature 1..20: note = HBV-sgRNA-1028
  source 1..20: mol_type = other DNA
tgcctgagtgccgtatggtg

SEQ ID NO: 1032 - DNA, 20 bp, synthetic construct
  misc_feature 1..20: note = HBV-sgRNA-1029
  source 1..20: mol_type = other DNA
tgcctgagtgctgtatggtg

SEQ ID NO: 1033 - DNA, 20 bp, synthetic construct
  misc_feature 1..20: note = HBV-sgRNA-1030
  source 1..20: mol_type = other DNA
tgcgagcaaaacaagcggct

SEQ ID NO: 1034 - DNA, 20 bp, synthetic construct
  misc_feature 1..20: note = HBV-sgRNA-1031
  source 1..20: mol_type = other DNA
tgcgagcgaaacaagctgct

SEQ ID NO: 1035 - DNA, 20 bp, synthetic construct
  misc_feature 1..20: note = HBV-sgRNA-1032
  source 1..20: mol_type = other DNA
tgcgggttgaggtcccaatc

SEQ ID NO: 1036 - DNA, 20 bp, synthetic construct
  misc_feature 1..20: note = HBV-sgRNA-1033
  source 1..20: mol_type = other DNA
tgctaggctgtgctgccaac

SEQ ID NO: 1037 - DNA, 20 bp, synthetic construct
  misc_feature 1..20: note = HBV-sgRNA-1034
  source 1..20: mol_type = other DNA
tgctagggtgtgctgccaac

SEQ ID NO: 1038 - DNA, 20 bp, synthetic construct
  misc_feature 1..20: note = HBV-sgRNA-1035
  source 1..20: mol_type = other DNA
tgctccagctcctaccttgt

SEQ ID NO: 1039 - DNA, 20 bp, synthetic construct
  misc_feature 1..20: note = HBV-sgRNA-1036
  source 1..20: mol_type = other DNA
tgctcccactcccaccttgt

SEQ ID NO: 1040 - DNA, 20 bp, synthetic construct
  misc_feature 1..20: note = HBV-sgRNA-1037
  source 1..20: mol_type = other DNA
tgctgtacaaaacctacgga

SEQ ID NO: 1041 - DNA, 20 bp, synthetic construct
  misc_feature 1..20: note = HBV-sgRNA-1038
  source 1..20: mol_type = other DNA
tgctgtacaaaaccttcgga

SEQ ID NO: 1042 - DNA, 20 bp, synthetic construct
  misc_feature 1..20: note = HBV-sgRNA-1039
  source 1..20: mol_type = other DNA
tgctgtaccaaaccttcgga

SEQ ID NO: 1043 - DNA, 20 bp, synthetic construct
  misc_feature 1..20: note = HBV-sgRNA-1040
  source 1..20: mol_type = other DNA
tggaaatgatgtatacttgc

SEQ ID NO: 1044 - DNA, 20 bp, synthetic construct
  misc_feature 1..20: note = HBV-sgRNA-1041
  source 1..20: mol_type = other DNA
tggacttctctcaattttct

SEQ ID NO: 1045 - DNA, 20 bp, synthetic construct
  misc_feature 1..20: note = HBV-sgRNA-1042
  source 1..20: mol_type = other DNA
tggatacgatgtatatttgc

SEQ ID NO: 1046 - DNA, 20 bp, synthetic construct
  misc_feature 1..20: note = HBV-sgRNA-1043
  source 1..20: mol_type = other DNA
tggcactagtaaactgagcc

SEQ ID NO: 1047 - DNA, 20 bp, synthetic construct
  misc_feature 1..20: note = HBV-sgRNA-1044
  source 1..20: mol_type = other DNA
tggccaagccccaaccagtg

SEQ ID NO: 1048 - DNA, 20 bp, synthetic construct
  misc_feature 1..20: note = HBV-sgRNA-1045
  source 1..20: mol_type = other DNA
tggccaagccccatccagtg

SEQ ID NO: 1049 - DNA, 20 bp, synthetic construct
  misc_feature 1..20: note = HBV-sgRNA-1046
  source 1..20: mol_type = other DNA
tggccagacgccaacaaggt

SEQ ID NO: 1050 - DNA, 20 bp, synthetic construct
  misc_feature 1..20: note = HBV-sgRNA-1047
  source 1..20: mol_type = other DNA
tggccagaggcaaatcaggt

SEQ ID NO: 1051 - DNA, 20 bp, synthetic construct
  misc_feature 1..20: note = HBV-sgRNA-1048
  source 1..20: mol_type = other DNA
tggccggacgccaacaaggt

SEQ ID NO: 1052 - DNA, 20 bp, synthetic construct
  misc_feature 1..20: note = HBV-sgRNA-1049
  source 1..20: mol_type = other DNA
tggcgattggtggaggcagg

SEQ ID NO: 1053 - DNA, 20 bp, synthetic construct
  misc_feature 1..20: note = HBV-sgRNA-1050
  source 1..20: mol_type = other DNA
tgggaacaagagctacagca

SEQ ID NO: 1054 - DNA, 20 bp, synthetic construct
  misc_feature 1..20: note = HBV-sgRNA-1051
  source 1..20: mol_type = other DNA
tgggaacaagatctacagca

SEQ ID NO: 1055 - DNA, 20 bp, synthetic construct
  misc_feature 1..20: note = HBV-sgRNA-1052
  source 1..20: mol_type = other DNA
tgggatatgtaattggaagt

SEQ ID NO: 1056 - DNA, 20 bp, synthetic construct
  misc_feature 1..20: note = HBV-sgRNA-1053
  source 1..20: mol_type = other DNA
tgggatatgtaattgggagt

SEQ ID NO: 1057 - DNA, 20 bp, synthetic construct
  misc_feature 1..20: note = HBV-sgRNA-1054
  source 1..20: mol_type = other DNA
tgggatctagcagagcttgg

SEQ ID NO: 1058 - DNA, 20 bp, synthetic construct
  misc_feature 1..20: note = HBV-sgRNA-1055
  source 1..20: mol_type = other DNA
tgggatcttgaagagtttgg

SEQ ID NO: 1059 - DNA, 20 bp, synthetic construct
  misc_feature 1..20: note = HBV-sgRNA-1056
  source 1..20: mol_type = other DNA
tggggaccctgcaccgaaca

SEQ ID NO: 1060 - DNA, 20 bp, synthetic construct
  misc_feature 1..20: note = HBV-sgRNA-1057
  source 1..20: mol_type = other DNA
tggggaccctgcgctgaaca

SEQ ID NO: 1061 - DNA, 20 bp, synthetic construct
  misc_feature 1..20: note = HBV-sgRNA-1058
  source 1..20: mol_type = other DNA
tggggaccctgtaccgaaca

SEQ ID NO: 1062 - DNA, 20 bp, synthetic construct
  misc_feature 1..20: note = HBV-sgRNA-1059
  source 1..20: mol_type = other DNA
tggtcccgtgctggtggttg

SEQ ID NO: 1063 - DNA, 20 bp, synthetic construct
  misc_feature 1..20: note = HBV-sgRNA-1060
  source 1..20: mol_type = other DNA
tggtcggccggtacaatagg

SEQ ID NO: 1064 - DNA, 20 bp, synthetic construct
  misc_feature 1..20: note = HBV-sgRNA-1061
  source 1..20: mol_type = other DNA
tggtcgggaaagaatcccag

SEQ ID NO: 1065 - DNA, 20 bp, synthetic construct
  misc_feature 1..20: note = HBV-sgRNA-1062
  source 1..20: mol_type = other DNA
tggtcggtcggaacggcaga

SEQ ID NO: 1066 - DNA, 20 bp, synthetic construct
  misc_feature 1..20: note = HBV-sgRNA-1063
  source 1..20: mol_type = other DNA
tggtcttccaaacctcgaaa

SEQ ID NO: 1067 - DNA, 20 bp, synthetic construct
  misc_feature 1..20: note = HBV-sgRNA-1064
  source 1..20: mol_type = other DNA
tggtcttccaaacctcgaca

SEQ ID NO: 1068 - DNA, 20 bp, synthetic construct
  misc_feature 1..20: note = HBV-sgRNA-1065
  source 1..20: mol_type = other DNA
tggtgaggtgaacaatgctc

SEQ ID NO: 1069 - DNA, 20 bp, synthetic construct
  misc_feature 1..20: note = HBV-sgRNA-1066
  source 1..20: mol_type = other DNA
tggtgaggtgaacaatgttc

SEQ ID NO: 1070 - DNA, 20 bp, synthetic construct
  misc_feature 1..20: note = HBV-sgRNA-1067
  source 1..20: mol_type = other DNA
tggtgagtgactggagattt

SEQ ID NO: 1071 - DNA, 20 bp, synthetic construct
  misc_feature 1..20: note = HBV-sgRNA-1068
  source 1..20: mol_type = other DNA
tggtgagtgattggaggttg

SEQ ID NO: 1072 - DNA, 20 bp, synthetic construct
  misc_feature 1..20: note = HBV-sgRNA-1069
  source 1..20: mol_type = other DNA
tgtagtatgccctgagcctg

SEQ ID NO: 1073 - DNA, 20 bp, synthetic construct
  misc_feature 1..20: note = HBV-sgRNA-1070
  source 1..20: mol_type = other DNA
tgtgcaggttttgcatggtc

SEQ ID NO: 1074 - DNA, 20 bp, synthetic construct
  misc_feature 1..20: note = HBV-sgRNA-1071
  source 1..20: mol_type = other DNA
tgtgtaaataatgtcgcgtc

SEQ ID NO: 1075 - DNA, 20 bp, synthetic construct
  misc_feature 1..20: note = HBV-sgRNA-1072
  source 1..20: mol_type = other DNA
tgtgtaaatagtgtctagtt

SEQ ID NO: 1076 - DNA, 20 bp, synthetic construct
  misc_feature 1..20: note = HBV-sgRNA-1073
  source 1..20: mol_type = other DNA
tgttctccatgttcagcgca

SEQ ID NO: 1077 - DNA, 20 bp, synthetic construct
  misc_feature 1..20: note = HBV-sgRNA-1074
  source 1..20: mol_type = other DNA
tgttctccatgttcggtaca

SEQ ID NO: 1078 - DNA, 20 bp, synthetic construct
  misc_feature 1..20: note = HBV-sgRNA-1075
  source 1..20: mol_type = other DNA
tgttctccatgttcggtgca

SEQ ID NO: 1079 - DNA, 20 bp, synthetic construct
  misc_feature 1..20: note = HBV-sgRNA-1076
  source 1..20: mol_type = other DNA
tgttgacataactgactact

SEQ ID NO: 1080 - DNA, 20 bp, synthetic construct
  misc_feature 1..20: note = HBV-sgRNA-1077
  source 1..20: mol_type = other DNA
tgttgtcctccaatttgtcc

SEQ ID NO: 1081 - DNA, 20 bp, synthetic construct
  misc_feature 1..20: note = HBV-sgRNA-1078
  source 1..20: mol_type = other DNA
tgtttcgctcgcagccggtc

SEQ ID NO: 1082 - DNA, 20 bp, synthetic construct
  misc_feature 1..20: note = HBV-sgRNA-1079
  source 1..20: mol_type = other DNA
tgttttgctcgcagcaggtc

SEQ ID NO: 1083 - DNA, 20 bp, synthetic construct
  misc_feature 1..20: note = HBV-sgRNA-1080
  source 1..20: mol_type = other DNA
ttaaagactgggaggagttg

SEQ ID NO: 1084 - DNA, 20 bp, synthetic construct
  misc_feature 1..20: note = HBV-sgRNA-1081
  source 1..20: mol_type = other DNA
ttaaaggtctttgtactagg

SEQ ID NO: 1085 - DNA, 20 bp, synthetic construct
  misc_feature 1..20: note = HBV-sgRNA-1082
  source 1..20: mol_type = other DNA
ttaatcattacttcaaaact

SEQ ID NO: 1086 - DNA, 20 bp, synthetic construct
  misc_feature 1..20: note = HBV-sgRNA-1083
  source 1..20: mol_type = other DNA
ttacacactctatggaaggc

SEQ ID NO: 1087 - DNA, 20 bp, synthetic construct
  misc_feature 1..20: note = HBV-sgRNA-1084
  source 1..20: mol_type = other DNA
ttacacactctttggaaggc

SEQ ID NO: 1088 - DNA, 20 bp, synthetic construct
  misc_feature 1..20: note = HBV-sgRNA-1085
  source 1..20: mol_type = other DNA
ttacatactctgtggaaggc

SEQ ID NO: 1089 - DNA, 20 bp, synthetic construct
  misc_feature 1..20: note = HBV-sgRNA-1086
  source 1..20: mol_type = other DNA
ttacatatcccatgaagtta

SEQ ID NO: 1090 - DNA, 20 bp, synthetic construct
  misc_feature 1..20: note = HBV-sgRNA-1087
  source 1..20: mol_type = other DNA
ttactgagtgggaggagttg

SEQ ID NO: 1091 - DNA, 20 bp, synthetic construct
  misc_feature 1..20: note = HBV-sgRNA-1088
  source 1..20: mol_type = other DNA
ttagaaaacttcctattaac

SEQ ID NO: 1092 - DNA, 20 bp, synthetic construct
  misc_feature 1..20: note = HBV-sgRNA-1089
  source 1..20: mol_type = other DNA
ttaggaaacttcctgtaaac

SEQ ID NO: 1093 - DNA, 20 bp, synthetic construct
  misc_feature 1..20: note = HBV-sgRNA-1090
  source 1..20: mol_type = other DNA
ttatatggatgatgtggtat

SEQ ID NO: 1094 - DNA, 20 bp, synthetic construct
  misc_feature 1..20: note = HBV-sgRNA-1091
  source 1..20: mol_type = other DNA
ttatatggatgatgtggttt

SEQ ID NO: 1095 - DNA, 20 bp, synthetic construct
  misc_feature 1..20: note = HBV-sgRNA-1092
  source 1..20: mol_type = other DNA
ttatttacacactctttgga

SEQ ID NO: 1096 - DNA, 20 bp, synthetic construct
  misc_feature 1..20: note = HBV-sgRNA-1093
  source 1..20: mol_type = other DNA
ttatttacatactctgtgga

SEQ ID NO: 1097 - DNA, 20 bp, synthetic construct
  misc_feature 1..20: note = HBV-sgRNA-1094
  source 1..20: mol_type = other DNA
ttccaaacctcgaaaaggca

SEQ ID NO: 1098 - DNA, 20 bp, synthetic construct
  misc_feature 1..20: note = HBV-sgRNA-1095
  source 1..20: mol_type = other DNA
ttccaaacctcgacaaggca

SEQ ID NO: 1099 - DNA, 20 bp, synthetic construct
  misc_feature 1..20: note = HBV-sgRNA-1096
  source 1..20: mol_type = other DNA
ttccaaattaacacccaccc

SEQ ID NO: 1100 - DNA, 20 bp, synthetic construct
  misc_feature 1..20: note = HBV-sgRNA-1097
  source 1..20: mol_type = other DNA
ttccaaattacttcccaccc

SEQ ID NO: 1101 - DNA, 20 bp, synthetic construct
  misc_feature 1..20: note = HBV-sgRNA-1098
  source 1..20: mol_type = other DNA
ttccaatgaggattaaagac

SEQ ID NO: 1102 - DNA, 20 bp, synthetic construct
  misc_feature 1..20: note = HBV-sgRNA-1099
  source 1..20: mol_type = other DNA
ttcccaccttatgagtccaa

SEQ ID NO: 1103 - DNA, 20 bp, synthetic construct
  misc_feature 1..20: note = HBV-sgRNA-1100
  source 1..20: mol_type = other DNA
ttccccaccttatgagtcca

SEQ ID NO: 1104 - DNA, 20 bp, synthetic construct
  misc_feature 1..20: note = HBV-sgRNA-1101
  source 1..20: mol_type = other DNA
ttcccgatacagagctgagg

SEQ ID NO: 1105 - DNA, 20 bp, synthetic construct
  misc_feature 1..20: note = HBV-sgRNA-1102
  source 1..20: mol_type = other DNA
ttccgaaagcccaggatgat

SEQ ID NO: 1106 - DNA, 20 bp, synthetic construct
  misc_feature 1..20: note = HBV-sgRNA-1103
  source 1..20: mol_type = other DNA
ttccttggactcataaggtg

SEQ ID NO: 1107 - DNA, 20 bp, synthetic construct
  misc_feature 1..20: note = HBV-sgRNA-1104
  source 1..20: mol_type = other DNA
ttcgtccccatgccttgtcg

SEQ ID NO: 1108 - DNA, 20 bp, synthetic construct
  misc_feature 1..20: note = HBV-sgRNA-1105
  source 1..20: mol_type = other DNA
ttctcaaaggtggagacagc

SEQ ID NO: 1109 - DNA, 20 bp, synthetic construct
  misc_feature 1..20: note = HBV-sgRNA-1106
  source 1..20: mol_type = other DNA
ttctctcccaaaagtaagac

SEQ ID NO: 1110 - DNA, 20 bp, synthetic construct
  misc_feature 1..20: note = HBV-sgRNA-1107
  source 1..20: mol_type = other DNA
ttctcttccaaaagtaagac

SEQ ID NO: 1111 - DNA, 20 bp, synthetic construct
  misc_feature 1..20: note = HBV-sgRNA-1108
  source 1..20: mol_type = other DNA
ttgaagagtttggtggaaag

SEQ ID NO: 1112 - DNA, 20 bp, synthetic construct
  misc_feature 1..20: note = HBV-sgRNA-1109
  source 1..20: mol_type = other DNA
ttgagttggctccgaacgca

SEQ ID NO: 1113 - DNA, 20 bp, synthetic construct
  misc_feature 1..20: note = HBV-sgRNA-1110
  source 1..20: mol_type = other DNA
ttgcgaaagcccaagatgat

SEQ ID NO: 1114 - DNA, 20 bp, synthetic construct
  misc_feature 1..20: note = HBV-sgRNA-1111
  source 1..20: mol_type = other DNA
ttgcgaaagcccaggatgat

SEQ ID NO: 1115 - DNA, 20 bp, synthetic construct
  misc_feature 1..20: note = HBV-sgRNA-1112
  source 1..20: mol_type = other DNA
ttgcgggtcaccatattctt

SEQ ID NO: 1116 - DNA, 20 bp, synthetic construct
  misc_feature 1..20: note = HBV-sgRNA-1113
  source 1..20: mol_type = other DNA
ttgcttgcctgagtgcagta

SEQ ID NO: 1117 - DNA, 20 bp, synthetic construct
  misc_feature 1..20: note = HBV-sgRNA-1114
  source 1..20: mol_type = other DNA
ttgggacctcaacccgcaca

SEQ ID NO: 1118 - DNA, 20 bp, synthetic construct
  misc_feature 1..20: note = HBV-sgRNA-1115
  source 1..20: mol_type = other DNA
ttgggacttcaaccccaaca

SEQ ID NO: 1119 - DNA, 20 bp, synthetic construct
  misc_feature 1..20: note = HBV-sgRNA-1116
  source 1..20: mol_type = other DNA
ttgggacttcaatcccaaca

SEQ ID NO: 1120 - DNA, 20 bp, synthetic construct
  misc_feature 1..20: note = HBV-sgRNA-1117
  source 1..20: mol_type = other DNA
ttgggattgaagtcccaatc

SEQ ID NO: 1121 - DNA, 20 bp, synthetic construct
  misc_feature 1..20: note = HBV-sgRNA-1118
  source 1..20: mol_type = other DNA
ttggggtgagttgatgaatc

SEQ ID NO: 1122 - DNA, 20 bp, synthetic construct
  misc_feature 1..20: note = HBV-sgRNA-1119
  source 1..20: mol_type = other DNA
ttggggttgaagtcccaatc

SEQ ID NO: 1123 - DNA, 20 bp, synthetic construct
  misc_feature 1..20: note = HBV-sgRNA-1120
  source 1..20: mol_type = other DNA
ttggtgagtgactggagatt

SEQ ID NO: 1124 - DNA, 20 bp, synthetic construct
  misc_feature 1..20: note = HBV-sgRNA-1121
  source 1..20: mol_type = other DNA
ttggtgagtgattggaggtt

SEQ ID NO: 1125 - DNA, 20 bp, synthetic construct
  misc_feature 1..20: note = HBV-sgRNA-1122
  source 1..20: mol_type = other DNA
ttggttcttctggactacca

SEQ ID NO: 1126 - DNA, 20 bp, synthetic construct
  misc_feature 1..20: note = HBV-sgRNA-1123
  source 1..20: mol_type = other DNA
ttggttcttctggactatca

SEQ ID NO: 1127 - DNA, 20 bp, synthetic construct
  misc_feature 1..20: note = HBV-sgRNA-1124
  source 1..20: mol_type = other DNA
ttgtgggtcaccatattctt

SEQ ID NO: 1128 - DNA, 20 bp, synthetic construct
  misc_feature 1..20: note = HBV-sgRNA-1125
  source 1..20: mol_type = other DNA
ttgttgctgtacaaaacctt

SEQ ID NO: 1129 - DNA, 20 bp, synthetic construct
  misc_feature 1..20: note = HBV-sgRNA-1126
  source 1..20: mol_type = other DNA
tttaaagactgggaggagtt

SEQ ID NO: 1130 - DNA, 20 bp, synthetic construct
  misc_feature 1..20: note = HBV-sgRNA-1127
  source 1..20: mol_type = other DNA
tttacacactctatggaagg

SEQ ID NO: 1131 - DNA, 20 bp, synthetic construct
  misc_feature 1..20: note = HBV-sgRNA-1128
  source 1..20: mol_type = other DNA
tttacacactctttggaagg

SEQ ID NO: 1132 - DNA, 20 bp, synthetic construct
  misc_feature 1..20: note = HBV-sgRNA-1129
  source 1..20: mol_type = other DNA
tttaccccgttgcccggcaa

SEQ ID NO: 1133 - DNA, 20 bp, synthetic construct
  misc_feature 1..20: note = HBV-sgRNA-1130
  source 1..20: mol_type = other DNA
tttaccccgttgctcggcaa

SEQ ID NO: 1134 - DNA, 20 bp, synthetic construct
  misc_feature 1..20: note = HBV-sgRNA-1131
  source 1..20: mol_type = other DNA
tttactgagtgggaggagtt

SEQ ID NO: 1135 - DNA, 20 bp, synthetic construct
  misc_feature 1..20: note = HBV-sgRNA-1132
  source 1..20: mol_type = other DNA
tttagtacaatatgttcctg

SEQ ID NO: 1136 - DNA, 20 bp, synthetic construct
  misc_feature 1..20: note = HBV-sgRNA-1133
  source 1..20: mol_type = other DNA
tttcagttatatggatgatg

SEQ ID NO: 1137 - DNA, 20 bp, synthetic construct
  misc_feature 1..20: note = HBV-sgRNA-1134
  source 1..20: mol_type = other DNA
tttcccaccttatgagtcca

SEQ ID NO: 1138 - DNA, 20 bp, synthetic construct
  misc_feature 1..20: note = HBV-sgRNA-1135
  source 1..20: mol_type = other DNA
tttcccaccttatgtgtcca

SEQ ID NO: 1139 - DNA, 20 bp, synthetic construct
  misc_feature 1..20: note = HBV-sgRNA-1136
  source 1..20: mol_type = other DNA
tttccgaaagcccaggatga

SEQ ID NO: 1140 - DNA, 20 bp, synthetic construct
  misc_feature 1..20: note = HBV-sgRNA-1137
  source 1..20: mol_type = other DNA
tttctcaaaggtggagacag

SEQ ID NO: 1141 - DNA, 20 bp, synthetic construct
  misc_feature 1..20: note = HBV-sgRNA-1138
  source 1..20: mol_type = other DNA
tttgaagtatgcctcaaggt

SEQ ID NO: 1142 - DNA, 20 bp, synthetic construct
  misc_feature 1..20: note = HBV-sgRNA-1139
  source 1..20: mol_type = other DNA
tttgagaaacactcatcctc

SEQ ID NO: 1143 - DNA, 20 bp, synthetic construct
  misc_feature 1..20: note = HBV-sgRNA-1140
  source 1..20: mol_type = other DNA
tttgagttggctccgaacgc

SEQ ID NO: 1144 - DNA, 20 bp, synthetic construct
  misc_feature 1..20: note = HBV-sgRNA-1141
  source 1..20: mol_type = other DNA
tttgcgaaagcccaagatga

SEQ ID NO: 1145 - DNA, 20 bp, synthetic construct
  misc_feature 1..20: note = HBV-sgRNA-1142
  source 1..20: mol_type = other DNA
tttgcgggtcaccatattct

SEQ ID NO: 1146 - DNA, 20 bp, synthetic construct
  misc_feature 1..20: note = HBV-sgRNA-1143
  source 1..20: mol_type = other DNA
tttgctgacgcaacccccac

SEQ ID NO: 1147 - DNA, 20 bp, synthetic construct
  misc_feature 1..20: note = HBV-sgRNA-1144
  source 1..20: mol_type = other DNA
tttggaagacccagcatcca

SEQ ID NO: 1148 - DNA, 20 bp, synthetic construct
  misc_feature 1..20: note = HBV-sgRNA-1145
  source 1..20: mol_type = other DNA
tttggaagatccagcatcca

SEQ ID NO: 1149 - DNA, 20 bp, synthetic construct
  misc_feature 1..20: note = HBV-sgRNA-1146
  source 1..20: mol_type = other DNA
tttggtggtctataagctgg

SEQ ID NO: 1150 - DNA, 20 bp, synthetic construct
  misc_feature 1..20: note = HBV-sgRNA-1147
  source 1..20: mol_type = other DNA
tttggtggtctatatgcagg

SEQ ID NO: 1151 - DNA, 20 bp, synthetic construct
  misc_feature 1..20: note = HBV-sgRNA-1148
  source 1..20: mol_type = other DNA
tttggtggtctgtaagcggg

SEQ ID NO: 1152 - DNA, 20 bp, synthetic construct
  misc_feature 1..20: note = HBV-sgRNA-1149
  source 1..20: mol_type = other DNA
tttgtccccatgccttttcg

SEQ ID NO: 1153 - DNA, 20 bp, synthetic construct
  misc_feature 1..20: note = HBV-sgRNA-1150
  source 1..20: mol_type = other DNA
tttgtctaagggcaaatatt

SEQ ID NO: 1154 - DNA, 20 bp, synthetic construct
  misc_feature 1..20: note = HBV-sgRNA-1151
  source 1..20: mol_type = other DNA
tttgtgggtcaccatattct

SEQ ID NO: 1155 - DNA, 20 bp, synthetic construct
  misc_feature 1..20: note = HBV-sgRNA-1152
  source 1..20: mol_type = other DNA
ttttcctgacattcatttgc

SEQ ID NO: 1156 - DNA, 20 bp, synthetic construct
  misc_feature 1..20: note = HBV-sgRNA-1153
  source 1..20: mol_type = other DNA
ttttctcattaactgtaagt

SEQ ID NO: 1157 - DNA, 20 bp, synthetic construct
  misc_feature 1..20: note = HBV-sgRNA-1154
  source 1..20: mol_type = other DNA
ttttgctcgcagcaggtctg

SEQ ID NO: 1158 - DNA, 20 bp, synthetic construct
  misc_feature 1..20: note = HBV-sgRNA-1155
  source 1..20: mol_type = other DNA
ttttgtacaatatgttcctg

SEQ ID NO: 1159 - DNA, 20 bp, synthetic construct
  misc_feature 1..20: note = HBV-sgRNA-1156
  source 1..20: mol_type = other DNA
ttttgtatgatgtgttcttg

SEQ ID NO: 1160 - DNA, 20 bp, synthetic construct
  misc_feature 1..20: note = HBV-sgRNA-1157
  source 1..20: mol_type = other DNA
ttttttcattaactgtaaga

SEQ ID NO: 1161 - DNA, 20 bp, synthetic construct
  misc_feature 1..20: note = HBV-sgRNA-1158
  source 1..20: mol_type = other DNA
gagttccactgcatggcctg

SEQ ID NO: 1162 - DNA, 20 bp, synthetic construct
  misc_feature 1..20: note = HBV-sgRNA-1159
  source 1..20: mol_type = other DNA
agtggtggagttccactgca

SEQ ID NO: 1163 - DNA, 20 bp, synthetic construct
  misc_feature 1..20: note = HBV-sgRNA-1160
  source 1..20: mol_type = other DNA
tgttgtggagttccactgca

SEQ ID NO: 1164 - DNA, 20 bp, synthetic construct
  misc_feature 1..20: note = HBV-sgRNA-1161
  source 1..20: mol_type = other DNA
gaattccactgcatggcctg

SEQ ID NO: 1165 - DNA, 20 bp, synthetic construct
  misc_feature 1..20: note = HBV-sgRNA-1162
  source 1..20: mol_type = other DNA
ggttgtggaattccactgca

SEQ ID NO: 1166 - protein, 302 aa, synthetic construct
  REGION 1..302: note = DNMT3A
MNHDQEFDPPKVYPPVPAEKRKPIRVLSLFDGIATGLLVLKDLGIQVDRYIASEVCEDSITVGMVRHQGKIMYVGDVRSVTQKHIQEWGPFDLVIGGSPCNDLSIVNPARKGLYEGTGRLFFEFYRLLHDARPKEGDDRPFFWLFENVVAMGVSDKRDISRFLESNPVMIDAKEVSAAHRARYFWGNLPGMNRPLASTVNDKLELQECLEHGRIAKFSKVRTITTRSNSIKQGKDQHFPVFMNEKEDILWCTEMERVFGFPVHYTDVSNMSRLARQRLLGRSWSVPVIRHLFAPLKEYFACV

SEQ ID NO: 1167 - protein, 215 aa, synthetic construct
  REGION 1..215: note = DNMT3L
MGPMEIYKTVSAWKRQPVRVLSLFRNIDKVLKSLGFLESGSGSGGGTLKYVEDVTNVVRRDVEKWGPFDLVYGSTQPLGSSCDRCPGWYMFQFHRILQYALPRQESQRPFFWIFMDNLLLTEDDQETTTRFLQTEAVTLQDVRGRDYQNAMRVWSNIPGLKSKHAPLTPKEEEYLQAQVRSRSKLDAPKVDLLVKNCLLPLREYFKYFSQNSLPL

SEQ ID NO: 1168 - protein, 62 aa, synthetic construct
  REGION 1..62: note = Exemplary KRAB domain
RTLVTFKDVFVDFTREEWKLLDTAQQIVYRNVMLENYKNLVSLGYQLTKPDVILRLEKGEEP

SEQ ID NO: 1169 - protein, 2111 aa, synthetic construct
  REGION 1..2111: note = DNMT3A-DNMT3L(3A3L)-dCas9-KRAB
MNHDQEFDPPKVYPPVPAEKRKPIRVLSLFDGIATGLLVLKDLGIQVDRYIASEVCEDSITVGMVRHQGKIMYVGDVRSVTQKHIQEWGPFDLVIGGSPCNDLSIVNPARKGLYEGTGRLFFEFYRLLHDARPKEGDDRPFFWLFENVVAMGVSDKRDISRFLESNPVMIDAKEVSAAHRARYFWGNLPGMNRPLASTVNDKLELQECLEHGRIAKFSKVRTITTRSNSIKQGKDQHFPVFMNEKEDILWCTEMERVFGFPVHYTDVSNMSRLARQRLLGRSWSVPVIRHLFAPLKEYFACVSSGNSNANSRGPSFSSGLVPLSLRGSHMGPMEIYKTVSAWKRQPVRVLSLFRNIDKVLKSLGFLESGSGSGGGTLKYVEDVTNVVRRDVEKWGPFDLVYGSTQPLGSSCDRCPGWYMFQFHRILQYALPRQESQRPFFWIFMDNLLLTEDDQETTTRFLQTEAVTLQDVRGRDYQNAMRVWSNIPGLKSKHAPLTPKEEEYLQAQVRSRSKLDAPKVDLLVKNCLLPLREYFKYFSQNSLPLGGPSSGAPPPSGGSPAGSPTSTEEGTSESATPESGPGTSTEPSEGSAPGSPAGSPTSTEEGTSTEPSEGSAPGTSTEPSEPKKKRKVMDKKYSIGLAIGTNSVGWAVITDEYKVPSKKFKVLGNTDRHSIKKNLIGALLFDSGETAEATRLKRTARRRYTRRKNRICYLQEIFSNEMAKVDDSFFHRLEESFLVEEDKKHERHPIFGNIVDEVAYHEKYPTIYHLRKKLVDSTDKADLRLIYLALAHMIKFRGHFLIEGDLNPDNSDVDKLFIQLVQTYNQLFEENPINASGVDAKAILSARLSKSRRLENLIAQLPGEKKNGLFGNLIALSLGLTPNFKSNFDLAEDAKLQLSKDTYDDDLDNLLAQIGDQYADLFLAAKNLSDAILLSDILRVNTEITKAPLSASMIKRYDEHHQDLTLLKALVRQQLPEKYKEIFFDQSKNGYAGYIDGGASQEEFYKFIKPILEKMDGTEELLVKLNREDLLRKQRTFDNGSIPHQIHLGELHAILRRQEDFYPFLKDNREKIEKILTFRIPYYVGPLARGNSRFAWMTRKSEETITPWNFEEVVDKGASAQSFIERMTNFDKNLPNEKVLPKHSLLYEYFTVYNELTKVKYVTEGMRKPAFLSGEQKKAIVDLLFKTNRKVTVKQLKEDYFKKIECFDSVEISGVEDRFNASLGTYHDLLKIIKDKDFLDNEENEDILEDIVLTLTLFEDREMIEERLKTYAHLFDDKVMKQLKRRRYTGWGRLSRKLINGIRDKQSGKTILDFLKSDGFANRNFMQLIHDDSLTFKEDIQKAQVSGQGDSLHEHIANLAGSPAIKKGILQTVKVVDELVKVMGRHKPENIVIEMARENQTTQKGQKNSRERMKRIEEGIKELGSQILKEHPVENTQLQNEKLYLYYLQNGRDMYVDQELDINRLSDYDVDAIVPQSFLKDDSIDNKVLTRSDKNRGKSDNVPSEEVVKKMKNYWRQLLNAKLITQRKFDNLTKAERGGLSELDKAGFIKRQLVETRQITKHVAQILDSRMNTKYDENDKLIREVKVITLKSKLVSDFRKDFQFYKVREINNYHHAHDAYLNAVVGTALIKKYPKLESEFVYGDYKVYDVRKMIAKSEQEIGKATAKYFFYSNIMNFFKTEITLANGEIRKRPLIETNGETGEIVWDKGRDFATVRKVLSMPQVNIVKKTEVQTGGFSKESILPKRNSDKLIARKKDWDPKKYGGFDSPTVAYSVLVVAKVEKGKSKKLKSVKELLGITIMERSSFEKNPIDFLEAKGYKEVKKDLIIKLPKYSLFELENGRKRMLASAGELQKGNELALPSKYVNFLYLASHYEKLKGSPEDNEQKQLFVEQHKHYLDEIIEQISEFSKRVILADANLDKVLSAYNKHRDKPIREQAENIIHLFTLTNLGAPAAFKYFDTTIDRKRYTSTKEVLDATLIHQSITGLYETRIDLSQLGGDAYPYDVPDYASLGSGSPKKKRKVEDPKKKRKVDGSGSETPGTSESATPESRTLVTFKDVFVDFTREEWKLLDTAQQIVYRNVMLENYKNLVSLGYQLTKPDVILRLEKGEEP

SEQ ID NO: 1170 - protein, 1368 aa, synthetic construct
  REGION 1..1368: note = Streptococcus pyogenes dCas9 (D10A, H840A)
MDKKYSIGLAIGTNSVGWAVITDEYKVPSKKFKVLGNTDRHSIKKNLIGALLFDSGETAEATRLKRTARRRYTRRKNRICYLQEIFSNEMAKVDDSFFHRLEESFLVEEDKKHERHPIFGNIVDEVAYHEKYPTIYHLRKKLVDSTDKADLRLIYLALAHMIKFRGHFLIEGDLNPDNSDVDKLFIQLVQTYNQLFEENPINASGVDAKAILSARLSKSRRLENLIAQLPGEKKNGLFGNLIALSLGLTPNFKSNFDLAEDAKLQLSKDTYDDDLDNLLAQIGDQYADLFLAAKNLSDAILLSDILRVNTEITKAPLSASMIKRYDEHHQDLTLLKALVRQQLPEKYKEIFFDQSKNGYAGYIDGGASQEEFYKFIKPILEKMDGTEELLVKLNREDLLRKQRTFDNGSIPHQIHLGELHAILRRQEDFYPFLKDNREKIEKILTFRIPYYVGPLARGNSRFAWMTRKSEETITPWNFEEVVDKGASAQSFIERMTNFDKNLPNEKVLPKHSLLYEYFTVYNELTKVKYVTEGMRKPAFLSGEQKKAIVDLLFKTNRKVTVKQLKEDYFKKIECFDSVEISGVEDRFNASLGTYHDLLKIIKDKDFLDNEENEDILEDIVLTLTLFEDREMIEERLKTYAHLFDDKVMKQLKRRRYTGWGRLSRKLINGIRDKQSGKTILDFLKSDGFANRNFMQLIHDDSLTFKEDIQKAQVSGQGDSLHEHIANLAGSPAIKKGILQTVKVVDELVKVMGRHKPENIVIEMARENQTTQKGQKNSRERMKRIEEGIKELGSQILKEHPVENTQLQNEKLYLYYLQNGRDMYVDQELDINRLSDYDVDAIVPQSFLKDDSIDNKVLTRSDKNRGKSDNVPSEEVVKKMKNYWRQLLNAKLITQRKFDNLTKAERGGLSELDKAGFIKRQLVETRQITKHVAQILDSRMNTKYDENDKLIREVKVITLKSKLVSDFRKDFQFYKVREINNYHHAHDAYLNAVVGTALIKKYPKLESEFVYGDYKVYDVRKMIAKSEQEIGKATAKYFFYSNIMNFFKTEITLANGEIRKRPLIETNGETGEIVWDKGRDFATVRKVLSMPQVNIVKKTEVQTGGFSKESILPKRNSDKLIARKKDWDPKKYGGFDSPTVAYSVLVVAKVEKGKSKKLKSVKELLGITIMERSSFEKNPIDFLEAKGYKEVKKDLIIKLPKYSLFELENGRKRMLASAGELQKGNELALPSKYVNFLYLASHYEKLKGSPEDNEQKQLFVEQHKHYLDEIIEQISEFSKRVILADANLDKVLSAYNKHRDKPIREQAENIIHLFTLTNLGAPAAFKYFDTTIDRKRYTSTKEVLDATLIHQSITGLYETRIDLSQLGGD

SEQ ID NO: 1171 - protein, 1053 aa, synthetic construct
  REGION 1..1053: note = Staphylococcus aureus dCas9 (Mutant: D10A and H557A)
MKRNYILGLAIGITSVGYGIIDYETRDVIDAGVRLFKEANVENNEGRRSKRGARRLKRRRRHRIQRVKKLLFDYNLLTDHSELSGINPYEARVKGLSQKLSEEEFSAALLHLAKRRGVHNVNEVEEDTGNELSTKEQISRNSKALEEKYVAELQLERLKKDGEVRGSINRFKTSDYVKEAKQLLKVQKAYHQLDQSFIDTYIDLLETRRTYYEGPGEGSPFGWKDIKEWYEMLMGHCTYFPEELRSVKYAYNADLYNALNDLNNLVITRDENEKLEYYEKFQIIENVFKQKKKPTLKQIAKEILVNEEDIKGYRVTSTGKPEFTNLKVYHDIKDITARKEIIENAELLDQIAKILTIYQSSEDIQEELTNLNSELTQEEIEQISNLKGYTGTHNLSLKAINLILDELWHTNDNQIAIFNRLKLVPKKVDLSQQKEIPTTLVDDFILSPVVKRSFIQSIKVINAIIKKYGLPNDIIIELAREKNSKDAQKMINEMQKRNRQTNERIEEIIRTTGKENAKYLIEKIKLHDMQEGKCLYSLEAIPLEDLLNNPFNYEVDAIIPRSVSFDNSFNNKVLVKQEENSKKGNRTPFQYLSSSDSKISYETFKKHILNLAKGKGRISKTKKEYLLEERDINRFSVQKDFINRNLVDTRYATRGLMNLLRSYFRVNNLDVKVKSINGGFTSFLRRKWKFKKERNKGYKHHAEDALIIANADFIFKEWKKLDKAKKVMENQMFEEKQAESMPEIETEQEYKEIFITPHQIKHIKDFKDYKYSHRVDKKPNRELINDTLYSTRKDDKGNTLIVNNLNGLYDKDNDKLKKLINKSPEKLLMYHHDPQTYQKLKLIMEQYGDEKNPLYKYYEETGNYLTKYSKKDNGPVIKKIKYYGNKLNAHLDITDDYPNSRNKVVKLSLKPYRFDVYLDNGVYKFVTVKNLDVIKKENYYEVNSKCYEEAKKLKKISNQAEFIASFYNNDLIKINGELYRVIGVNNDLLNRIEVNMIDITYREYLENMNDKRPPRIIKTIASKTQSIKKYSTDILGNLYEVKSKKHPQIIKKG

SEQ ID NO: 1172 - protein, 1053 aa, synthetic construct
  REGION 1..1053: note = Staphylococcus aureus dCas9 (Mutant: D10A and N580A)
MKRNYILGLAIGITSVGYGIIDYETRDVIDAGVRLFKEANVENNEGRRSKRGARRLKRRRRHRIQRVKKLLFDYNLLTDHSELSGINPYEARVKGLSQKLSEEEFSAALLHLAKRRGVHNVNEVEEDTGNELSTKEQISRNSKALEEKYVAELQLERLKKDGEVRGSINRFKTSDYVKEAKQLLKVQKAYHQLDQSFIDTYIDLLETRRTYYEGPGEGSPFGWKDIKEWYEMLMGHCTYFPEELRSVKYAYNADLYNALNDLNNLVITRDENEKLEYYEKFQIIENVFKQKKKPTLKQIAKEILVNEEDIKGYRVTSTGKPEFTNLKVYHDIKDITARKEIIENAELLDQIAKILTIYQSSEDIQEELTNLNSELTQEEIEQISNLKGYTGTHNLSLKAINLILDELWHTNDNQIAIFNRLKLVPKKVDLSQQKEIPTTLVDDFILSPVVKRSFIQSIKVINAIIKKYGLPNDIIIELAREKNSKDAQKMINEMQKRNRQTNERIEEIIRTTGKENAKYLIEKIKLHDMQEGKCLYSLEAIPLEDLLNNPFNYEVHHIIPRSVSFDNSFNNKVLVKQEEASKKGNRTPFQYLSSSDSKISYETFKKHILNLAKGKGRISKTKKEYLLEERDINRFSVQKDFINRNLVDTRYATRGLMNLLRSYFRVNNLDVKVKSINGGFTSFLRRKWKFKKERNKGYKHHAEDALIIANADFIFKEWKKLDKAKKVMENQMFEEKQAESMPEIETEQEYKEIFITPHQIKHIKDFKDYKYSHRVDKKPNRELINDTLYSTRKDDKGNTLIVNNLNGLYDKDNDKLKKLINKSPEKLLMYHHDPQTYQKLKLIMEQYGDEKNPLYKYYEETGNYLTKYSKKDNGPVIKKIKYYGNKLNAHLDITDDYPNSRNKVVKLSLKPYRFDVYLDNGVYKFVTVKNLDVIKKENYYEVNSKCYEEAKKLKKISNQAEFIASFYNNDLIKINGELYRVIGVNNDLLNRIEVNMIDITYREYLENMNDKRPPRIIKTIASKTQSIKKYSTDILGNLYEVKSKKHPQIIKKG

SEQ ID NO: 1173 - protein, 1053 aa, synthetic construct
  REGION 1..1053: note = Staphylococcus aureus dCas9 (Mutant: D10A and N580A)
MKRNYILGLAIGITSVGYGIIDYETRDVIDAGVRLFKEANVENNEGRRSKRGARRLKRRRRHRIQRVKKLLFDYNLLTDHSELSGINPYEARVKGLSQKLSEEEFSAALLHLAKRRGVHNVNEVEEDTGNELSTKEQISRNSKALEEKYVAELQLERLKKDGEVRGSINRFKTSDYVKEAKQLLKVQKAYHQLDQSFIDTYIDLLETRRTYYEGPGEGSPFGWKDIKEWYEMLMGHCTYFPEELRSVKYAYNADLYNALNDLNNLVITRDENEKLEYYEKFQIIENVFKQKKKPTLKQIAKEILVNEEDIKGYRVTSTGKPEFTNLKVYHDIKDITARKEIIENAELLDQIAKILTIYQSSEDIQEELTNLNSELTQEEIEQISNLKGYTGTHNLSLKAINLILDELWHTNDNQIAIFNRLKLVPKKVDLSQQKEIPTTLVDDFILSPVVKRSFIQSIKVINAIIKKYGLPNDIIIELAREKNSKDAQKMINEMQKRNRQTNERIEEIIRTTGKENAKYLIEKIKLHDMQEGKCLYSLEAIPLEDLLNNPFNYEVHAIIPRSVSFDNSFNNKVLVKQEEASKKGNRTPFQYLSSSDSKISYETFKKHILNLAKGKGRISKTKKEYLLEERDINRFSVQKDFINRNLVDTRYATRGLMNLLRSYFRVNNLDVKVKSINGGFTSFLRRKWKFKKERNKGYKHHAEDALIIANADFIFKEWKKLDKAKKVMENQMFEEKQAESMPEIETEQEYKEIFITPHQIKHIKDFKDYKYSHRVDKKPNRELINDTLYSTRKDDKGNTLIVNNLNGLYDKDNDKLKKLINKSPEKLLMYHHDPQTYQKLKLIMEQYGDEKNPLYKYYEETGNYLTKYSKKDNGPVIKKIKYYGNKLNAHLDITDDYPNSRNKVVKLSLKPYRFDVYLDNGVYKFVTVKNLDVIKKENYYEVNSKCYEEAKKLKKISNQAEFIASFYNNDLIKINGELYRVIGVNNDLLNRIEVNMIDITYREYLENMNDKRPPRIIKTIASKTQSIKKYSTDILGNLYEVKSKKHPQIIKKG

SEQ ID NO: 1174 - protein, 984 aa, synthetic construct
  REGION 1..984: note = Campylobacter jejuni dCas9(D8A, H559A)
MARILAFAIGISSIGWAFSENDELKDCGVRIFTKVENPKTGESLALPRRLARSARKRLARRKARLNHLKHLIANEFKLNYEDYQSFDESLAKAYKGSLISPYELRFRALNELLSKQDFARVILHIAKRRGYDDIKNSDDKEKGAILKAIKQNEEKLANYQSVGEYLYKEYFQKFKENSKEFTNVRNKKESYERCIAQSFLKDELKLIFKKQREFGFSFSKKFEEEVLSVAFYKRALKDFSHLVGNCSFFTDEKRAPKNSPLAFMFVALTRIINLLNNLKNTEGILYTKDDLNALLNEVLKNGTLTYKQTKKLLGLSDDYEFKGEKGTYFIEFKKYKEFIKALGEHNLSQDDLNEIAKDITLIKDEIKLKKALAKYDLNQNQIDSLSKLEFKDHLNISFKALKLVTPLMLEGKKYDEACNELNLKVAINEDKKDFLPAFNETYYKDEVTNPVVLRAIKEYRKVLNALLKKYGKVHKINIELAREVGKNHSQRAKIEKEQNENYKAKKDAELECEKLGLKINSKNILKLRLFKEQKEFCAYSGEKIKISDLQDEKMLEIDAIYPYSRSFDDSYMNKVLVFTKQNQEKLNQTPFEAFGNDSAKWQKIEVLAKNLPTKKQKRILDKNYKDKEQKNFKDRNLNDTRYIARLVLNYTKDYLDFLPLSDDENTKLNDTQKGSKVHVEAKSGMLTSALRHTWGFSAKDRNNHLHHAIDAVIIAYANNSIVKAFSDFKKEQESNSAELYAKKISELDYKNKRKFFEPFSGFRQKVLDKIDEIFVSKPERKKPSGALHEETFRKEEEFYQSYGGKEGVLKALELGKIRKVNGKIVKNGDMFRVDIFKHKKTNKFYAVPIYTMDFALKVLPNKAVARSKKGEIKDWILMDENYEFCFSLYKDSLILIQTKDMQEPEFVYYNAFTSSTVSLIVSKHDNKFETLSKNQKILFKNANEKEVIAKSIGIQNLKVFEKYIVSALGEVTKAEFRQREDFKK

SEQ ID NO: 1175 - protein, 1084 aa, synthetic construct
  REGION 1..1084: note = Corynebacterium diphtheria dCas9(D8A, H573A)
MKYHVGIAVGTFSVGLAAIEVDDAGMPIKTLSLVSHIHDSGLDPDEIKSAVTRLASSGIARRTRRLYRRKRRRLQQLDKFIQRQGWPVIELEDYSDPLYPWKVRAELAASYIADEKERGEKLSVALRHIARHRGWRNPYAKVSSLYLPDGPSDAFKAIREEIKRASGQPVPETATVGQMVTLCELGTLKLRGEGGVLSARLQQSDYAREIQEICRMQEIGQELYRKIIDVVFAAESPKGSASSRVGKDPLQPGKNRALKASDAFQRYRIAALIGNLRVRVDGEKRILSVEEKNLVFDHLVNLTPKKEPEWVTIAEILGIDRGQLIGTATMTDDGERAGARPPTHDTNRSIVNSRIAPLVDWWKTASALEQHAMVKALSNAEVDDFDSPEGAKVQAFFADLDDDVHAKLDSLHLPVGRAAYSEDTLVRLTRRMLSDGVDLYTARLQEFGIEPSWTPPTPRIGEPVGNPAVDRVLKTVSRWLESATKTWGAPERVIIEHVREGFVTEKRAREMDGDMRRRAARNAKLFQEMQEKLNVQGKPSRADLWRYQSVQRQNCQCAYCGSPITFSNSEMDAIVPRAGQGSTNTRENLVAVCHRCNQSKGNTPFAIWAKNTSIEGVSVKEAVERTRHWVTDTGMRSTDFKKFTKAVVERFQRATMDEEIDARSMESVAWMANELRSRVAQHFASHGTTVRVYRGSLTAEARRASGISGKLKFFDGVGKSRLDRRHHAIDAAVIAFTSDYVAETLAVRSNLKQSQAHRQEAPQWREFTGKDAEHRAAWRVWCQKMEKLSALLTEDLRDDRVVVMSNVRLRLGNGSAHKETIGKLSKVKLSSQLSVSDIDKASSEALWCALTREPGFDPKEGLPANPERHIRVNGTHVYAGDNIGLFPVSAGSIALRGGYAELGSSFHHARVYKITSGKKPAFAMLRVYTIDLLPYRNQDLFSVELKPQTMSMRQAEKKLRDALATGNAEYLGWLVVDDELVVDTSKIATDQVKAVEAELGTIRRWRVDGFFSPSKLRLRPLQMSKEGIKKESAPELSKIIDRPGWLPAVNKLFSDGNVTVVRRDSLGRVRLESTAHLPVTWKVQ

SEQ ID NO: 1176 - protein, 1107 aa, synthetic construct
  REGION 1..1107: note = Eubacterium ventriosum dCas9(D8A, H592A)
MGYTVGLAIGVASVGVAVLDENDNIVEAVSNIFDEADTSNNKVRRTLREGRRTKRRQKTRIEDFKQLWETSGYIIPHKLHLNIIELRNKGLTELLSLDELYCVLLSMLKHRGISYLEDADDGEKGNAYKKGLAFNEKQLKEKMPCEIQLERMKKYGKYHGEFIIEINDEKEYQSNVFTTKAYKKELEKIFETQRCNGNKINTKFIKKYMEIYERKREYYIGPGNEKSRTDYGIYTTRTDEEGNFIDEKNIFGKLIGKCSVYPEEYRASSASYTAQEFNLLNDLNNLKINNEKLTEFQKKEIVEIIKDASSVNMRKIIKKVIDEDIEQYSGARIDKKGKEIYHTFEIYRKLKKELKTINVDIDSFTREELDKTMDILTLNTERESIVKAFDEQKFVYEENLIKKLIEFRKNNQRLFSGWHSFSYKAMLQLIPVMYKEPKEQMQLLTEMNVFKSKKEKYVNYKYIPENEVVKEIYNPVVVKSIRTTVKILNALIKKYGYPESVVIEMPRDKNSDDEKEKIDMNQKKNQEEYEKILNKIYDEKGIEITNKDYKKQKKLVLKLKLWNEQEGLCLYSGKKIAIEDLLNHPEFFEIDAIIPKSISLDDSRSNKVLVYKTENSIKENDTPYHYLTRINGKWGFDEYKANVLELRRRGKIDDKKVNNLLCMEDITKIDVVKGFINRNLNDTRYASRVVLNEMQSFFESRKYCNTKVKVIRGSLTYQMRQDLHLKKNREESYSHHAVDAMLIAFSQKGYEAYRKIQKDCYDFETGEILDKEKWNKYIDDDEFDDILYKERMNEIRKKIIEAEEKVKYNYKIDKKCNRGLCNQTIYGTREKDGKIHKISSYNIYDDKECNSLKKMINSGKGSDLLMYNNDPKTYRDMLKILETYSSEKNPFVAYNKETGDYFRKYSKNHNGPKVEKVKYYSGQINSCIDISHKYGHAKNSKKVVLVSLNPYRTDVYYDNDTGKYYLVGVKYNHIKCVGNKYVIDSETYNELLRKEGVLNSDENLEDLNSKNITYKFSLYKNDIIQYEKGGEYYTERFLSRIKEQKNLIETKPINKPNFQRKNKKGEWENTRNQIALAKTKYVGKLVTDVLGNCYIVNMEKFSLVVDK

SEQ ID NO: 1177 - protein, 1130 aa, synthetic construct
  REGION 1..1130: note = Streptococcus pasteurianus dCas9(D10A, H599A)
MTNGKILGLAIGIASVGVGIIEAKTGKVVHANSRLFSAANAENNAERRGFRGSRRLNRRKKHRVKRVRDLFEKYGIVTDFRNLNLNPYELRVKGLTEQLKNEELFAALRTISKRRGISYLDDAEDDSTGSTDYAKSIDENRRLLKNKTPGQIQLERLEKYGQLRGNFTVYDENGEAHRLINVFSTSDYEKEARKILETQADYNKKITAEFIDDYVEILTQKRKYYHGPGNEKSRTDYGRFRTDGTTLENIFGILIGKCNFYPDEYRASKASYTAQEYNFLNDLNNLKVSTETGKLSTEQKESLVEFAKNTATLGPAKLLKEIAKILDCKVDEIKGYREDDKGKPDLHTFEPYRKLKFNLESINIDDLSREVIDKLADILTLNTEREGIEDAIKRNLPNQFTEEQISEIIKVRKSQSTAFNKGWHSFSAKLMNELIPELYATSDEQMTILTRLEKFKVNKKSSKNTKTIDEKEVTDEIYNPVVAKSVRQTIKIINAAVKKYGDFDKIVIEMPRDKNADDEKKFIDKRNKENKKEKDDALKRAAYLYNSSDKLPDEVFHGAKQLETKIRLWYQQGERCLYSGKPISIQELVHNSNNFEIDHILPLSLSFDDSLANKVLVYAWTNQEKGQKTPYQVIDSMDAAWSFREMKDYVLKQKGLGKKKRDYLLTTENIDKIEVKKKFIERNLVDTRYASRVVLNSLQSALRELGKDTKVSVVRGQFTSQLRRKWKIDKSRETYHHHAVDALIIAASSQLKLWEKQDNPMFVDYGKNQVVDKQTGEILSVSDDEYKELVFQPPYQGFVNTISSKGFEDEILFSYQVDSKYNRKVSDATIYSTRKAKIGKDKKEETYVLGKIKDIYSQNGFDTFIKKYNKDKTQFLMYQKDSLTWENVIEVILRDYPTTKKSEDGKNDVKCNPFEEYRRENGLICKYSKKGKGTPIKSLKYYDKKLGNCIDITPEESRNKVILQSINPWRADVYFNPETLKYELMGLKYSDLSFEKGTGNYHISQEKYDAIKEKEGIGKKSEFKFTLYRNDLILIKDIASGEQEIYRFLSRTMPNVNHYVELKPYDKEKFDNVQELVEALGEADKVGRCIKGLNKPNISIYKVRTDVLGNKYFVKKKGDKPKLDFKNNKK

SEQ ID NO: 1178 - protein, 1125 aa, synthetic construct
  REGION 1..1125: note = Lactobacillus farciminis dCas9(D10A, H611A)
MTDRISLGLAIGVASVGFSVLDIDKGKVIELGARLFNATVAAGNQDRRDMRGSRRLLNRNKQRRKDVSKLFQEYGLLDNFDRDNFHTAFNNNWNPYELRVKGLTKQLNKEELADSLYQIIKRRGISYALKDADANEDGTDYSSSLKINSQELIEKTPAQIQLQRLNDYGKVRGKVIVGDDIDDQKVLLNVFPTNAYEKEARQIIATQQQFYPEILTGEFVKEYCQILTRKRDYFVGPGNEKSRTDYGIYKTDGRTLDNLFEELIGHDKIYPDELRASAASYTAQLFNVLNDLNNLRILSYEDGKLTQIDKEKIIAEIKNNTTVVNMLNVIKKVTGCQKDDIKGFRLNEKDKPEISSMPIYRKAHKDFLKVGIDITDWPIDFIDRLSFILTLNTENGEIRKQINKRLVPDFDFLNDDLVQLIIDNKDSFDIKTNNKWHRFSLKTMNKLIPTMIERPVEQMTLLTEMGLIKKDTKRFEGNKYLPYKEIANDIFNPVASKSVREALKIVNAVLKKYGHIEYIVIEMPRDKNLDEERKQIADFQKKNKKIKDAAFNAFVKAVGSKKNVKIALSKNRKLQMGIRLWHQQQGIDPYNGEEINANDLISNPDKFEIDAIIPQSISFDDGINNKTLCFASMNQVKGQKTPYEFLNEGHGQGYAKFKAIVSKNKNFSKAKRDNYLFEENVSNIETRKRFLSRNLVDTRYSSRVVLNSLQEFFHEKSDDTKVTVIRGKFTSNMRKHWHIDKTRDTFHHHAIDASIIAATPFLRMWKKGSTIFPTKINETSIDIETGEILDDKNFDKVMYEEPYSGFISEIMNADDRIKFSHQVDKKMNRKVSDATIYSTRIGKLSKDKKDAEYVVAKVKDIYSVDGYENFKKVYKKDKTKFLLYKYDPRTFSELEKIVIDYPDKIEKVQTNGKIKAVDISPFELYRRDNGMVRKYSKKTGPAIKQLKYLDKKLGSHIDITPKNANNKHVVLQSLKPWRTDVYLNHETGEYEIMGIKYSDLKFNKNEGYGIKKDKYLKIKNIEGVSENSEFMFSLYRKDRIKVQDMETNESVELLFWSRNFSNKKYAELKPISQIDNDKVLPIYGRGRLIKRLIPKNCKIWKVNTSILGDTYYLEKESNYPQKILD

SEQ ID NO: 1179 - protein, 1179 aa, synthetic construct
  REGION 1..1179: note = Sphaerochaeta globosa dCas9(D30A, H635A)
MSKKVSRRYEEQAQEICQRLGSRPYSIGLALGVGSIGVAVAAYDPIKKQPSDLVFVSSRIFIPSTGAAERRQKRGQRNSLRHRANRLKFLWKLLAERNLMLSYSEQDVPDPARLRFEDAVVRANPYELRLKGLNEQLTLSELGYALYHIANHRGSSSVRTFLDEEKSSDDKKLEEQQAMTEQLAKEKGISTFIEVLTAFNTNGLIGYRNSESVKSKGVPVPTRDIISNEIDVLLQTQKQFYQEILSDEYCDRIVSAILFENEKIVPEAGCCPYFPDEKKLPRCHFLNEERRLWEAINNARIKMPMQEGAAKRYQSASFSDEQRHILFHIARSGTDITPKLVQKEFPALKTSIIVLQGKEKAIQKIAGFRFRRLEEKSFWKRLSEEQKDDFFSAWTNTPDDKRLSKYLMKHLLLTENEVVDALKTVSLIGDYGPIGKTATQLLMKHLEDGLTYTEALERGMETGEFQELSVWEQQSLLPYYGQILTGSTQALMGKYWHSAFKEKRDSEGFFKPNTNSDEEKYGRIANPVVHQTLNELRKLMNELITILGAKPQEITVELARELKVGAEKREDIIKQQTKQEKEAVLAYSKYCEPNNLDKRYIERFRLLEDQAFVCPYCLEHISVADIAAGRADVDAIFPRDDTADNSYGNKVVAHRQCNDIKGKRTPYAAFSNTSAWGPIMHYLDETPGMWRKRRKFETNEEEYAKYLQSKGFVSRFESDNSYIAKAAKEYLRCLFNPNNVTAVGSLKGMETSILRKAWNLQGIDDLLGSRHWSKDADTSPTMRKNRDDNRHHGLDAIVALYCSRSLVQMINTMSEQGKRAVEIEAMIPIPGYASEPNLSFEAQRELFRKKILEFMDLHAFVSMKTDNDANGALLKDTVYSILGADTQGEDLVFVVKKKIKDIGVKIGDYEEVASAIRGRITDKQPKWYPMEMKDKIEQLQSKNEAALQKYKESLVQAAAVLEESNRKLIESGKKPIQLSEKTISKKALELVGGYYYLISNNKRTKTFVVKEPSNEVKGFAFDTGSNLCLDFYHDAQGKLCGEIIRKIQAMNPSYKPAYMKQGYSLYVRLYQGDVCELRASDLTEAESNLAKTTHVRLPNAKPGRTFVIIITFTEMGSGYQIYFSNLAKSKKGQDTSFTLTTIKNYDVRKVQLSSAGLVRYVSPLLVDKIEKDEVALCGE

SEQ ID NO: 1180 - protein, 1168 aa, synthetic construct
  REGION 1..1168: note = Azospirillum (strain B510) dCas9(D75A, H680A)
MARPAFRAPRREHVNGWTPDPHRISKPFFILVSWHLLSRVVIDSSSGCFPGTSRDHTDKFAEWECAVQPYRLSFALGTNSIGWGLLNLDRQGKPREIRALGSRIFSDGRDPQDKASLAVARRLARQMRRRRDRYLTRRTRLMGALVRFGLMPADPAARKRLEVAVDPYLARERATRERLEPFEIGRALFHLNQRRGYKPVRTATKPDEEAGKVKEAVERLEAAIAAAGAPTLGAWFAWRKTRGETLRARLAGKGKEAAYPFYPARRMLEAEFDTLWAEQARHHPDLLTAEAREILRHRIFHQRPLKPPPVGRCTLYPDDGRAPRALPSAQRLRLFQELASLRVIHLDLSERPLTPAERDRIVAFVQGRPPKAGRKPGKVQKSVPFEKLRGLLELPPGTGFSLESDKRPELLGDETGARIAPAFGPGWTALPLEEQDALVELLLTEAEPERAIAALTARWALDEATAAKLAGATLPDFHGRYGRRAVAELLPVLERETRGDPDGRVRPIRLDEAVKLLRGGKDHSDFSREGALLDALPYYGAVLERHVAFGTGNPADPEEKRVGRVANPTVHIALNQLRHLVNAILARHGRPEEIVIELARDLKRSAEDRRREDKRQADNQKRNEERKRLILSLGERPTPRNLLKLRLWEEQGPVENRRCPYSGETISMRMLLSEQVDIDAILPFSVSLDDSAANKVVCLREANRIKRNRSPWEAFGHDSERWAGILARAEALPKNKRWRFAPDALEKLEGEGGLRARHLNDTRHLSRLAVEYLRCVCPKVRVSPGRLTALLRRRWGIDAILAEADGPPPEVPAETLDPSPAEKNRADHRHHALDAVVIGCIDRSMVQRVQLAAASAEREAAAREDNIRRVLEGFKEEPWDGFRAELERRARTIVVSHRPEHGIGGALHKETAYGPVDPPEEGFNLVVRKPIDGLSKDEINSVRDPRLRRALIDRLAIRRRDANDPATALAKAAEDLAAQPASRGIRRVRVLKKESNPIRVEHGGNPSGPRSGGPFHKLLLAGEVHHVDVALRADGRRWVGHWVTLFEAHGGRGADGAAAPPRLGDGERFLMRLHKGDCLKLEHKGRVRVMQVVKLEPSSNSVVVVEPHQVKTDRSKHVKISCDQLRARGARRVTVDPLGRVRVHAPGARVGIGGDAGRTAMEPAEDIS

SEQ ID NO: 1181 - protein, 1003 aa, synthetic construct
  REGION 1..1003: note = Gluconacetobacter diazotrophicus dCas9(D11A, H587A)
MIDESLTFGIALGIGSCGWAVLRRPSAFGRKGVIEGMGSWCFDVPETSKERTPTNQIRRSNRLLRRVIRRRRNRMAAIRRLLHAAGLLPSTDSDALKRPGHDPWELRARGLDKPLKPVEFAVVLGHIAKRRGFKSAAKRKATNISSDDKKMLTALEATRERLGRYRTVGEMFARDPDFASRRRNREGKYDRTTARDDLEHEVHALFAAQRRLGQGFASPELEEAFTASAFHQRPMQDSERLVGFCPFERTEKRAAKLTPSFERFRLLARLLNLRITTPDGERPLTVDEIALVTRDLGKTAKLSIKRVRTLIGLEDNQRFTTIRPEDEDRDIVARTGGAMTGTATLRKALGEALWTDMQERPEQLDAIVQVLSFFEANETITEKLREIGLTLAVLDVLLTALDAGVFAKFKGAAHISTKAARNLLPHLEQGRRYDEACTMAGYDHAASRLSHHGQIVAKTQFNALVTEIGESIANPIARKALIEGLKQIWAMRNHWGLPGSIHVELARDVGNSIEKRREIEKHIEKNTALRARERREVHDLLDLEDVNGDTLLRYRLWKEQGGKCLYTGKAIHIRQIAATDNSVQVDAILPWSRFGDDSFNNKTLCLASANQQKKRSTPYEWLSGQTGDAWNAFVQRIETNKELRGFKKRNYLLKNAKEAEEKFRSRNLNDTRYAARLFAEAVKLLYAFGERQEKGGNRRVFTRPGALTAALRQAWGVESLKKQDGKRINDDRHHALDALTVAAVDEAEIQRLTKSFHEWEQQGLGRPLRRVEPPWESFRADVEATYPEVFVARPERRRARGEGHAATIRQVKERECTPIVFERKAVSSLKEADLERIKDGERNEAIVEAIRSWIATGRPADAPPRSPRGDIITKIRLATTIKAAVPVRGGTAGRGEMVRADVFSKPNRRGKDEWYLVPVYPHQIMNRKAWPKPPMRSIVANKDEDEWTEVGPEHQFRFSLYPRSNIEIIRPSGEVIEGYFVGLHRNTGALIPTPVGPDSYVIA

SEQ ID NO: 1182 - protein, 1082 aa, synthetic construct
  REGION 1..1082: note = Neisseria cinerea dCas9(D16A, H588A)
MAAFKPNPMNYILGLAIGIASVGWAIVEIDEEENPIRLIDLGVRVFERAEVPKTGDSLAAARRLARSVRRLTRRRAHRLLRARRLLKREGVLQAADFDENGLIKSLPNTPWQLRAAALDRKLTPLEWSAVLLHLIKHRGYLSQRKNEGETADKELGALLKGVADNTHALQTGDFRTPAELALNKFEKESGHIRNQRGDYSHTFNRKDLQAELNLLFEKQKEFGNPHVSDGLKEGIETLLMTQRPALSGDAVQKMLGHCTFEPTEPKAAKNTYTAERFVWLTKLNNLRILEQGSERPLTDTERATLMDEPYRKSKLTYAQARKLLDLDDTAFFKGLRYGKDNAEASTLMEMKAYHAISRALEKEGLKDKKSPLNLSPELQDEIGTAFSLFKTDEDITGRLKDRVQPEILEALLKHISFDKFVQISLKALRRIVPLMEQGNRYDEACTEIYGDHYGKKNTEEKIYLPPIPADEIRNPVVLRALSQARKVINGVVRRYGSPARIHIETAREVGKSFKDRKEIEKRQEENRKDREKSAAKFREYFPNFVGEPKSKDILKLRLYEQQHGKCLYSGKEINLGRLNEKGYVEIDAALPFSRTWDDSFNNKVLALGSENQNKGNQTPYEYFNGKDNSREWQEFKARVETSRFPRSKKQRILLQKFDEDGFKERNLNDTRYINRFLCQFVADHMLLTGKGKRRVFASNGQITNLLRGFWGLRKVRAENDRHHALDAVVVACSTIAMQQKITRFVRYKEMNAFDGKTIDKETGEVLHQKAHFPQPWEFFAQEVMIRVFGKPDGKPEFEEADTPEKLRTLLAEKLSSRPEAVHKYVTPLFISRAPNRKMSGQGHMETVKSAKRLDEGISVLRVPLTQLKLKDLEKMVNREREPKLYEALKARLEAHKDDPAKAFAEPFYKYDKAGNRTQQVKAVRVEQVQKTGVWVHNHNGIADNATIVRVDVFEKGGKYYLVPIYSWQVAKGILPDRAVVQGKDEEDWTVMDDSFEFKFVLYANDLIKLTAKKNEFLGYFVSLNRATGAIDIRTHDTDSTKGKNGIFQSVGVKTALSFQKYQIDELGKEIRPCRLKKRPPVR

SEQ ID NO: 1183 - protein, 1140 aa, synthetic construct
  REGION 1..1140: note = Roseburia intestinalis dCas9(D24A, H628A)
MRENGSDERRRNMDEKMDYRIGLAIGIASVGWAVLQNNSDDEPVRIVDLGVRIFDTAEIPKTGESLAGPRRAARTTRRRLRRRKHRLDRIKWLFENQGLINIDDFLKRYNMAGLPDVYQLRYEALDRKLTDEELAQVLLHIAKHRGFRSTRKAETAAKENGAVLKATDENQKRMQEKGYRTVGEMIYLDEAFRTGCSWSEKGYILTPRNKAENYQHTMLRAMLVEEVKEIFSSQRRLGNEKATEELEEKYLEIMTSQRSFDLGPGMQPDGKPSPYAMEGFSDRVGKCTFLGDQGELRGAKGTYTAEYFVALQKINHTKLVNQDGETRNFTEEERRALTLLLFTQKEVKYAAVRKKLGLPEDILFYNLNYKKAATKEEQQKENQNTEKAKFIGMPYYHDYKKCLEERVKYLTENEVRDLFDEIGMILTCYKNDDSRTERLAKLGLVPIEMEGLLAYTPTKFQHLSMKAMRNIIPFLEKGMTYDKACEEAGYDFKADSKGTKQKLLTGENVNQTINEITNPVVKRSVSQTVKVINAIIRTYGSPQAINIELAREMSKTFEERRKIKGDMEKRQKNNEDVKKQIQELGKLSPTGQDILKYRLWQEQQGICMYSGKTIPLEELFKPGYDIDAILPYSITFDDSFRNKVLVTSQENRQKGNRTPYEYMGNDEQRWNEFETRVKTTIRDYKKQQKLLKKHFSEEERSEFKERNLTDTKYITTVIYNMIRQNLEMAPLNRPEKKKQVRAVNGAITAYLRKRWGLPQKNRETDTHHAMDAVVIACCTDGMIQKISRYTKVRERCYSKGTEFVDAETGEIFRPEDYSRAEWDEIFGVHIPKPWETFRAELDVRMGDDPKGFLDTHSDVALELDYPEYIYENLRPIFVSRMPNHKVTGAAHADTIRSPRHFKDEGIVLTKTALTDLKLDKDGEIDGYYNPQSDLLLYEALKKQLLLYGNDAKKAFAQDFHKPKADGTEGPVVRKVKIQKKQTMGVFVDSGNGIAENGGMVRIDVFRVNGKYYFVPVYTADVVKKVLPNRASTAHKPYGEWKVMEDKDFLFSLYSRDLIHIKSKKDIPIKMVNGGMEGIKETYAYYIGADISAANIQGIAHDSRYKFRGLGIQSLDVLEKCQIDVLGHVSVVRSEKRMGFS

SEQ ID NO: 1184 - protein, 1037 aa, synthetic construct
  REGION 1..1037: note = Parvibaculum lavamentivorans dCas9(D8A, H601A)
MERIFGFAIGTTSIGFSVIDYSSTQSAGNIQRLGVRIFPEARDPDGTPLNQQRRQKRMMRRQLRRRRIRRKALNETLHEAGFLPAYGSADWPVVMADEPYELRRRGLEEGLSAYEFGRAIYHLAQHRHFKGRELEESDTPDPDVDDEKEAANERAATLKALKNEQTTLGAWLARRPPSDRKRGIHAHRNVVAEEFERLWEVQSKFHPALKSEEMRARISDTIFAQRPVFWRKNTLGECRFMPGEPLCPKGSWLSQQRRMLEKLNNLAIAGGNARPLDAEERDAILSKLQQQASMSWPGVRSALKALYKQRGEPGAEKSLKFNLELGGESKLLGNALEAKLADMFGPDWPAHPRKQEIRHAVHERLWAADYGETPDKKRVIILSEKDRKAHREAAANSFVADFGITGEQAAQLQALKLPTGWEPYSIPALNLFLAELEKGERFGALVNGPDWEGWRRTNFPHRNQPTGEILDKLPSPASKEERERISQLRNPTVVRTQNELRKVVNNLIGLYGKPDRIRIEVGRDVGKSKREREEIQSGIRRNEKQRKKATEDLIKNGIANPSRDDVEKWILWKEGQERCPYTGDQIGFNALFREGRYEVEAIWPRSRSFDNSPRNKTLCRKDVNIEKGNRMPFEAFGHDEDRWSAIQIRLQGMVSAKGGTGMSPGKVKRFLAKTMPEDFAARQLNDTRYAAKQILAQLKRLWPDMGPEAPVKVEAVTGQVTAQLRKLWTLNNILADDGEKTRADHRHHAIDALTVACTHPGMTNKLSRYWQLRDDPRAEKPALTPPWDTIRADAEKAVSEIVVSHRVRKKVSGPLHKETTYGDTGTDIKTKSGTYRQFVTRKKIESLSKGELDEIRDPRIKEIVAAHVAGRGGDPKKAFPPYPCVSPGGPEIRKVRLTSKQQLNLMAQTGNGYADLGSNHHIAIYRLPDGKADFEIVSLFDASRRLAQRNPIVQRTRADGASFVMSLAAGEAIMIPEGSKKGIWIVQGVWASGQVVLERDTDADHSTTTRPMPNPILKDDAKKVSIDPIGRVRPSND

SEQ ID NO: 1185 - protein, 1132 aa, synthetic construct
  REGION 1..1132: note = Nitratifractor salsuginis (strain DSM 16511) dCas9(D8A, H611A)
MKKILGVALGITSFGYAILQETGKDLYRCLDNSVVMRNNPYDEKSGESSQSIRSTQKSMRRLIEKRKKRIRCVAQTMERYGILDYSETMKINDPKNNPIKNRWQLRAVDAWKRPLSPQELFAIFAHMAKHRGYKSIATEDLIYELELELGLNDPEKESEKKADERRQVYNALRHLEELRKKYGGETIAQTIHRAVEAGDLRSYRNHDDYEKMIRREDIEEEIEKVLLRQAELGALGLPEEQVSELIDELKACITDQEMPTIDESLFGKCTFYKDELAAPAYSYLYDLYRLYKKLADLNIDGYEVTQEDREKVIEWVEKKIAQGKNLKKITHKDLRKILGLAPEQKIFGVEDERIVKGKKEPRTFVPFFFLADIAKFKELFASIQKHPDALQIFRELAEILQRSKTPQEALDRLRALMAGKGIDTDDRELLELFKNKRSGTRELSHRYILEALPLFLEGYDEKEVQRILGFDDREDYSRYPKSLRHLHLREGNLFEKEENPINNHAVKSLASWALGLIADLSWRYGPFDEIILETTRDALPEKIRKEIDKAMREREKALDKIIGKYKKEFPSIDKRLARKIQLWERQKGLDLYSGKVINLSQLLDGSADIEAIVPQSLGGLSTDYNTIVTLKSVNAAKGNRLPGDWLAGNPDYRERIGMLSEKGLIDWKKRKNLLAQSLDEIYTENTHSKGIRATSYLEALVAQVLKRYYPFPDPELRKNGIGVRMIPGKVTSKTRSLLGIKSKSRETNFHHAEDALILSTLTRGWQNRLHRMLRDNYGKSEAELKELWKKYMPHIEGLTLADYIDEAFRRFMSKGEESLFYRDMFDTIRSISYWVDKKPLSASSHKETVYSSRHEVPTLRKNILEAFDSLNVIKDRHKLTTEEFMKRYDKEIRQKLWLHRIGNTNDESYRAVEERATQIAQILTRYQLMDAQNDKEIDEKFQQALKELITSPIEVTGKLLRKMRFVYDKLNAMQIDRGLVETDKNMLGIHISKGPNEKLIFRRMDVNNAHELQKERSGILCYLNEMLFIFNKKGLIHYGCLRSYLEKGQGSKYIALFNPRFPANPKAQPSKFTSDSKIKQVGIGSATGIIKAHLDLDGHVRSYEVFGTLPEGSIEWFKEESGYGRVEDDPHH

SEQ ID NO: 1186 - protein, 997 aa, synthetic construct
  REGION 1..997: note = Campylobacter lari dCas9(D7A, H567A)
MKILGFAIGINSIGWAFVENDELKDCGVRIFTEAENPSNKESLALPRRNARSSRRRLKRRKARLVAIKRILAKELKLNFKDYVAADGELPKAYEGKLTSIYELRYKALIQQLETKDLARVILHIAKHRGYMNKNEKKSNDTKKGKILSALKNNALKLENYQSVGEYFYKEFFQKYKENTKNFIKIRNTKDNYNNCVLSSDLEKELKLILEKQKEFGYNYSEDFINEILKVAFFQRPLKDFSHLVGACTFFEEEKRACKNSYSAWEFVALTKIINEIKSLEKISGEIVPTQTINEILNLILDKGSITYKKFRSCINLHESISFKSLKYDKENAENAKLIDFRKLVEFKKALGVHSLSRQELDQISTHITLIKDNVKLKTVLEKYNLSNEQINNLLEIEFNDYINLSFKALGMILPLMREGKRYYEACEITNLKPKTVDEKEDFLPAFCDSIFAHELSNPVVNRAISEYRKVLNALLKKYGKVHKIHLELARDVGLSKKAREKIEDQQKNNKAINDWALKECENIGIKASAKNILKLKLWKEQKEICIYSGNKISIEHLKDEKALEVDAIYPYSRSFDDSFINKVLVFTKENQEKLNKTPFEAFGKNIEKWSKIQTLAQNLPYKKKNKILDENFKDKQQQDFISRNLNDTRYITTLIAKYTKEYLNFLPLSENENTNLKSGEKGSKIHIQTISGMLTSVLRHTWGFDKKDRNNHLHHALDAIIVAYSTSSIIKAFSDFKKNQELLKARFYAKELTSDNYKHQVKFFEPFKGFREKILSKIDEIFVSTPPRKRARGALHEETFYSEDKMIKKYNSKEGLQIALSCGRVRKIGTKYVENDTMVRVDIFKKQNKFYAIPIYVMDFALGILPNKIVITGKDKNNNPKQWQTIDESYEFCFSLYKNDLILLQKKNMQEPEFAYYNSFDIDRSRIKIKKHDNKFENLTSNQKLLFTNKDKGKNRTGIQNLKIFEKYIVTPLGDKIKADFQPRENISLKTSKKHGL

SEQ ID NO: 1187 - protein, 1388 aa, synthetic construct
  REGION 1..1388: note = Streptococcus thermophilus (strain LMD-9) dCas9(D10A, H847A)
MTKPYSIGLAIGTNSVGWAVTTDNYKVPSKKMKVLGNTSKKYIKKNLLGVLLFDSGITAEGRRLKRTARRRYTRRRNRILYLQEIFSTEMATLDDAFFQRLDDSFLVPDDKRDSKYPIFGNLVEEKAYHDEFPTIYHLRKYLADSTKKADLRLVYLALAHMIKYRGHFLIEGEFNSKNNDIQKNFQDFLDTYNAIFESDLSLENSKQLEEIVKDKISKLEKKDRILKLFPGEKNSGIFSEFLKLIVGNQADFRKCFNLDEKASLHFSKESYDEDLETLLGYIGDDYSDVFLKAKKLYDAILLSGFLTVTDNETEAPLSSAMIKRYNEHKEDLALLKEYIRNISLKTYNEVFKDDTKNGYAGYIDGKTNQEDFYVYLKKLLAEFEGADYFLEKIDREDFLRKQRTFDNGSIPYQIHLQEMRAILDKQAKFYPFLAKNKERIEKILTFRIPYYVGPLARGNSDFAWSIRKRNEKITPWNFEDVIDKESSAEAFINRMTSFDLYLPEEKVLPKHSLLYETFNVYNELTKVRFIAESMRDYQFLDSKQKKDIVRLYFKDKRKVTDKDIIEYLHAIYGYDGIELKGIEKQFNSSLSTYHDLLNIINDKEFLDDSSNEAIIEEIIHTLTIFEDREMIKQRLSKFENIFDKSVLKKLSRRHYTGWGKLSAKLINGIRDEKSGNTILDYLIDDGISNRNFMQLIHDDALSFKKKIQKAQIIGDEDKGNIKEVVKSLPGSPAIKKGILQSIKIVDELVKVMGGRKPESIVVEMARENQYTNQGKSNSQQRLKRLEKSLKELGSKILKENIPAKLSKIDNNALQNDRLYLYYLQNGKDMYTGDDLDIDRLSNYDIDAIIPQAFLKDNSIDNKVLVSSASNRGKSDDVPSLEVVKKRKTFWYQLLKSKLISQRKFDNLTKAERGGLSPEDKAGFIQRQLVETRQITKHVARLLDEKFNNKKDENNRAVRTVKIITLKSTLVSQFRKDFELYKVREINDFHHAHDAYLNAVVASALLKKYPKLEPEFVYGDYPKYNSFRERKSATEKVYFYSNIMNIFKKSISLADGRVIERPLIEVNEETGESVWNKESDLATVRRVLSYPQVNVVKKVEEQNHGLDRGKPKGLFNANLSSKPKPNSNENLVGAKEYLDPKKYGGYAGISNSFTVLVKGTIEKGAKKKITNVLEFQGISILDRINYRKDKLNFLLEKGYKDIELIIELPKYSLFELSDGSRRMLASILSTNNKRGEIHKGNQIFLSQKFVKLLYHAKRISNTINENHRKYVENHKKEFEELFYYILEFNENYVGAKKNGKLLNSAFQSWQNHSIDELCSSFIGPTGSERKGLFELTSRGSAADFEFLGVKIPRYRDYTPSSLLKDATLIHQSVTGLYETRIDLAKLGEG

SEQ ID NO: 1188 - DNA, 63 bp, synthetic construct
  misc_feature 1..63: note = P2A
  source 1..63: mol_type = other DNA
gctactaacttcagcctgctgaagcaggctggcgacgtggaggagaaccctggacctgccacc

SEQ ID NO: 1189 - DNA, 710 bp, synthetic construct
  misc_feature 1..710: note = EGFP
  source 1..710: mol_type = other DNA
atggtgagcaagggcgaggagctgttcaccggggtggtgcccatcctggtcgagctggacggcgacgtaaacggccacaagttcagcgtgtccggcgagggcgagggcgatgccacctacggcaagctgaccctgaagttcatctgcaccaccggcaagctgcccgtgccctggcccaccctcgtgaccaccctgacctacggcgtgcagtgcttcagccgctaccccgaccacatgaagcagcacgacttcttcaagtccgccatgcccgaaggctacgtccaggagcgcaccatcttcttcaaggacgacggcaactacaagacccgcgccgaggtgaagttcgagggcgacaccctggtgaaccgcatcgagctgaagggcatcgacttcaaggaggacggcaacatcctggggcacaagctggagtacaactacaacagccacaacgtctatatcatggccgacaagcagaagaacggcatcaaggtgaacttcaagatccgccacaacatcgaggacggcagcgtgcagctcgccgaccactaccagcagaacacccccatcggcgacggccccgtgctgctgcccgacaaccactacctgagcacccagtccgccctgagcaaagaccccaacgagaagcgcgatcacatggtcctgctggagttcgtgaccgccgccgggatcactctcggcatggacgagct

SEQ ID NO: 1190 - RNA, 100 nt, synthetic construct
  misc_feature 1..100: note = scaffold sequence
  misc_feature 1: note = n =
  misc_feature 2: note = n =
  misc_feature 3: note = n =
  misc_feature 4: note = n =
  misc_feature 5: note = n =
  misc_feature 6: note = n =
  misc_feature 7: note = n =
  misc_feature 8: note = n =
  misc_feature 9: note = n =
  misc_feature 10: note = n =
  misc_feature 11: note = n =
  misc_feature 12: note = n =
  misc_feature 13: note = n =
  misc_feature 14: note = n =
  misc_feature 15: note = n =
  misc_feature 16: note = n =
  misc_feature 17: note = n =
  misc_feature 18: note = n =
  misc_feature 19: note = n =
  misc_feature 20: note = n =
  source 1..100: mol_type = other RNA
nnnnnnnnnnnnnnnnnnnngttttagagctagaaatagcaagttaaaataaggctagtccgttatcaacttgaaaaagtggcaccgagtcggtgctttt

SEQ ID NO: 1191 - RNA, 6967 nt, synthetic construct
  misc_feature 1..6967: note = EPIREG mRNA
  source 1..6967: mol_type = other RNA
aggactcactatttgttttcgcgcccagttgcaaaaagtgtcgacatttgcttctgacacaactgtgttcactagcaacctcaaacagacaccgccaccatggtgcctgccgccaagagagtgaagctggacggcagcaaccacgaccaagagttcgaccctcctaaggtgtaccctcctgtgccagccgagaagcggaagcctatcagagtgctgagcctgttcgacggaatcgccacaggactgctggtgctgaaggatctgggaatccaggtggaccggtatatcgccagcgaagtgtgcgaggacagcatcacagttggcatggttcgacaccagggcaagattatgtacgtgggcgacgtgcggagcgtgacccagaaacacattcaagagtggggccccttcgacctggttatcggcggcagcccttgcaacgatctgagcatcgtgaaccccgccagaaagggcctgtatgaaggcaccggcagactgttcttcgagttctacagactgctgcacgacgccagacctaaagagggcgacgacagaccattcttctggctgttcgagaacgtggtggctatgggcgtgtccgacaagcgggacatcagccggtttctggaaagcaaccccgtgatgatcgacgccaaagaggtgtccgctgctcaccgggccagatacttttggggcaatctgcccggcatgaacagacctctggccagcaccgtgaacgacaagctggaactgcaagagtgcctggaacacggccggatcgccaagtttagcaaagtgcggaccatcaccaccaggtccaacagcatcaagcagggcaaagaccagcacttccccgtgttcatgaatgagaaagaggacatcctgtggtgcaccgagatggaaagagtgttcggcttccctgtgcactacaccgacgtgtccaacatgagcagactggccagacagaggctgctgggcagatcttggagcgtgccagtgatcagacacctgttcgcccctctgaaagaatacttcgcctgcgtgtccagcggcaacagcaacgccaatagcagaggccctagcttcagctctggactggtgcctttgagcctgagaggcagccacatgttcgagacagtgcctgtgtggcggagacagcccgttagagtgctgtccctgtttgaggacatcaagaaagagctgaccagcctgggcttcctggaaagcggatctgatcctggccagctgaagcacgtggtggacgtgaccgataccgtgcggaaggatgtggaagaatggggcccttttgatctggtgtacggcgccacacctcctctgggccacacatgtgatagacctccaagctggtatctgttccagttccaccggctgctgcagtacgctagacccaagcctggaagccccaggcctttcttttggatgttcgtggacaacctggtcctgaacaaagaggacctggacgtcgccagccggttcctcgaaatggaacctgtgacaatccccgacgtgcacggcggatctctgcagaatgctgtcagagtgtggtctaacatccccgccatcagaagcagcagacactgggcccttgtgtccgaggaagaactgtctctgctggcccagaacaagcagagcagcaagctggccgccaagtggcctacaaagctggtcaagaactgcttcctgcctctgcgcgagtacttcaagtatttcagcggcggacctagctctggcgcccctccacctagcggaggatctccagcaggatctcctaccagcaccgaggaaggcacaagcgagtctgccacacctgagtctggccctggcacatctacagagcctagcgagggatctgcccctggatctcctgctggcagccctacatctaccgaagagggaaccagcacagagccttccgaaggttctgctcctggcacaagcaccgagccaagcgagatgaacaacagccagggcagagtgaccttcgaggatgtgaccgtgaacttcacccaaggcgagtggcagagactgaaccccgagcagagaaacctgtaccgggacgtgatgctggaaaactacagcaacctggtgtccgtcggccagggcgagacaacaaagcctgacgtgatcctgcggctggaacagggaaaagagccttggctggaagaggaagaggtgctcggatctggacgggccgagaagaacggcgatattggcggacagatctggaagcctaaggacgtgaaagagagcctgagcggctctgaaacacctggaacaagcgaaggcggaccaggcacctctaccgaaccatctgagggaagcgctccaggttctcctgccggctctccaacaagcacagaagagggcacctccactgagccctctgaaggcagtgctcctggaacttccaccgaaccttccgagccaaagaagaaacgcaaggtgggctccgacaagaagtacagcatcggcctggccatcggcaccaactctgtgggctgggccgtgatcaccgacgagtacaaggtgcccagcaagaaattcaaggtgctgggcaacaccgaccggcacagcatcaagaagaacctgatcggcgccctgctgttcgacagcggagaaacagccgaggccacccggctgaagagaaccgccagaagaagatacaccagacggaagaaccggatctgctatctgcaagagatcttcagcaacgagatggccaaggtggacgacagcttcttccacagactggaagagtccttcctggtggaagaggataagaagcacgagcggcaccccatcttcggcaacatcgtggacgaggtggcctaccacgagaagtaccccaccatctaccacctgagaaagaaactggtggacagcaccgacaaggccgacctgcggctgatctatctggccctggcccacatgatcaagttccggggccacttcctgatcgagggcgacctgaaccccgacaacagcgacgtggacaagctgttcatccagctggtgcagacctacaaccagctgttcgaggaaaaccccatcaacgccagcggcgtggacgccaaggccatcctgtctgccagactgagcaagagcagacggctggaaaatctgatcgcccagctgcccggcgagaagaagaatggcctgttcggcaacctgattgccctgagcctgggcctgacccccaacttcaagagcaacttcgacctggccgaggatgccaaactgcagctgagcaaggacacctacgacgacgacctggacaacctgctggcccagatcggcgaccagtacgccgacctgtttctggccgccaagaacctgtccgacgccatcctgctgagcgacatcctgagagtgaacaccgagatcaccaaggcccccctgagcgcctctatgatcaagagatacgacgagcaccaccaggacctgaccctgctgaaagctctcgtgcggcagcagctgcctgagaagtacaaagagattttcttcgaccagagcaagaacggctacgccggctacatcgatggcggagccagccaggaagagttctacaagttcatcaagcccatcctggaaaagatggacggcaccgaggaactgctcgtgaagctgaacagagaggacctgctgcggaagcagcggaccttcgacaacggcagcatcccccaccagatccacctgggagagctgcacgccattctgcggcggcaggaagatttttacccattcctgaaggacaaccgggaaaagatcgagaagatcctgaccttccgcatcccctactacgtgggccctctggccaggggaaacagcagattcgcctggatgaccagaaagagcgaggaaaccatcaccccctggaacttcgaggaagtggtggacaagggcgccagcgcccagagcttcatcgagcggatgaccaacttcgataagaacctgcccaacgagaaggtgctgcccaagcacagcctgctgtacgagtacttcaccgtgtacaacgagctgaccaaagtgaaatacgtgaccgagggaatgagaaagcccgccttcctgagcggcgagcagaaaaaagccatcgtggacctgctgttcaagaccaaccggaaagtgaccgtgaagcagctgaaagaggactacttcaagaaaatcgagtgcttcgactccgtggaaatctccggcgtggaagatcggttcaacgcctccctgggcacataccacgatctgctgaaaattatcaaggacaaggacttcctggacaatgaggaaaacgaggacattctggaagatatcgtgctgaccctgacactgtttgaggacagagagatgatcgaggaacggctgaaaacctatgcccacctgttcgacgacaaagtgatgaagcagctgaagcggcggagatacaccggctggggcaggctgagccggaagctgatcaacggcatccgggacaagcagtccggcaagacaatcctggatttcctgaagtccgacggcttcgccaacagaaacttcatgcagctgatccacgacgacagcctgacctttaaagaggacatccagaaagcccaggtgtccggccagggcgatagcctgcacgagcacattgccaatctggccggcagccccgccattaagaagggcatcctgcagacagtgaaggtggtggacgagctcgtgaaagtgatgggccggcacaagcccgagaacatcgtgatcgaaatggccagagagaaccagaccacccagaagggacagaagaacagccgcgagagaatgaagcggatcgaagagggcatcaaagagctgggcagccagatcctgaaagaacaccccgtggaaaacacccagctgcagaacgagaagctgtacctgtactacctgcagaatgggcgggatatgtacgtggaccaggaactggacatcaaccggctgtccgactacgatgtggacgctatcgtgcctcagagctttctgaaggacgactccatcgataacaaagtgctgactcggagcgacaagaaccggggcaagagcgacaacgtgccctccgaagaggtcgtgaagaagatgaagaactactggcgccagctgctgaatgccaagctgattacccagaggaagttcgacaatctgaccaaggccgagagaggcggcctgagcgaactggataaggccggcttcatcaagagacagctggtggaaacccggcagatcacaaagcacgtggcacagatcctggactcccggatgaacactaagtacgacgagaacgacaaactgatccgggaagtgaaagtgatcaccctgaagtccaagctggtgtccgatttccggaaggatttccagttttacaaagtgcgcgagatcaacaactaccaccacgcccacgacgcctacctgaacgccgtcgtgggaaccgccctgatcaaaaagtaccctaagctggaaagcgagttcgtgtacggcgactacaaggtgtacgacgtgcggaagatgatcgccaagagcgagcaggaaatcggcaaggctaccgccaagtacttcttctacagcaacatcatgaactttttcaagaccgagattaccctggccaacggcgagatccggaagcggcctctgatcgagacaaacggcgaaacaggcgagatcgtgtgggataagggccgggactttgccaccgtgcggaaagtgctgtctatgccccaagtgaatatcgtgaaaaagaccgaggtgcagacaggcggcttcagcaaagagtctatcctgcccaagaggaacagcgacaagctgatcgccagaaagaaggactgggaccctaagaagtacggcggcttcgacagccccaccgtggcctattctgtgctggtggtggccaaagtggaaaagggcaagtccaagaaactgaagagtgtgaaagagctgctggggatcaccatcatggaaagaagcagcttcgagaagaatcccatcgactttctggaagccaagggctacaaagaagtgaaaaaggacctgatcatcaagctgcctaagtactccctgttcgagctggaaaacggccggaagagaatgctggcctctgccggcgaactgcagaagggaaacgaactggccctgccctccaaatatgtgaacttcctgtacctggccagccactatgagaagctgaagggctcccccgaggataatgagcagaaacagctgtttgtggaacagcacaaacactacctggacgagatcatcgagcagatcagcgagttctccaagagagtgatcctggccgacgctaatctggacaaggtgctgagcgcctacaacaagcacagagacaagcctatcagagagcaggccgagaatatcatccacctgtttaccctgaccaatctgggagcccctgccgccttcaagtactttgacaccaccatcgaccggaagaggtacaccagcaccaaagaggtgctggacgccaccctgatccaccagagcatcaccggcctgtacgagacacggatcgacctgtctcagctgggaggcgacgcctatccctatgacgtgcccgattatgccagcctgggcagcggctcccccaagaaaaaacgcaaggtggaagatcctaagaaaaagcggaaagtgtgataatagggatcccaagcacgcagcaatgcagctcaaaacgcttagcctagccacacccccacgggaaacagcagtgattaacctttagcaataaacgaaagtttaactaagctatactaaccccagggttggtcaatttcgtgccagccacaccctggtactgcatgcacgcaatgctagctgcccctttcccgtcctgggcaccccgagtctcccccgaccccgggtcccaggtatgctcccacctccacctgccccactcaccacctctgctagttccagacacctccgaagatgg

SEQ ID NO: 1192 - DNA, 6570 bp, synthetic construct
  misc_feature 1..6570: note = EPIREG CDS
  source 1..6570: mol_type = other DNA
atggtgcctgccgccaagagagtgaagctggacggcagcaaccacgaccaagagttcgaccctcctaaggtgtaccctcctgtgccagccgagaagcggaagcctatcagagtgctgagcctgttcgacggaatcgccacaggactgctggtgctgaaggatctgggaatccaggtggaccggtatatcgccagcgaagtgtgcgaggacagcatcacagttggcatggttcgacaccagggcaagattatgtacgtgggcgacgtgcggagcgtgacccagaaacacattcaagagtggggccccttcgacctggttatcggcggcagcccttgcaacgatctgagcatcgtgaaccccgccagaaagggcctgtatgaaggcaccggcagactgttcttcgagttctacagactgctgcacgacgccagacctaaagagggcgacgacagaccattcttctggctgttcgagaacgtggtggctatgggcgtgtccgacaagcgggacatcagccggtttctggaaagcaaccccgtgatgatcgacgccaaagaggtgtccgctgctcaccgggccagatacttttggggcaatctgcccggcatgaacagacctctggccagcaccgtgaacgacaagctggaactgcaagagtgcctggaacacggccggatcgccaagtttagcaaagtgcggaccatcaccaccaggtccaacagcatcaagcagggcaaagaccagcacttccccgtgttcatgaatgagaaagaggacatcctgtggtgcaccgagatggaaagagtgttcggcttccctgtgcactacaccgacgtgtccaacatgagcagactggccagacagaggctgctgggcagatcttggagcgtgccagtgatcagacacctgttcgcccctctgaaagaatacttcgcctgcgtgtccagcggcaacagcaacgccaatagcagaggccctagcttcagctctggactggtgcctttgagcctgagaggcagccacatgttcgagacagtgcctgtgtggcggagacagcccgttagagtgctgtccctgtttgaggacatcaagaaagagctgaccagcctgggcttcctggaaagcggatctgatcctggccagctgaagcacgtggtggacgtgaccgataccgtgcggaaggatgtggaagaatggggcccttttgatctggtgtacggcgccacacctcctctgggccacacatgtgatagacctccaagctggtatctgttccagttccaccggctgctgcagtacgctagacccaagcctggaagccccaggcctttcttttggatgttcgtggacaacctggtcctgaacaaagaggacctggacgtcgccagccggttcctcgaaatggaacctgtgacaatccccgacgtgcacggcggatctctgcagaatgctgtcagagtgtggtctaacatccccgccatcagaagcagcagacactgggcccttgtgtccgaggaagaactgtctctgctggcccagaacaagcagagcagcaagctggccgccaagtggcctacaaagctggtcaagaactgcttcctgcctctgcgcgagtacttcaagtatttcagcggcggacctagctctggcgcccctccacctagcggaggatctccagcaggatctcctaccagcaccgaggaaggcacaagcgagtctgccacacctgagtctggccctggcacatctacagagcctagcgagggatctgcccctggatctcctgctggcagccctacatctaccgaagagggaaccagcacagagccttccgaaggttctgctcctggcacaagcaccgagccaagcgagatgaacaacagccagggcagagtgaccttcgaggatgtgaccgtgaacttcacccaaggcgagtggcagagactgaaccccgagcagagaaacctgtaccgggacgtgatgctggaaaactacagcaacctggtgtccgtcggccagggcgagacaacaaagcctgacgtgatcctgcggctggaacagggaaaagagccttggctggaagaggaagaggtgctcggatctggacgggccgagaagaacggcgatattggcggacagatctggaagcctaaggacgtgaaagagagcctgagcggctctgaaacacctggaacaagcgaaggcggaccaggcacctctaccgaaccatctgagggaagcgctccaggttctcctgccggctctccaacaagcacagaagagggcacctccactgagccctctgaaggcagtgctcctggaacttccaccgaaccttccgagccaaagaagaaacgcaaggtgggctccgacaagaagtacagcatcggcctggccatcggcaccaactctgtgggctgggccgtgatcaccgacgagtacaaggtgcccagcaagaaattcaaggtgctgggcaacaccgaccggcacagcatcaagaagaacctgatcggcgccctgctgttcgacagcggagaaacagccgaggccacccggctgaagagaaccgccagaagaagatacaccagacggaagaaccggatctgctatctgcaagagatcttcagcaacgagatggccaaggtggacgacagcttcttccacagactggaagagtccttcctggtggaagaggataagaagcacgagcggcaccccatcttcggcaacatcgtggacgaggtggcctaccacgagaagtaccccaccatctaccacctgagaaagaaactggtggacagcaccgacaaggccgacctgcggctgatctatctggccctggcccacatgatcaagttccggggccacttcctgatcgagggcgacctgaaccccgacaacagcgacgtggacaagctgttcatccagctggtgcagacctacaaccagctgttcgaggaaaaccccatcaacgccagcggcgtggacgccaaggccatcctgtctgccagactgagcaagagcagacggctggaaaatctgatcgcccagctgcccggcgagaagaagaatggcctgttcggcaacctgattgccctgagcctgggcctgacccccaacttcaagagcaacttcgacctggccgaggatgccaaactgcagctgagcaaggacacctacgacgacgacctggacaacctgctggcccagatcggcgaccagtacgccgacctgtttctggccgccaagaacctgtccgacgccatcctgctgagcgacatcctgagagtgaacaccgagatcaccaaggcccccctgagcgcctctatgatcaagagatacgacgagcaccaccaggacctgaccctgctgaaagctctcgtgcggcagcagctgcctgagaagtacaaagagattttcttcgaccagagcaagaacggctacgccggctacatcgatggcggagccagccaggaagagttctacaagttcatcaagcccatcctggaaaagatggacggcaccgaggaactgctcgtgaagctgaacagagaggacctgctgcggaagcagcggaccttcgacaacggcagcatcccccaccagatccacctgggagagctgcacgccattctgcggcggcaggaagatttttacccattcctgaaggacaaccgggaaaagatcgagaagatcctgaccttccgcatcccctactacgtgggccctctggccaggggaaacagcagattcgcctggatgaccagaaagagcgaggaaaccatcaccccctggaacttcgaggaagtggtggacaagggcgccagcgcccagagcttcatcgagcggatgaccaacttcgataagaacctgcccaacgagaaggtgctgcccaagcacagcctgctgtacgagtacttcaccgtgtacaacgagctgaccaaagtgaaatacgtgaccgagggaatgagaaagcccgccttcctgagcggcgagcagaaaaaagccatcgtggacctgctgttcaagaccaaccggaaagtgaccgtgaagcagctgaaagaggactacttcaagaaaatcgagtgcttcgactccgtggaaatctccggcgtggaagatcggttcaacgcctccctgggcacataccacgatctgctgaaaattatcaaggacaaggacttcctggacaatgaggaaaacgaggacattctggaagatatcgtgctgaccctgacactgtttgaggacagagagatgatcgaggaacggctgaaaacctatgcccacctgttcgacgacaaagtgatgaagcagctgaagcggcggagatacaccggctggggcaggctgagccggaagctgatcaacggcatccgggacaagcagtccggcaagacaatcctggatttcctgaagtccgacggcttcgccaacagaaacttcatgcagctgatccacgacgacagcctgacctttaaagaggacatccagaaagcccaggtgtccggccagggcgatagcctgcacgagcacattgccaatctggccggcagccccgccattaagaagggcatcctgcagacagtgaaggtggtggacgagctcgtgaaagtgatgggccggcacaagcccgagaacatcgtgatcgaaatggccagagagaaccagaccacccagaagggacagaagaacagccgcgagagaatgaagcggatcgaagagggcatcaaagagctgggcagccagatcctgaaagaacaccccgtggaaaacacccagctgcagaacgagaagctgtacctgtactacctgcagaatgggcgggatatgtacgtggaccaggaactggacatcaaccggctgtccgactacgatgtggacgctatcgtgcctcagagctttctgaaggacgactccatcgataacaaagtgctgactcggagcgacaagaaccggggcaagagcgacaacgtgccctccgaagaggtcgtgaagaagatgaagaactactggcgccagctgctgaatgccaagctgattacccagaggaagttcgacaatctgaccaaggccgagagaggcggcctgagcgaactggataaggccggcttcatcaagagacagctggtggaaacccggcagatcacaaagcacgtggcacagatcctggactcccggatgaacactaagtacgacgagaacgacaaactgatccgggaagtgaaagtgatcaccctgaagtccaagctggtgtccgatttccggaaggatttccagttttacaaagtgcgcgagatcaacaactaccaccacgcccacgacgcctacctgaacgccgtcgtgggaaccgccctgatcaaaaagtaccctaagctggaaagcgagttcgtgtacggcgactacaaggtgtacgacgtgcggaagatgatcgccaagagcgagcaggaaatcggcaaggctaccgccaagtacttcttctacagcaacatcatgaactttttcaagaccgagattaccctggccaacggcgagatccggaagcggcctctgatcgagacaaacggcgaaacaggcgagatcgtgtgggataagggccgggactttgccaccgtgcggaaagtgctgtctatgccccaagtgaatatcgtgaaaaagaccgaggtgcagacaggcggcttcagcaaagagtctatcctgcccaagaggaacagcgacaagctgatcgccagaaagaaggactgggaccctaagaagtacggcggcttcgacagccccaccgtggcctattctgtgctggtggtggccaaagtggaaaagggcaagtccaagaaactgaagagtgtgaaagagctgctggggatcaccatcatggaaagaagcagcttcgagaagaatcccatcgactttctggaagccaagggctacaaagaagtgaaaaaggacctgatcatcaagctgcctaagtactccctgttcgagctggaaaacggccggaagagaatgctggcctctgccggcgaactgcagaagggaaacgaactggccctgccctccaaatatgtgaacttcctgtacctggccagccactatgagaagctgaagggctcccccgaggataatgagcagaaacagctgtttgtggaacagcacaaacactacctggacgagatcatcgagcagatcagcgagttctccaagagagtgatcctggccgacgctaatctggacaaggtgctgagcgcctacaacaagcacagagacaagcctatcagagagcaggccgagaatatcatccacctgtttaccctgaccaatctgggagcccctgccgccttcaagtactttgacaccaccatcgaccggaagaggtacaccagcaccaaagaggtgctggacgccaccctgatccaccagagcatcaccggcctgtacgagacacggatcgacctgtctcagctgggaggcgacgcctatccctatgacgtgcccgattatgccagcctgggcagcggctcccccaagaaaaaacgcaaggtggaagatcctaagaaaaagcggaaagtgtga

SEQ ID NO: 1193 - DNA, 8906 bp, synthetic construct
  misc_feature 1..8906: note = EPIREG plasmid DNA
  source 1..8906: mol_type = other DNA
tgataatagggatcccaagcacgcagcaatgcagctcaaaacgcttagcctagccacacccccacgggaaacagcagtgattaacctttagcaataaacgaaagtttaactaagctatactaaccccagggttggtcaatttcgtgccagccacaccctggtactgcatgcacgcaatgctagctgcccctttcccgtcctgggcaccccgagtctcccccgaccccgggtcccaggtatgctcccacctccacctgccccactcaccacctctgctagttccagacacctccgaagatggaaaaaaaaaaaaaaaaaaaaaaaaaaaaaaaaaaaaaaaaaaaaaaaaaaaaaaaaaaaaaaaaaaaaaaaaaaaaaaaaaaaaaaaaaaaaaaaaaaaaaaaaaaaaaaaaaaaaaaaaaaaagcttggatcattgtcactttcaccgtcatcaccgaaacgcgcgatgcagctctggcccgtgtctcaaaatctctgatgttacattgcacaagataaaaatatatcatcatgaacaataaaactgtctgcttacataaacagtaatacaaggggtgttatgagccatattcaacgggaaacgtcgaggccgcgattaaattccaacatggatgctgatttatatgggtataaatgggctcgcgataatgtcgggcaatcaggtgcgacaatctatcgcttgtatgggaagcccgatgcgccagagttgtttctgaaacatggcaaaggtagcgttgccaatgatgttacagatgagatggtcagactaaactggctgacggaatttatgcctcttccgaccatcaagcattttatccgtactcctgatgatgcatggttactcaccactgcgatccccggaaaaacagcattccaggtattagaagaatatcctgattcaggtgaaaatattgttgatgcgctggcagtgttcctgcgccggttgcattcgattcctgtttgtaattgtccttttaacagcgatcgcgtatttcgtctcgctcaggcgcaatcacgaatgaataacggtttggttgatgcgagtgattttgatgacgagcgtaatggctggcctgttgaacaagtctggaaagaaatgcataaacttttgccattctcaccggattcagtcgtcactcatggtgatttctcacttgataaccttatttttgacgaggggaaattaataggttgtattgatgttggacgagtcggaatcgcagaccgataccaggatcttgccatcctatggaactgcctcggtgagttttctccttcattacagaaacggctttttcaaaaatatggtattgataatcctgatatgaataaattgcagtttcatttgatgctcgatgagtttttctaatcagaattggttaattggttgtaacattattcagattgggcttgatttaaaacttcatttttaatttaaaaggatctaggtgaagatcctttttgataatctcatgaccaaaatcccttaacgtgagttttcgttccactgagcgtcagaccccgtagaaaagatcaaaggatcttcttgagatcctttttttctgcgcgtaatctgctgcttgcaaacaaaaaaaccaccgctaccagcggtggtttgtttgccggatcaagagctaccaactctttttccgaaggtaactggcttcagcagagcgcagataccaaatactgttcttctagtgtagccgtagttaggccaccacttcaagaactctgtagcaccgcctacatacctcgctctgctaatcctgttaccagtggctgctgccagtggcgataagtcgtgtcttaccgggttggactcaagacgatagttaccggataaggcgcagcggtcgggctgaacggggggttcgtgcacacagcccagcttggagcgaacgacctacaccgaactgagatacctacagcgtgagctatgagaaagcgccacgcttcccgaagggagaaaggcggacaggtatccggtaagcggcagggtcggaacaggagagcgcacgagggagcttccagggggaaacgcctggtatctttatagtcctgtcgggtttcgccacctctgacttgagcgtcgatttttgtgatgctcgtcaggggggcggagcctatggaaaaacgccagcaacgcggcctttttacggttcctggccttttgctggccttttgctcacattctagataatacgactcactataaggactcactatttgttttcgcgcccagttgcaaaaagtgtcgacatttgcttctgacacaactgtgttcactagcaacctcaaacagacaccgccaccatggtgcctgccgccaagagagtgaagctggacggcagcaaccacgaccaagagttcgaccctcctaaggtgtaccctcctgtgccagccgagaagcggaagcctatcagagtgctgagcctgttcgacggaatcgccacaggactgctggtgctgaaggatctgggaatccaggtggaccggtatatcgccagcgaagtgtgcgaggacagcatcacagttggcatggttcgacaccagggcaagattatgtacgtgggcgacgtgcggagcgtgacccagaaacacattcaagagtggggccccttcgacctggttatcggcggcagcccttgcaacgatctgagcatcgtgaaccccgccagaaagggcctgtatgaaggcaccggcagactgttcttcgagttctacagactgctgcacgacgccagacctaaagagggcgacgacagaccattcttctggctgttcgagaacgtggtggctatgggcgtgtccgacaagcgggacatcagccggtttctggaaagcaaccccgtgatgatcgacgccaaagaggtgtccgctgctcaccgggccagatacttttggggcaatctgcccggcatgaacagacctctggccagcaccgtgaacgacaagctggaactgcaagagtgcctggaacacggccggatcgccaagtttagcaaagtgcggaccatcaccaccaggtccaacagcatcaagcagggcaaagaccagcacttccccgtgttcatgaatgagaaagaggacatcctgtggtgcaccgagatggaaagagtgttcggcttccctgtgcactacaccgacgtgtccaacatgagcagactggccagacagaggctgctgggcagatcttggagcgtgccagtgatcagacacctgttcgcccctctgaaagaatacttcgcctgcgtgtccagcggcaacagcaacgccaatagcagaggccctagcttcagctctggactggtgcctttgagcctgagaggcagccacatgttcgagacagtgcctgtgtggcggagacagcccgttagagtgctgtccctgtttgaggacatcaagaaagagctgaccagcctgggcttcctggaaagcggatctgatcctggccagctgaagcacgtggtggacgtgaccgataccgtgcggaaggatgtggaagaatggggcccttttgatctggtgtacggcgccacacctcctctgggccacacatgtgatagacctccaagctggtatctgttccagttccaccggctgctgcagtacgctagacccaagcctggaagccccaggcctttcttttggatgttcgtggacaacctggtcctgaacaaagaggacctggacgtcgccagccggttcctcgaaatggaacctgtgacaatccccgacgtgcacggcggatctctgcagaatgctgtcagagtgtggtctaacatccccgccatcagaagcagcagacactgggcccttgtgtccgaggaagaactgtctctgctggcccagaacaagcagagcagcaagctggccgccaagtggcctacaaagctggtcaagaactgcttcctgcctctgcgcgagtacttcaagtatttcagcggcggacctagctctggcgcccctccacctagcggaggatctccagcaggatctcctaccagcaccgaggaaggcacaagcgagtctgccacacctgagtctggccctggcacatctacagagcctagcgagggatctgcccctggatctcctgctggcagccctacatctaccgaagagggaaccagcacagagccttccgaaggttctgctcctggcacaagcaccgagccaagcgagatgaacaacagccagggcagagtgaccttcgaggatgtgaccgtgaacttcacccaaggcgagtggcagagactgaaccccgagcagagaaacctgtaccgggacgtgatgctggaaaactacagcaacctggtgtccgtcggccagggcgagacaacaaagcctgacgtgatcctgcggctggaacagggaaaagagccttggctggaagaggaagaggtgctcggatctggacgggccgagaagaacggcgatattggcggacagatctggaagcctaaggacgtgaaagagagcctgagcggctctgaaacacctggaacaagcgaaggcggaccaggcacctctaccgaaccatctgagggaagcgctccaggttctcctgccggctctccaacaagcacagaagagggcacctccactgagccctctgaaggcagtgctcctggaacttccaccgaaccttccgagccaaagaagaaacgcaaggtgggctccgacaagaagtacagcatcggcctggccatcggcaccaactctgtgggctgggccgtgatcaccgacgagtacaaggtgcccagcaagaaattcaaggtgctgggcaacaccgaccggcacagcatcaagaagaacctgatcggcgccctgctgttcgacagcggagaaacagccgaggccacccggctgaagagaaccgccagaagaagatacaccagacggaagaaccggatctgctatctgcaagagatcttcagcaacgagatggccaaggtggacgacagcttcttccacagactggaagagtccttcctggtggaagaggataagaagcacgagcggcaccccatcttcggcaacatcgtggacgaggtggcctaccacgagaagtaccccaccatctaccacctgagaaagaaactggtggacagcaccgacaaggccgacctgcggctgatctatctggccctggcccacatgatcaagttccggggccacttcctgatcgagggcgacctgaaccccgacaacagcgacgtggacaagctgttcatccagctggtgcagacctacaaccagctgttcgaggaaaaccccatcaacgccagcggcgtggacgccaaggccatcctgtctgccagactgagcaagagcagacggctggaaaatctgatcgcccagctgcccggcgagaagaagaatggcctgttcggcaacctgattgccctgagcctgggcctgacccccaacttcaagagcaacttcgacctggccgaggatgccaaactgcagctgagcaaggacacctacgacgacgacctggacaacctgctggcccagatcggcgaccagtacgccgacctgtttctggccgccaagaacctgtccgacgccatcctgctgagcgacatcctgagagtgaacaccgagatcaccaaggcccccctgagcgcctctatgatcaagagatacgacgagcaccaccaggacctgaccctgctgaaagctctcgtgcggcagcagctgcctgagaagtacaaagagattttcttcgaccagagcaagaacggctacgccggctacatcgatggcggagccagccaggaagagttctacaagttcatcaagcccatcctggaaaagatggacggcaccgaggaactgctcgtgaagctgaacagagaggacctgctgcggaagcagcggaccttcgacaacggcagcatcccccaccagatccacctgggagagctgcacgccattctgcggcggcaggaagatttttacccattcctgaaggacaaccgggaaaagatcgagaagatcctgaccttccgcatcccctactacgtgggccctctggccaggggaaacagcagattcgcctggatgaccagaaagagcgaggaaaccatcaccccctggaacttcgaggaagtggtggacaagggcgccagcgcccagagcttcatcgagcggatgaccaacttcgataagaacctgcccaacgagaaggtgctgcccaagcacagcctgctgtacgagtacttcaccgtgtacaacgagctgaccaaagtgaaatacgtgaccgagggaatgagaaagcccgccttcctgagcggcgagcagaaaaaagccatcgtggacctgctgttcaagaccaaccggaaagtgaccgtgaagcagctgaaagaggactacttcaagaaaatcgagtgcttcgactccgtggaaatctccggcgtggaagatcggttcaacgcctccctgggcacataccacgatctgctgaaaattatcaaggacaaggacttcctggacaatgaggaaaacgaggacattctggaagatatcgtgctgaccctgacactgtttgaggacagagagatgatcgaggaacggctgaaaacctatgcccacctgttcgacgacaaagtgatgaagcagctgaagcggcggagatacaccggctggggcaggctgagccggaagctgatcaacggcatccgggacaagcagtccggcaagacaatcctggatttcctgaagtccgacggcttcgccaacagaaacttcatgcagctgatccacgacgacagcctgacctttaaagaggacatccagaaagcccaggtgtccggccagggcgatagcctgcacgagcacattgccaatctggccggcagccccgccattaagaagggcatcctgcagacagtgaaggtggtggacgagctcgtgaaagtgatgggccggcacaagcccgagaacatcgtgatcgaaatggccagagagaaccagaccacccagaagggacagaagaacagccgcgagagaatgaagcggatcgaagagggcatcaaagagctgggcagccagatcctgaaagaacaccccgtggaaaacacccagctgcagaacgagaagctgtacctgtactacctgcagaatgggcgggatatgtacgtggaccaggaactggacatcaaccggctgtccgactacgatgtggacgctatcgtgcctcagagctttctgaaggacgactccatcgataacaaagtgctgactcggagcgacaagaaccggggcaagagcgacaacgtgccctccgaagaggtcgtgaagaagatgaagaactactggcgccagctgctgaatgccaagctgattacccagaggaagttcgacaatctgaccaaggccgagagaggcggcctgagcgaactggataaggccggcttcatcaagagacagctggtggaaacccggcagatcacaaagcacgtggcacagatcctggactcccggatgaacactaagtacgacgagaacgacaaactgatccgggaagtgaaagtgatcaccctgaagtccaagctggtgtccgatttccggaaggatttccagttttacaaagtgcgcgagatcaacaactaccaccacgcccacgacgcctacctgaacgccgtcgtgggaaccgccctgatcaaaaagtaccctaagctggaaagcgagttcgtgtacggcgactacaaggtgtacgacgtgcggaagatgatcgccaagagcgagcaggaaatcggcaaggctaccgccaagtacttcttctacagcaacatcatgaactttttcaagaccgagattaccctggccaacggcgagatccggaagcggcctctgatcgagacaaacggcgaaacaggcgagatcgtgtgggataagggccgggactttgccaccgtgcggaaagtgctgtctatgccccaagtgaatatcgtgaaaaagaccgaggtgcagacaggcggcttcagcaaagagtctatcctgcccaagaggaacagcgacaagctgatcgccagaaagaaggactgggaccctaagaagtacggcggcttcgacagccccaccgtggcctattctgtgctggtggtggccaaagtggaaaagggcaagtccaagaaactgaagagtgtgaaagagctgctggggatcaccatcatggaaagaagcagcttcgagaagaatcccatcgactttctggaagccaagggctacaaagaagtgaaaaaggacctgatcatcaagctgcctaagtactccctgttcgagctggaaaacggccggaagagaatgctggcctctgccggcgaactgcagaagggaaacgaactggccctgccctccaaatatgtgaacttcctgtacctggccagccactatgagaagctgaagggctcccccgaggataatgagcagaaacagctgtttgtggaacagcacaaacactacctggacgagatcatcgagcagatcagcgagttctccaagagagtgatcctggccgacgctaatctggacaaggtgctgagcgcctacaacaagcacagagacaagcctatcagagagcaggccgagaatatcatccacctgtttaccctgaccaatctgggagcccctgccgccttcaagtactttgacaccaccatcgaccggaagaggtacaccagcaccaaagaggtgctggacgccaccctgatccaccagagcatcaccggcctgtacgagacacggatcgacctgtctcagctgggaggcgacgcctatccctatgacgtgcccgattatgccagcctgggcagcggctcccccaagaaaaaacgcaaggtggaagatcctaagaaaaagcggaaagtg

SEQ ID NO: 1194 - protein, 2190 aa, synthetic construct
  REGION 1..2190: note = EPIREG amino acid
  SITE 2190: note = misc_feature - Xaa =
MVPAAKRVKLDGSNHDQEFDPPKVYPPVPAEKRKPIRVLSLFDGIATGLLVLKDLGIQVDRYIASEVCEDSITVGMVRHQGKIMYVGDVRSVTQKHIQEWGPFDLVIGGSPCNDLSIVNPARKGLYEGTGRLFFEFYRLLHDARPKEGDDRPFFWLFENVVAMGVSDKRDISRFLESNPVMIDAKEVSAAHRARYFWGNLPGMNRPLASTVNDKLELQECLEHGRIAKFSKVRTITTRSNSIKQGKDQHFPVFMNEKEDILWCTEMERVFGFPVHYTDVSNMSRLARQRLLGRSWSVPVIRHLFAPLKEYFACVSSGNSNANSRGPSFSSGLVPLSLRGSHMFETVPVWRRQPVRVLSLFEDIKKELTSLGFLESGSDPGQLKHVVDVTDTVRKDVEEWGPFDLVYGATPPLGHTCDRPPSWYLFQFHRLLQYARPKPGSPRPFFWMFVDNLVLNKEDLDVASRFLEMEPVTIPDVHGGSLQNAVRVWSNIPAIRSSRHWALVSEEELSLLAQNKQSSKLAAKWPTKLVKNCFLPLREYFKYFSGGPSSGAPPPSGGSPAGSPTSTEEGTSESATPESGPGTSTEPSEGSAPGSPAGSPTSTEEGTSTEPSEGSAPGTSTEPSEMNNSQGRVTFEDVTVNFTQGEWQRLNPEQRNLYRDVMLENYSNLVSVGQGETTKPDVILRLEQGKEPWLEEEEVLGSGRAEKNGDIGGQIWKPKDVKESLSGSETPGTSEGGPGTSTEPSEGSAPGSPAGSPTSTEEGTSTEPSEGSAPGTSTEPSEPKKKRKVGSDKKYSIGLAIGTNSVGWAVITDEYKVPSKKFKVLGNTDRHSIKKNLIGALLFDSGETAEATRLKRTARRRYTRRKNRICYLQEIFSNEMAKVDDSFFHRLEESFLVEEDKKHERHPIFGNIVDEVAYHEKYPTIYHLRKKLVDSTDKADLRLIYLALAHMIKFRGHFLIEGDLNPDNSDVDKLFIQLVQTYNQLFEENPINASGVDAKAILSARLSKSRRLENLIAQLPGEKKNGLFGNLIALSLGLTPNFKSNFDLAEDAKLQLSKDTYDDDLDNLLAQIGDQYADLFLAAKNLSDAILLSDILRVNTEITKAPLSASMIKRYDEHHQDLTLLKALVRQQLPEKYKEIFFDQSKNGYAGYIDGGASQEEFYKFIKPILEKMDGTEELLVKLNREDLLRKQRTFDNGSIPHQIHLGELHAILRRQEDFYPFLKDNREKIEKILTFRIPYYVGPLARGNSRFAWMTRKSEETITPWNFEEVVDKGASAQSFIERMTNFDKNLPNEKVLPKHSLLYEYFTVYNELTKVKYVTEGMRKPAFLSGEQKKAIVDLLFKTNRKVTVKQLKEDYFKKIECFDSVEISGVEDRFNASLGTYHDLLKIIKDKDFLDNEENEDILEDIVLTLTLFEDREMIEERLKTYAHLFDDKVMKQLKRRRYTGWGRLSRKLINGIRDKQSGKTILDFLKSDGFANRNFMQLIHDDSLTFKEDIQKAQVSGQGDSLHEHIANLAGSPAIKKGILQTVKVVDELVKVMGRHKPENIVIEMARENQTTQKGQKNSRERMKRIEEGIKELGSQILKEHPVENTQLQNEKLYLYYLQNGRDMYVDQELDINRLSDYDVDAIVPQSFLKDDSIDNKVLTRSDKNRGKSDNVPSEEVVKKMKNYWRQLLNAKLITQRKFDNLTKAERGGLSELDKAGFIKRQLVETRQITKHVAQILDSRMNTKYDENDKLIREVKVITLKSKLVSDFRKDFQFYKVREINNYHHAHDAYLNAVVGTALIKKYPKLESEFVYGDYKVYDVRKMIAKSEQEIGKATAKYFFYSNIMNFFKTEITLANGEIRKRPLIETNGETGEIVWDKGRDFATVRKVLSMPQVNIVKKTEVQTGGFSKESILPKRNSDKLIARKKDWDPKKYGGFDSPTVAYSVLVVAKVEKGKSKKLKSVKELLGITIMERSSFEKNPIDFLEAKGYKEVKKDLIIKLPKYSLFELENGRKRMLASAGELQKGNELALPSKYVNFLYLASHYEKLKGSPEDNEQKQLFVEQHKHYLDEIIEQISEFSKRVILADANLDKVLSAYNKHRDKPIREQAENIIHLFTLTNLGAPAAFKYFDTTIDRKRYTSTKEVLDATLIHQSITGLYETRIDLSQLGGDAYPYDVPDYASLGSGSPKKKRKVEDPKKKRKVX

SEQ ID NO: 1195 - protein, 203 aa, synthetic construct
  REGION 1..203: note = human DNMT3L
MFETVPVWRRQPVRVLSLFEDIKKELTSLGFLESGSDPGQLKHVVDVTDTVRKDVEEWGPFDLVYGATPPLGHTCDRPPSWYLFQFHRLLQYARPKPGSPRPFFWMFVDNLVLNKEDLDVASRFLEMEPVTIPDVHGGSLQNAVRVWSNIPAIRSSRHWALVSEEELSLLAQNKQSSKLAAKWPTKLVKNCFLPLREYFKYFS

SEQ ID NO: 1196 - protein, 100 aa, synthetic construct
  REGION 1..100: note = ZIM3 KRAB
MNNSQGRVTFEDVTVNFTQGEWQRLNPEQRNLYRDVMLENYSNLVSVGQGETTKPDVILRLEQGKEPWLEEEEVLGSGRAEKNGDIGGQIWKPKDVKESL